European Patent Application EP 4 636 073 A1, published October 22, 2025. Title: Peribacillus aracenensis BBB004 estimulante del metabolismo adaptativo de plantas frente a estrés hídrico, mejoradora de la nutrición vegetal y del contenido de polifenoles. Applicant: BIOBAB R&D S.L. Application WO PCT/ES2023/070709, filed November 29, 2023. The sequence listing filed with the application follows.

SEQUENCE LISTING (324 sequences)

SEQ ID NO: 1 - DNA, 432 bp, Peribacillus Aracenensis
  source 1..432: mol_type = genomic DNA
atggaaataacggttagacaagtagataaagaagaagtttgggaattaaggcataaagttatgtgggcagataagccctttgactatataaaattagaagacgatgatttaggtattcattatgggctttttaaaggagatgatttgatttctgtcatctcactttttataaacaatagagaatgtcagttccgtaaatttgcaacccttcaactagaacaaggtaaagggtacggaagtacattgttagactatattataaaggaagcacagaacaatggcgtgaagagaatttggtgtaatgccagaaagaataaggtggatttttataaaaagtttggcttacaagagactaactccagctttatgaaagagggtaaatcctacgttataatggaagcttatgtgcagtcaattatggggattacctga

SEQ ID NO: 2 - DNA, 153 bp, Peribacillus Aracenensis
  source 1..153: mol_type = genomic DNA
atggaagcaggattttttaaggttataaaagtggatataaaaattagcctgaacccttacatgggctcaggttttttatttctgaatggaatttgcccatatgtatttttgtgtaagtttggaatatttatcaatacaatgacaattgaatag

SEQ ID NO: 3 - DNA, 210 bp, Peribacillus Aracenensis
  source 1..210: mol_type = genomic DNA
ttgctgatcgctgtgtggccaggaaaggcattttttccagagaggttgtattgtgtgtgtaggttccttcatcaagaaaaggctgaaatctttgaatggatatggacttaccatgtcaagttgacaactaaaaaaggctatgctgccatctggctcgatattcaatcggtgcctgatggcggacaagccccctttaaaattaagttttaa

SEQ ID NO: 4 - DNA, 138 bp, Peribacillus Aracenensis
  source 1..138: mol_type = genomic DNA
atgaaccccattatagagaagctgctgaagtttatgttggaaaataagaatgacatccaaattgcagaactttcgaatcgattttcaaagcgggcttcatatgaacttgtcctaatcaatataaggggccatgcttag

SEQ ID NO: 5 - DNA, 450 bp, Peribacillus Aracenensis
  source 1..450: mol_type = genomic DNA
ttgaagataagccagtctcaaacttggtttgggatgagtccagttgattggaacggaaggtacgagactcctgcgggaaaagcgcgtccaaaggagaccccacaggcgcaaaagcgccgaggaggctcccggaccgcccgcggaaagcgagtgcctggagtggaaatcaacgttccttttacaaaccctcaaataaccgtttcagtgatttcagaaacccgctcccttttttcgaaaactgaacacatccccatgatatatggctttacattaaatgaagaagtattgaatggttttggcacatccaatctaaggatgtgtttttcatttggccatcccctcattaaagttcaattgaatcaacattttcctattaataagatcctcgttaatccctttaaaactcactttttattccttccatttacccgttatgccatctggctttag

SEQ ID NO: 6 - DNA, 108 bp, Peribacillus Aracenensis
  source 1..108: mol_type = genomic DNA
atgcaagccggaagagataattctcttctggttttttgttcacagtggttatttggaggaacaattgcagaaaggtccaaaaaagaggatgaaaaaagaaaaaaataa

SEQ ID NO: 7 - DNA, 201 bp, Peribacillus Aracenensis
  source 1..201: mol_type = genomic DNA
atgattttaacaagaaaaaaatctacggaaaagaaggttttttccattttacacaggggaatagaagtatattataataatattttaaaaatttcgagaaagaaaattatgcacgaaggagaattttgttgtaatatggtagagaaaacacgcattaaatttcgaagttgttttttagtagataaggaggatgggaaatga

SEQ ID NO: 8 - DNA, 180 bp, Peribacillus Aracenensis
  source 1..180: mol_type = genomic DNA
gtggtatcagaaagattaggccattcaaaagttactatcacattggataaatatactcagttactcagaatatacaggactcctctgcagaaaacttttcaaaagctacaggaaaaaagagcacggaacaataaaagtggtcatttaactaaaaaagcaatggagaatcccattgcataa

SEQ ID NO: 9 - DNA, 687 bp, Peribacillus Aracenensis
  source 1..687: mol_type = genomic DNA
atgagtagtgataaaaataaagataaagataaaagagataaaggtacaggttccttaagcaattctaaaaatgaacctttaaaggaagaagcatgtccatcatcgagataccaggaatgcgttgatcgtgcttttcgtattcccatatttttaagcaccacaaatgcgttaaatccaatacaacaacagtttcaaaaccgacttattttagagattgagaacgcattgctttttccacgtacattgcctgtaagtgaacaatatccagaaaccattttaacaagtattcgtcggttggtttcatcaagttatggaatgttagcaatcaactttcgtcgcttcctcgtcgagattactgatactaatgtaggacaacctccatcttccactcctttctgggaagggtcagtttttttacaaattgaaccctctatggcttttcaatttggactacccatattattagtaagggaagctaatactgacacaaataatggaatttgggcaggaggaattgcccctctcaatacattcatagtttgggattctgaaaatcaatctgttgatgaattctttagtagtattcaatggagagaagcctttgcgaattggattgcggaggtaagaaatggatattataatcagacagagcctaaattcaagtacagatgtagtacacaagattaa

SEQ ID NO: 10 - DNA, 951 bp, Peribacillus Aracenensis
  source 1..951: mol_type = genomic DNA
atgattggggtgggtttactgaatattggctatctcttcatcatattgaatatgattgttttaggtctttcaatcccggccggcagtatagcaatggcaaccattcccgtatggctgtttacggcaatgacgcttggcatcgcctgtatgatcttactgccagcagcgaaaatatacgaaagaatcaagtggaaagggctaggatataaaacgtacttcgggatattcatgcaatccctttttaccgttacattatatacggtcttcctgttatatggtttgaaatactctagtgtgatagcggctggaatcataaatagtatggtgccagccgtaacgctggttctttccttcatattattgggagagagattgaacatccgtaagggcatagccatcatgctagctgtttcagctgtcctggtaatggagctcgcaggtgcgagtactgagggggaatccagtgcattagggattgctttcatgatattggcagttgtgtcattgggattgttttttgtatatgcaaagaaattcgcagtggatgtgccaccggtgacaatggcagcaggactgtgcttaatggggtttctaactacgctgccgatggccattcatgaggcgatatcttttgattggggaaaaatgacgcttggtttatggggagctgtcatagcctataccttgcttgggtgggtatttgcttatattttcacgtacttaggaatttcaaaggttccagcaagcaccatcgggatggcaacggcaatcatcccgattactgcaatgctatatgccgtgttattcctgggcgataaattacgaaaggtcgatatcattgcgactgttttattaattctatcgatattcattgcagaatcaaaagaaagtgtaaaggaaggaaaagagtccatgccagttatcgggaaagatgatgcggtaggcaaataa

SEQ ID NO: 11 - DNA, 90 bp, Peribacillus Aracenensis
  source 1..90: mol_type = genomic DNA
atggaggactcccttgatttcaagtatgtaaagtgtatatggattgtcgccaatgaatgggcaggacagtttgcaactcctcaatattag

SEQ ID NO: 12 - DNA, 255 bp, Peribacillus Aracenensis
  source 1..255: mol_type = genomic DNA
atggaactcgaggggcaggatagaagaataacagatatttgcagaaaaaatctgaatgaaatcggcgatattatgtttaagcaaagcatcaggtttctcttaatgtattttgtagtattaaccgtttggaaatttattgctaacaaagaggttaattggattgataacataatggtcagttttatcatgttcttgattattccgttatataaatggtcgggaattccatataagtggagtaaggacaagcaatga

SEQ ID NO: 13 - DNA, 255 bp, Peribacillus Aracenensis
  source 1..255: mol_type = genomic DNA
atggcaggaatccatttaccaatcgaaaaggaaagaaccacgcagatagtttataagcaaattaaaaaagcgattgtatttggtggcattaccggtgatgaagtatttacaaaagttcaattagcggaagggttaaatacttcaagaacgcctgtaagggcagctattcaagatttcaagaaacaatttaacagcttaacagcgaaccttaattgttttacggcacgtagcttatttggaaccttattcgtatga

SEQ ID NO: 14 - DNA, 159 bp, Peribacillus Aracenensis
  source 1..159: mol_type = genomic DNA
atggatggaggtcaaacctgttgcgatggactgggaaatgaatcgccttgtccgacttgctgctgttctagccattcgcctaaggaatttactagtgttgcggatatggaaaagggaatcgacattttaagtgaaatactatataaattagcctattaa

SEQ ID NO: 15 - DNA, 135 bp, Peribacillus Aracenensis
  source 1..135: mol_type = genomic DNA
atggccgccacccagactgtagatcaactcaatgaaactcaagtttgcctacgttttttttttatggcttataccatttggacgttgatttctgctccaggcactcgctccaatcaactttgtaataaactttag

SEQ ID NO: 16 - DNA, 912 bp, Peribacillus Aracenensis
  source 1..912: mol_type = genomic DNA
atggacataagacaactgcgatattttattgcgatggtagaagaaagaaaaattactgctgcagctgaaaagcttcatatctcccagcctccattaagccaacacttgaaagcgatggaagatgaactaggaactaaattactagtgaggaataggagaaatttagaagttactgaagcggggaaatctttatataaatatgccttacaaatgactcagttaatggaagaagctaaaatggaaattaaggaaattggaaatggagtaaacggaagacttacgataggcataaatactttttcggtagtcgaattatcaaaattacttcaacaattccaccaaaaataccctaaagttacctataaaatacaacaaaatgaatcgtctcaactttgtaaattagtgagagaccgaatagtagagctagcgattatacaattaccgctcgagttagatgatttttcagtcatccatctaaatacagaacctttttactttattacgtcaaacaaccagaagtcttttaatcatgaggtctcacttgctgaaattcaaaactaccgactcattttacctagcacggaaggattaggtgtccattatatgattttggaggcattttcgaggcatcaactgcgtcctaacattgttgccgagtgttcggatatctcccttttattggatttagttgaatctggctttggagcgtcaattgttccagaaaccgtaatcaaaaaatacaaaagtcactatttacaagcttccaaagttatggttaccgagctaacttcatcaacgggaataatatggttgaaggactattacctgtcaggcgcagctcaaaattttattaacctattaacagagaccatgttcgctcccaataaaaacttgacggcctttcccaattga

SEQ ID NO: 17 - DNA, 1290 bp, Peribacillus Aracenensis
  source 1..1290: mol_type = genomic DNA
atggagatacttcgttttaaaagcactttaagtacatttcaatggtttatttttctactggcgaactctattgcattaccgatcgtaattggtggcatctttcatatgtcaatcggggaaatttctgaattaatgcagcgaacatttttggtagtaggaattagttcttttatgcaaggatgtttcgggcatcgctatccaattgctgacggaccagcaggttcatgggttagtgtgtttgtaatattggcagatgtcgctattcagcaggggcaaaacacgaatgaaaccttacaaattttagaaggcggattgatcgttgctggtcttttgctcttcatccttggtataaccggttttgttaatcagctgctatttttgttcacgcctttagtaaccggatcctttcttttgatcctggctcttcaacttagtggtgtttttttggaaggaatgattgcatttcaaggagagcactcccgtcctgattatggagcatcagcgatttcattcggtgtatttttactgatcattacgttatccgttaaagggaaaggctggattaaaagttacgccgttctaattgggattttattaggatggtcgctatatttcttattgggtaaaacctccaatttgttatcccaatcagattctttcattaaactaccggaaatatttgcttggggagtcccacagctgaatggcggaatcatattaacttctattctgtttatgtttcttttagtatcaaatacgattgcatccattacagctgttaaacaagtggtgccagaatctcggaaagatgaaaaacaaaccctcaatcgtggtatttgggctggaggcatttcccattttatagcttctatattttctacgattggaatcgttccattgccagtatccgctggttttatccaattgacagggcaaaaacaaattcaaccgtttcttatagcatgcttggctttatcggggatagcttttatccctgcaatcgttaactttttctctttgcttccagtccctattgctagtgctgcactaatggcatcattcgttcaaatgatcggcattgccattcagtctattcaacgggaagaactagaccaacgccgattgactatattaggaatcacattgttgatgggcattggaataatgtttctgcctgcagggatttttcaaggtcttccttctattttgcaatatgtctgcagcaacgggttgcttgttggtactatgattgtaatcctgctggaacagctatggaaaacaaaagattaa

SEQ ID NO: 18 - DNA, 462 bp, Peribacillus Aracenensis
  source 1..462: mol_type = genomic DNA
atgagtcacgaagaattcatgcaactggcaatagagttagcttacgataataccaaaaacaaaaagggaaagccgtttggtgcactcatcgttaaaaatggggagattgttgcaaaaggagtaaacgatgttctagaaacacacgatccaactgcgcacgcggagatgcaggctattcgtaaagcttgctgcacccttggcactgctgatctttccgaatgtgaactctacgcaagcggggagccttgccccatgtgtttaagcgccatttacttggcacattttaaaaatgtttactatgcatatactgcggacgaggaagaaaaaattgggctaggaacgaaatacgtttatcagcaaatagctctcccaatggaagagcgagacattaaattaattaagatagatagaaacccccaaaaaaatgatccttttgctctttggaaagaaattacctattaa

SEQ ID NO: 19 - DNA, 708 bp, Peribacillus Aracenensis
  source 1..708: mol_type = genomic DNA
atgtggaagtgggcggcatttataggatgtattctcttgcttcaaggatgtgtcccaaatgacagtgatgaaccgaaaaaacaagtaaaggagagagaaatcgtgagagaaggagtaaatgaacagctacttcaagctgccgaacgtggagatactgataccattagagaactgattaaggaaggcgtaaatattaatgtacaagactcaaagggacgaactgctaccatgattgcaacatatagcaatgatgtagagactgcaaaagtcctaattgaggcaggtgcggacgtcaacatccaagatgacatgaaaaatactcccttcctatatgctggtgcagaaggatatattgaaatcttgaagtttacgattgatggaggtgccgaccccaccattactaacagatatggaggaacagctttgataccagcctcggaacatgggtacgtcgatgtagtcaaagaacttgttacccatactgaaattgatgtaaatcatgtcaatagcctaggttggacagctttaatcgaggcaatcattctgaataatggaaacgcaaggcagcagcaaacggtgcaattgctgatagaacatggagcggatgtgaacataccagacaataaaaatgtgactcctttacaacacgcacgtcaggaagggtataaagagattgagaagattttgttaaaagcaggagcaaaataa

SEQ ID NO: 20 - DNA, 174 bp, Peribacillus Aracenensis
  source 1..174: mol_type = genomic DNA
atgtctcctggcatgccccatccttttgtatgcctagttatttcgcaaatggttctcgcttctatttcattcgaaacggtttatgcggttttaacaggtaaatttattgaatcaagaagtggcaattgttatgatagggttgaagagaaaacttggaaggagcaaatgccatga

SEQ ID NO: 21 - DNA, 504 bp, Peribacillus Aracenensis
  source 1..504: mol_type = genomic DNA
atgtcctttatggtctggcaaaaggcaaaaatgatcgtagtatcattggaatccactcaaagctttgtcatcaataaaactgtcaacggtgaagaaatcactccttttctgaaccaattcattaaagagagctattatttcaataacttttatcaccaaactggccaggggaaaacatccgattcagaatttattattgagaattccctctatcctttaggtaggggtgccgtatttttcactcatgcccaaaatgaatacaaagccatccccgaaatcttaacggaaaaaggttacaatacggctaccttccatgccaataataaaagcttttggagtactccgacaaaatcatttatggggatttgctccgattttatgagcaacgttgataaaggaaacctggcacaatccaggtttttttgttttttcgggagaatcagtagcactacaattatgaaacacattagacttcctgaacatctttctgttttcgcctcataa

SEQ ID NO: 22 - DNA, 195 bp, Peribacillus Aracenensis
  source 1..195: mol_type = genomic DNA
atggtactatcatttaagatgaaggaaggtgtgaaggaattggataactcttattttgtaggttgggggacattggcactcataaacgccggacttgctcaaggaaaaaatagaacggcattgaattggttcttgctatcattatttttgggtccgctcgctacatttatacttttattcgcaaagaaaagataa

SEQ ID NO: 23 - DNA, 1149 bp, Peribacillus Aracenensis
  source 1..1149: mol_type = genomic DNA
atgtataataattacattcttgatttgtcaagtctacccaaggaattaaggttattactggagattatgaagacggatgaacataatattataggctcagtaaaaaaagaactatatgtagacatcgactgggaagtatttctacaattagctaggcatcatcgcgtttacccattagtttattctaaactgaaaaatactcatgataatcaaatacctccgcatgttattcaaaccttatacaaagaatacaaaaaaaatacattccaaatgcttcacttaagcggagaaatggaacaagtgagtgaaatttttaataaaaatagtattcgtattctttttttaaagggcccaattattgctcaggaactctatggagatatttcccttcggacatcaaaggatatagatatattaatctcaatgactgatattaaaaaagctgagaaaattcttttaaattgtgggtatgagaaagaggaaagtcccaatattcttaacgagtggaaatggagaactcaccatatttcatattatcattcacaaaagcaaattcaaattgaaattcattggagactaaatccttttccatcaaaggaaccaagctttgaaaagttatgggaaaggaaaaggactagtaaccttacaacatatccagtttatcttttgggagaagaggatttatttttatatcttattactcatggtgcccggcacggttggtttcgtcttcgttggttgatagatatagatcaaatggttttaaaaggtctaagggagaaacaaataatctcatcgttgaaaaaatataaatatcaccgtatagtaggacaagcgcttattttaacttctcaactattaaatactcccgtaaactcagagctgaaaaaattaacaatagacaactattcggaaaaattggcacaaaaatcaatattgttcataagtgaaaaaagtcaatttgaatatccgaaagattatatggatttattaaaaactaattggcaaaaattcatttctttgattatgagaatttaccccagatatatagatgctaatactttaaaattgcctttgcccttacattttttatatttcccattacgtccttttttatgggtctggagaaagacgaggaaatctacttga

SEQ ID NO: 24 - DNA, 1761 bp, Peribacillus Aracenensis
  source 1..1761: mol_type = genomic DNA
ttgaatcgtagaaacctgttacggaattttgtaatatttatttttgctttcctttttggctatacaataaaaaaggaaggtgaaaatatgttattagaaaaagttgatcctaccatagtaagcagtaaggatggaaagttgattggtgaaaaaatcaaagcgttaaatgaacaattggcggataattctaagaatatcacaagtttatcaaagaaaaatgaagtaagtattacggattacgagaataaaaaggttgaggatgattggtttcctgcattccaagcagcattaaaatctattggtagcactggtagtataaaatttccaggaaatacaacatacaacatgtattctcctttgattctcccgttaacagggagtagaataagattgttttcaaacgatggagctataatttccgcaaaacataaccgagattgtatcattttaaattcccataatgagaactattcagctcacattatcgaaggtctagttattcaaggaccaaataaggaatatccaaaagatggttatatccctccaagtattggagcgggtgttcggatgaatacttcatactactgtacattacgtgacgttcgtatacaggggtttaaatatggcattcacattagaaaaggagttaagaataattttgaaggaagtacctatattagatttaatcaatacggaatttacttagatggaggtgcttctaatgtaaataatttcaaaggaataggaatacgtgaaaacagaaaagccggagtttatgtcaatcatactagttctgattcctatccaacgcataatacattttccgactgtattatagaatcaaatataccattcccttataaagtgggaggtaatgctcctgatgatagtataggtgtttatctaggtggagcatattacaatatatttgataactgctactttgaaaatcatcaatatgctatttatttaacagataatgcggacggtaacaagtttaataaatgtagactttctccgagtgaagataaaactagactagataaggtaatatttgatggaatgggtgtaaacaataatacgtttagtgaatgtatatcattgtcttttgacaatacgacaccaaacgttgagtcaaacgtctctggtcagctttataatcaatttattaattgtgaaggttttaattttatatcttctagtctagtttctagtgtagatattataaataatcgacctaaccaaactggttttggaacgccctttggggcattatcaattccttcacacggtttctacaacaatcctagagaaggaacaactagaggaagaataactggaataggtacagatactgcggtgttgaatgctcaaggttatggagaaataatgattggagagcttttaacagcaacgacaacgattacaaatatcactaatttacgtaaagggcagtattttacgctaagtaattatcaaactaatcatgcattaaatataaaatcttcgaaagatggaattaatggtattgttttaaaaaatagacgagatgcaactctttccaaattctctgacactattttgttctatgtaactcagttaggaaaaattgtagaagtagggcgtaatttcaatgaagaagtcatgttaggtatttcttcatcaccatcttttgtgggtcaggtagcagtggaaaaaggagcagcttatattgctattggtaacgagtcgaagttacactggaaaaaaataacaaactaa

SEQ ID NO: 25 - DNA, 1320 bp, Peribacillus Aracenensis
  source 1..1320: mol_type = genomic DNA
atgaaagtttctgttgctggtactggttatgttggtctggttactgctgtatgtcttgctgaaaagggtaataaagtaacttgtgtcgatatagatgaacaaaaaataaaattattaaatagcggtatatctcctatttttgaaccagaacttgaagaattaatgaggaataatagggataggattaactatgtaattgattataaagaagcgtatagtgatgctgatgtaataattattgctgtaggaacaccagaaaaaaaagatggttctgccaatcttcaatatatctatgaagttgctaaagaggtggcgaatacattaataaaagattgtgttgtggtaattaaatcaactgtacctataggaactaatgataagattgaaaaattaataaaagaaaatctaaaatatgatgttaatgtggatgtagtttcaaatcctgaatttctagcacaaggtactgctgttaaggataccttgcatgcgacaagaattgttctaggagtagagtctgaaaatgcagagaaaataatgagggaagtttatagtgaatttaatattccttttgtgatagctgatcgaaaaagtgcagaaatgataaaatatgcagccaatgattttttagcattaaagatttcatatatcaatgaaattgcgaacttatgtgagattgtcggggccaatatcgaagatgttactaaaggaatgggattggatccgagaataggggaacaatttttaaatgcaggtattggttatgggggttcttgctttcctaaagatacaaaagcgttacattggctagcaaggtataatgattatgagattaaaacaatcaaagcaacaatagaggtaaatgaaaatcaaaaaattaaattggttaagaaagctagaaagtattttaatagttttaatggacttaatgttgcagtccttggacttacttttaaaccaggaacagatgatttaagagaggcaccatctcttgataatatccctatactcctaaatgatggggcgaaagttaatgtctgggatccagtagggatggagaatttcaaaaaagttttctcaaataatgttgcatatagtgagtcaatagaagaggctataactaatgctgatttatgtttgatttttactgaatggccggaaattaaagatttcgatatagacaaatataaaaaattaatgaaaagacctttggttattgatggaaggaattgttatagtattagagacgcacaaaaatcggggataatatatgattcaataggtaggaaaacaacagaaaaagaaatattaatgaaagtataa

SEQ ID NO: 26 - DNA, 1338 bp, Peribacillus Aracenensis
  source 1..1338: mol_type = genomic DNA
atgaaaaatgtgtatgcttttctaaagagaaaaatatttagtaatgaggtagcatctaagacaattaaaaattctagttggttagttagtgataaaatatttacgatgttaattgggttatttattaccgcaataattgccaggtattttggacctgaagattttggacagttcaattacgctctagcatttgtctcattatttacagcgctatctacattaggattagagacattaactgtaaaaaaaataatagataaagatattgatgaaggcaccattctttgcacgagtcttattctaagagttacaggtgggctaacattaacaactctagctacaatggtaattatgcttattgaaccaaacagcaaaaatcttcacatggtagtcataattatgtctttaaccatggtattcaaatcttgtgaagtaattgagtattggttacaaacgtatcaaaaagcaaaagtttcttctattattcgaatgtcagtatatattattatagcggctttaaagatcgcgttagtttttttctcagggaatttaattcactatgctttaatctatttattagattctatcctaatcggtttttctctaataatagcgtattttagaattagaaaaaataaatttccatggcgatttagcttaaagtatactaaaagcattttatcccaaagttggtatttaatactatcaggattaatgataacactatatatgagaatcgatcaggttatgttaggttttatgctaccaaataaaagcgaagcgggtatttattctgcagctgttagagtagctgaaatgtggtactttgttcctatggctattataacttcgtttaaccctataattatgagtaagaagagaaataatgaaaatagttttcttcattcaattcaacttttatttacattagtagcatgggtatgtatagggtttggtttattaattttaatattttctgagattattataagtctcttatatggacatgaatttattaaagcatcaggtattttaactatcagtgtttgggctggtacgtttgcgttgttaggttcagcgagatcaacttggttaattagtgagggcttacagaaatatacattagtctttacttttgcaggttgtattactaatattactttaaattattggttaatacccactcatggtggttttggagctgcttgtgcaactcttatatctcaaatcgttggagtatttattattcctgtattttttaataaaactagaatgtctactattatgatgataaaagcatttaatataaggcgagtattcaattatattaagcaataa

SEQ ID NO: 27 - DNA, 1164 bp, Peribacillus Aracenensis
  source 1..1164: mol_type = genomic DNA
atgaatattcctattatagtagttgcatacaatagagatctttctcttaaaagacttttaaattctctggcaagggccgagtatgggaaccaaaaagttgatttgataattagtattgataaaagtcagaatgaaaaagtctcagaagtagctcgagatttcatttggaaatacggagaaaaaacagttatagagcataaagagaatttaggcttaaaaaagcatgttttaaaatgtggagactttgcgattgatagggacgcaataatcatgcttgaggatgacttgtatgtttcagaatcgttttataaatttgctactcaagctgtgaatttttatgaagaagataatgatattgctggaatttcattatatacatacagagtcacagattttgctgatcaaagaacctttactccactacaagatcaaaatgatgtcttttttatgaatgtcccatcatcctggggacaaatatggaccaaaaaccaatggaaatcttttaaaaaatggtatgaggaaaataaatacgaattaatagattataggaatctgcttcctgaacaagtgcttaattggggcgattcttcatggaaaaaattcttctatatgtatattactagtgaaaaaaaatatattgtttatcctagaattgctttaagtactaatatgggtgagagtggaactcataatgttgttaattcaaccacttatcaatctttattaatgggtggctttacaagagactatatttttgtagatgtaaatgaatcgaaaactaagtatgattctttttttgaaagcgagaatatagtttctttgttaaacgatcaagttactatagattattacggactaaaacaaaaattcataaaaacaggctatttacttactactgcaaaacttaattataaaattgttagaaaatggagtttgtcattagtgccgtatgaattaaatataattaataatatcgaaggaaatgatatatttctttacgatctttcaaaaaaaacagaggggaataaaaaggttaagaaaatcagtacacaaacaattaagtatgaactaccgggaattacgaagaagaaagctttaaatataacatacacagagtattatgccgcctttataagaagaatgaacaaaatgttaaaaaaataa

SEQ ID NO: 28 - DNA, 1218 bp, Peribacillus Aracenensis
  source 1..1218: mol_type = genomic DNA
atgagtaattcaaagctactaaataaattcttagtaatttttatatttatagatatattattactgcctaactttaaatattttgttatgccaatatctttgcctttagttttgtgggtaattttcacaaaaagagtaaccattcaaaaggatagagagtttttattatttttaatactatctattttggtattagtgagtgtatgcctatcttttttacaagtacctaattaccttgcaaacgggttgaatgtatggttagaaaatataaaaagagcatttcaattgattacatcgtttgcatactattttctaattcgagattacttaaataaatatcctgttaaaattaaaaatattttacttttgtttgtttttttctatgttatcttaggaataatttcaatgttaaatattggggtttattttgggataaaagaatttttaggtataagggatccttttatgaatccgttttttgttaataataatgattatttatttagatatagttacttatttattgatcctaataattctgcatatttatttcagatggttactttttatttacttcttaatgaaaaacttaatataacagagaaacttttaattttcctaagtataattttctctcttatattaagtatgagtactggtgccgtgctatcattaatagtctttgtttttctttctataatcttaagaatccgagaattacctaagattagaattacgtataaaaaattaataacaacaataataaccccttttatactgataataatattttattttgcgaaatttcttttagaaaattacttgaatcatatagcgaattatagtatggatagaatgttaggaaatacagacggtggtaggttaaataaatatggatatatgtttgggaatagtattccaaatttaattggggaaggttatacattaattagagatagtgttatttttagacctcatagtgaccagttaaggtttttatactcatatggtatcgttgcatatttaattgcaatctggttcttttttcgaggattgttatttaatgcaaaatatttatttttaatacctgctttttttgcgttttctattaattcactaattgatgaacaaaaattattgatatccttattaatattattagcttatttaaagactattcatttaataaaaaggcaaaacaagcaagaaggagtgtaa

SEQ ID NO: 29 - DNA, 1227 bp, Peribacillus Aracenensis
  source 1..1227: mol_type = genomic DNA
atgaaaattttatactttgggagtgtttgtgatgaagaatggtttgatacagtttctagtaaaaaaagcatgccatcacaggttgcccaatatatgtttgaaaaagctctagtaagtggcttttcgaatattgaaaatatcgatatgaatatctattatttgtaccaagagccatattacccaaaaggaacatatttaagatttaagaaaagaataaagaaattaaacaacaaatatatagtgagctatttatctaatataaatttgccgtttattaaagaaattttttctttttttcaaggattaacattgacaatgatttggggattaaaaaatcgaaataatgatcaaaaagtaattttaactccatttaactatacacctttatccttaggtatatacctagcttcaaaagtttttcgaataaaacgtgttaatattttcactgatctatcaagtgatatattgagcttaaaaagacaaaaggacatgccgaggtttaaaaaatttctattaccttattatataaagttagttgattttatagagcataactatgatggctatgttttattcactgaaccaatgaatagcagggtgaacccgttaggtaaaccctatatagttatggaaggaattttcaataatgatttagttttatccaatgtagccaagagaaggtcgattatgtatgctggaactttggcttttgaatatggagtaaaaaatattatagatgcttttgaagagattaaagatgatgaattagaactctggctttttggggatggagatatgaaagaatatataaacgagctgtgcaaaagggacaaaagagttcacttctttggatttctacctcgagaacaagtatttgagtatgaaaagaaggcaactttacttgtaaatattagagatcctaaagataaatataccatgtactcttttccttctaagacttttgaatatatggtatcgggtactccatttcttacgactaaattaatgggtatccctgaagaatattataaattcatgtatacaattgatagtatagatataaatactttgaaaagtaagatagaggaaattctgtctacaccacaaagtacattgaatgaattaggtttggaagcaaggcaatttgttattaaaaataaaaatagtaacacccaaaccttaaaaattaatacattaatggaaaaaatatcgagtgaaagcatctaa

SEQ ID NO: 30 - DNA, 1077 bp, Peribacillus Aracenensis
  source 1..1077: mol_type = genomic DNA
atgaatattatggtttttgatgttccagctgaaaaaggtggtgcgctctctgttttaaatgatttttacgatgaagttgttgagagtgagcattcaaacattaattggatatttgtattaagtaacccaatattgaatgagacggaaaatattagagttctaaggtttccatggataaagaaaagttgggggcatcgactttattttgatcaagtcgttgcacctaatttggtgaaaaaatataaagtggataaggtattttcccttcaaaatattacaattcctcgtgtgaattgtgaacaaatcctatatgtacatcaacctttaccttttgtcgattataaattttctttcaaagataatagacttttttgggtatatcaaaatattataggtaaaaatataataaattcaataaacaaatcacagagggttatagttcaaacggaatggatgcgacaagctgtaatagaaaaatccaaagtagatagccgcaaggttgaaattattccgcctataattaatttagaagttaaaaagtactttggaccaaataataagtcattatcaactttcttttatcctgcgagtggcgccgagtataaaaaccaccaagtaatcgtagatgcaagtaaaaaattgaaaaagttaggcaagataaatcatgaagtaatattcacacttaacggagatgaaaataatcacataaaaaatttatatagactagtgcataaagaacagctacccattcgttttgaaggaaataaaacaagaaatgaagtttttgacttatacactaaatctatattaatttttccatcttatatagaaacctttggattaccgatgcttgaagcaagaattcataaaggaatcattcttgctgcagaaacaccttttgctcgagaaatattaagaggatatgaaaacgcaaaatattttgaagcatctaattcagaggaactatgcgtattaatgcaacaatatataaataaaaaggtactctataaacctctacttgaagtacaacaaaatgaaattaagcatgagagaaaattaataacgcttctaacttaa

SEQ ID NO: 31 - DNA, 1128 bp, Peribacillus Aracenensis
  source 1..1128: mol_type = genomic DNA
atgaaaaaattaaaagtaatgacagtcgttggcactaggcctgagattataagattatctgctgttattaataaattagaagagtcagatgcggtagagcatatacttgttcatacgggtcaaaattatgattatgaattaaatgaagtgttttttaatgattttaaacttaaaaaacctaattatttccttgatgctgcaaacggaacagcagtagaaactatcgggaatattttgattagaattgatcctattatggaagaagtaaaaccagatgctcttttggtattaggtgatactaatagctgcttatgtgctattgcagctaagagaagacatattcctattttccatatggaagcaggcaacagatgctttgatcaaagagtaccagaagaaactaatagaaaaattgtcgatcatacagctgatattaatttaacctatagtgacattgcaagagaatatttattaagagagggactacctgccgatagaataataaaaactggaagtccaatgtttgaagtcctcaattcaagaaaaggtgacattgaagaatcagatgtattagagaggctaaatcttactgagggaaattattttgtagtgtcagctcatagggaagaaaatattaattcagaaactaatttcatgaatttagtagatagtttaaatgccgttgcagaaaaatataatatgcctgtaattgtaagtacccatcctaggacaagaaatatgatcaatgctaaaggaatagagtttaatcctctagtaaaaacgatgaaacctttagggtttaatgattatgtgaagcttcaaactaaagctaaagcggttcttagtgatagcggaacaattagcgaagaatcttctattcttggatttaaagcactcaatattagacaagctcatgagagacctgaagcaatggaagaagcatcggtaatgatggttggtttaaaaaaggaaagaatattacaggggctagagatattgaagacacaagaaaaagatacactgagacttgttggtgattatagtatgccgaatgtatctgataaggttttaaggattatactgtcctatatggattatgtgaatagggttgtttgggggaagggctaa

SEQ ID NO: 32 - DNA, 1110 bp, Peribacillus Aracenensis
  source 1..1110: mol_type = genomic DNA
gtgaaaatactcgttacaggtgcaaatggatttgttggaaaaaatttaattgcagaattacaaaataaaggatatgaagatattcttaaggttactagagaaacggaaccatctttattagatacttatacaaaagaatgtgattttgtttttcatttggcgggagtaaaccgtcctgatgatgaaaaggaatttatgcaaggtaatttccacttcactcttggattactagagctattaaaaaaacataataataaatcacctgtacttattacttcgtctatacaggcagataaagataatccatatggcaaaagtaaaaaagcaggtgaggacgttctgtttgaatatagtcatcaaacaggagcagaggcatatgtatacagactccctaatttatttggaaagtggagtaaacctaactacaatacggttgtagcaacgttttgttataatattgctagaagttcagaaatccaaattaataatcaagatgccgaattaacactctgttatattgatgatgttctagaagagtttataaaagctttagagggaaatccgactaaaaagaatcaatattgctttgtgaaaacaacacatactattaaattaggggatttagctgaacgtataaaaagctttaaagaaagtagattagaattaagcattcctaatatggaagacgccttaacgaaaaagctttacagtacatatttaagctttttaccagaagacaacttttcttatgatttaaaaatgaattgtgatcatagaggttcttttacagagtttataagaactcctgaaagaggacaagtgtcagtaaatgtatcaaaacctggcattaccaaaggaaatcactggcatcatactaaaaatgaaaagtttttagtagtaagtggtgaaggacttattagatttagaaagatagattcagatgaaattattgaatatagagttagcggcgaaaagttacaagttgtagatatacctactggatatacacattccattgtaaatgtaggagaatgtgatcttgtaacagttatgtgggttaatgaatgttttgatccagaaaaacctgatacttacttcttggaggtataa

SEQ ID NO: 33 - DNA, 1032 bp, Peribacillus Aracenensis
  source 1..1032: mol_type = genomic DNA
atgtttaagaataaaactttattaataacaggtggtactggttcatttggaaatgcagttatggagaggttcttggatagtgatattaaagaaattcgaatcttttcacgtgacgaaaaaaagcaagatgatatgcggaagttatatagaaatgaaaaattgaagttttatattggtgacgttagagatcttgcaagtgttaaaaatgcaatgcacggagtagattatgtttttcatgcggctgctcttaaacaagttccttcttgcgaattcttcccactagaagctgtaaaaactaatattttagggacagataatgtgttaacagcagctatagattatgaagtcaaaaaggtcatttgtctttcgactgataaagcagcctatccaattaatgcaatggggatttcaaaagccatgatggaaaaagtttttgttgctaaagcaaaaactgtcgatccagaaagaacacttatttgtggaactaggtatggtaatgtaatggcatctcgtggatctgtcataccattatttattgaacaaatcaaaagtggtaagccactaaccattaccgatcctaatatgactaggtatctcatgagtcttgaagaagcagtcgagctagttatatttgccttccaaaatgcagtcgctggtgacattatggtacaaaaagcacctgcaagttatattggagatttagcacaagctattaaagaattatttaaggcagataatgagattaaggttatcggtacaagacatggagaaaaattatatgaaacccttcttacgagagaagaatatgtagttgcagaggatttaggtggtttcttccgggtttcagcagataaaagagatttaaattatgataaatattttgctgaaggagataaaaagttatctactgaagaagaatataactctcacaatacgcaaatcttaagtatagaacagattaaagaaaaactactagaattagagtatgttcaaaatgaactcaagtatatgaaggtactttcttcaaaataa

SEQ ID NO: 34 - DNA, 1212 bp, Peribacillus Aracenensis
  source 1..1212: mol_type = genomic DNA
gtgaatgtattatttttaacacttttagatttttcaacaattgaagaaagtggtatttacactgatttattacgagaatttgttaaagatcagcataatgtttttattatttctcccacagaaaagaggaagcaaaaaacaactaggttgattgataagggaaattataaaatacttaaattgcagattggtaacattcaaaaaacaaatatgattgaaaaaggcatatcaactcttactttggaatcaaattttttaaggggtattaaaaattatttttcaaatgttaaatttgatttagtaatttattcaaccccgccaataacactccaaaaagctgttgaatatgtaaaaatgagagataatgcaaaagcatatctattgttaaaagacattttcccacagaatgccgtagatcttggcatgataaagaaaacagggattataggttttttatacagttatttccgatataaagaaaagagattatataaaatatcggattatattggttgcatgtctcaagcaaatgttgattttttattgaaacacaatcctgaaatacccccaaatattgttgaaatatgtcctaatagcatagagccaatgaataacaaaaaagatgaggaattaatagttgagataaaaaagaaatatagcatacctctgggtaagaccacttttatttatggtggaaatattgggagaccacaggggattgactttttgattgagtgtttggcggctaacaaagctaatgacaaggtttattttgttatagttggatcgggtacagagtataataagcttaaaactttttttgacaatgaaaaaccgagtaatgcccttttattttctcagttaccaaaagtggaatatgaagttctagctaattcgtgcgatgttggattaatttttcttgataatcgatttacaataccaaatttcccatctagacttctttcctatatgcaggcttcaatgcctgtcctagcagctactgatgtaaacactgatatcggagaaattgttgaacatggtgaatttggattttggtgtgaaagtagtaatgttgagcaattcaataaaaaagtacaccagttatgtgataatgaattaagaatacagatgggattaaacgctagaaggtacttagaagataattatacagccaagcactcttacgaaataattatgaatcatattaaataa

SEQ ID NO: 35 - DNA, 618 bp, Peribacillus Aracenensis
  source 1..618: mol_type = genomic DNA
atgaaaaataaactccttataatcggtgccagtgggcacgggaaagttgttgctgatattgcgttgaagatgaataaatggtcgaacattgcttttttagatgacaacgaaaatattaagtcatcaatggggataaaagtgattggtaaatcaactgatgtatttaagcacatacaagattacgatatctttgtaggtattggtaataattccacacgagaaaaggtgtatgggaaacttgaagcaaagagagtaaacatccccacattgattcatccaactgctgttatcggggaaaaagttgagttggcacccggtacagtcgtgatggctggagtagtggttaattgctgcacaagaatcggaaagggatgcattatcaatacaggggcttcgatagatcatgacaatataattgaagattttgttcatatatcaccaggttctcacttagctggtacggttaaagttgagcatggttcttggttaggtattggcagcatagtaagtaataatgtaaacattactagtgggtgtgaatttggagctggtgcagtagttattaatgatataactgaacccggtacttatgtaggggtaccggtgaggagagtttag

SEQ ID NO: 36 - DNA, 648 bp, Peribacillus Aracenensis
  source 1..648: mol_type = genomic DNA
atgaaaccttctaagggtggtatttatagaagatttggaaagagagcgatggatttcatactatctttgctagcaattataacttttagtccgatcatcttgggtgttgctttgcttgtaagaataaagcttggtagtccagtgttgtttaaacaaaaaaggccaggacttaatgagaatgtttttatgatgtataagtttagaacaatgactgatgagagagatgaaaacggagagttactttctgataatattaggttgacgaagtttgggagattcttacgttctacatcgcttgatgaacttccagaactttttaatattatcaaaggggatatgtccattgtaggacctagaccattgttggtgcaatatctgcctctttataataagcatcaaaaacggcgtcatgaagtaagaccaggattgtctggtttggcgcaggttaatggtagaaattctattaattgggaaagtaaatttaatcttgatgtggaatatgtggaaaatgtaagcttcagtggagactggaagattatttttcaaactattaaaaaggtctttgtcagggaaggcataaattcagaagctgctgcaacgatggagccatttaatgggtccaataaaaaggaaagaatagaattatga

SEQ ID NO: 37 - DNA, 1116 bp, Peribacillus Aracenensis
  source 1..1116: mol_type = genomic DNA
atgaaggatcgattatttctatcatcaccacatatgagtgatgaaggttatgaaatggattatataaaggaagcttttgatacgaattggattgcgcctcttggggaaaacgtgaatcaatttgaaatagaattagcaaataaggtaggaagtaaagctgctgcagcactatcttcaggcacaggcgcaatccatttagctcttaaagcagcaggagttaaagaaggggatattgtgttttgtcctacattaacattctcagcaactgtcaacccggtaatttatcaaaatgctattcctgtttttatagatagtgattatgagacttggaatatgtgtcctaaagctttggaagaagcttttgagaaatatcctgaagtgaaggccgtaattatagtgcatctttatggactttctgcagatatggataagatcatggagatttgcaataagcataaggtagcagtaatagaagatgctgctgaaagcttaggtacttattataaagaaaaacatactggaaccattggtgattatggtattttctcttttaatgggaataagattatcactacttctggcggtgggatgctagtttcaaataatgaagagcgtattgctaagacaagattttgggcgactcagagtagagaccaagcgaggcactatcagcatagcgaattaggatttaattaccggatgagcaatgtagttgctgggattggtagagggcagcttaaggtattagatcaaagagttgagaagaaaaattatatctttgatttttataaaagagaacttagttcacttgacggtgtagagttcatgcctagtaatgagtggaataaaccaaattactggttaagttctatgactttgaatggtatggttagaccgatagatataatggaagctcttgaaaaagagaacatagagtcaagaccaatttggaagccgatgcatatgcagccgttttttgagaagtatgactttgtcggaacgggtgtttcggaaaagctgtttgagaatggtgtttgtttaccctctgatacaaagttaacggataaggatttggaaagagttgttgaaattattaaagggttgtgggaaaggtaa

SEQ ID NO: 38 - DNA, 894 bp, Peribacillus Aracenensis
  source 1..894: mol_type = genomic DNA
gtgaaaaaaatcacaaaagcaatcattcctgcagcaggattgggcactcgttttttgcctgccacaaaagctatgccaaaggagatgctgccaatcgttgataaaccaacgattcagtacatagtggaggaagccgttgcatcaggaataaaagacataataatcgtaactggaaaaggcaaacgtgcgattgaggaccattttgattacgctccggagctcgaacaaaatctattggaaaaaggaaaagtagagttgctcaaaaaggtacaatactcctctaaacttgctaatatccattacattagacagaaggagccaaaaggattgggtcacgctgtatggtgtgcacgtaaatttattggggacgagccatttgccgttcttttaggggatgatattgtccagagtgaaacgccttgcttaaagcagttgattaatcagtttgaggaaaaaaacaattcaattatcggagttcaaaccgtacctaatgaagaaaccaatcgctatgggataattgaccctgcttttcaaaatggacgactatttcaagttaataactttgtagaaaaaccagcattaggaacagcgccttccaatttggccataatgggaagatatatcctaactcctgaaatcttcagtatgcttgaacagcaggaagctggtgcaggcggggaaattcagttaaccgatgcgattcaacagttaaaccaagtacaacaagtttttgcctatgattttgaaggaaaacgatatgatgttggggagaaattggggtttgtaaaaacgacattaaagtttgcccttcagaatgaagatattaaagatgagttagtagagtttttagaacaaatggttaaggatatttccgcagaaaagattaatgcatag

SEQ ID NO: 39 - DNA, 1821 bp, Peribacillus Aracenensis
  source 1..1821: mol_type = genomic DNA
ttggcctaccgaaaacgattaacacttctggccctattagattcattaatagtattatcggccatttatgtaagttatttattcttgtatccctatttggaaatatttaaattaccaacactcttagtcacatcagtctccctattaatcagccatcatttttttgcttctatttataaactgtataagaaggcatgggagtatgcaagtataagagagttactgtccattattaaagccgtaagcttatcggttatcacagttatcgccatccagttaatggtttttcaagatgtttatgtaagagccatggcattgacctggatgatgcatgtcatccttattggcggttcgcgattttcttggagaatgctacgtgaccgtttgataaataatcaaaaggaaaccagaaacacattggtgatcggtgcgggatctgctgggaccatggttgtacgtcaacttcttaataatcatgatacagaacttaagccagtagcattcattgatgatgatccgaaaaaagataagctagacatattaggaatacccgttgtcggtaactcaaaaaatatccctgaaatggtgaggaaatataatatagataatattgtcattgcgataccttcattaagtaaaaaagaattgaaggtcatatttgatgaatgtgtgaaaactaatgctaaaacacaaatcatgccgatgattgaagatattatattaggtaaagtagctgttaatcagtttaaagaagtggaagtggaagatcttttaggaagagaacccgttgaattggatataacaagtatatcggaatatgtaacaggcaagaccatcctagttacagggtctggtggctcaattggttccgagatttgccgccaaatatgcagattctcacctaggaaacttatcctcctagggcatggagaaaatagcatttatcagattgagatggaactgaaaaagctatatgccgatcaaattgagctcatacctatcatcgcagatattcaagatcgtgatagaatttttgaagtaatggaaacctaccgacctgatgttgtataccatgcggctgcacacaaacatgttccactaatggaatacaatccacgtgaagctgttaagaataacgtttttggtacaaagaatgttgcagaagcatcagatacctttggtgtaggtgcgtttgtgatgatttcgtctgataaagccgttaacccaacaaacgttatgggatcgacgaagcgaattgctgaaatgattatccagcagttagcgaaaaatagcacaacaaaatttgttgcggttcgttttggaaatgttttaggcagcagaggaagtgtcattcctttatttaagaaacaaattcaagccggtggaccagtaacggtcacacatccagatatgacaaggtattttatgactataccagaagcatccagattagtcattcaggcaagttctttggcaagaggtggagaaattttcgttcttgatatgggtgaacctgttaagattgttgaattagcgacaaaccttatccagttatcaggttattccatagacgaaattggaatcgaatattcaggaatccgtcctggtgagaaaatgtatgaagaattattaggggagaaagaggtacatagtgaagcagtgttccctaaaatctttatcggaaaagcggtactggaacaggaagaggaaatacagtatcttttaaactcttatgatgatttttccatatcagaacttaaagaatttgtaataaatttagcaaatcgaagaaagaacaaagctttctcagcagtgaaatag

SEQ ID NO: 40 - DNA, 765 bp, Peribacillus Aracenensis
  source 1..765: mol_type = genomic DNA
ttgatcgatatacattgtcacattctcccaggaatggatgatggatctgcggacatgaaggaaagcttgaatatggcaagaaaagcggtagaagcaggaatcacccatttatttgccacgccccatcacttaaacgagaaatatgtaaatgttaaaagtaacatcattgaccgtgcagtgagattaaatgaaagtttacaagaagcaaatattcctcttaccattcatctcggacaagaagtaagaatacaccgagacatatttacatcacttgaaaaggaagaaattctaacactggacgataacggtacgtatatactgttagagctcccgtcgggaaaggttcctacatatacactagaagtgatatatgagctgctgcttaaaggaataacaccaattatcgtacatccggagagaaataaggaattgatagcgaatcataaactattatttgaattggttcaggagggcgcgttaactcaaattacctctggcagtatcatcgggaacttcggtaaaagtattcaatcattttcaaaaaagataatcaaacataatctagctcatttcattgcaacagatgcacacaatataggatctagagggttcacgttacagcaagcctatgaaaccatcacaaagacttacggaattcagcgtacttattactttaaagaaaatgctgaacagttattaaatgaccaaagtcctactattgaaaaaccattgccattcaaaaagaaaattttagggattttttag

SEQ ID NO: 41 - DNA, 678 bp, Peribacillus Aracenensis
  source 1..678: mol_type = genomic DNA
ttgagaagtaaagataaaaaacaggtgaacttgattgcacaaactaaccctaaatcacctatcactgaacaatatcgattaataagaactaacattcaattttcctcagtggataaagacatacaaaccatcgtggtaacttcttcggagcctaatgatgggaaatcgacaacagctgccaatctcgctattgtgctggcacaggaggaaaaaaaagttgtgcttgtagatgcagacttaaggaaaccatcggttcattatgcttttagtcttagtaatatagagggacttacaagtgtgcttacgaagaaaatgagtatagaaaaagcactcatgaaaacgaatgtgcctaatctggaaattctgacaagtggaccaataccacctaacccttcggaattattgaattccaaagcgatagaaacagcgattgaagaattaaaagtaatgtatgattatatcatttttgacacaccacctgttttggtagtgccggattcccagattgtagctaataaatgtgatggcgtaatcatggtagtatctagcggcaagacaaacaaacagagtgcagtaaaagcaaaggagcttttagtgaaagctaatacatccctgcttggagtcgtattgaatggcgttgaaacggataacagcaattattattactatcaatcttaa

SEQ ID NO: 42 - DNA, 690 bp, Peribacillus Aracenensis
  source 1..690: mol_type = genomic DNA
atggaagaaactattagtattgcagatatttttaaaacattaaagaaacgttggaagctaatcatgctactgacattaattgccgctttgattagtggaacgatttcttatttctttttaacacccgtttaccaatcttcaacacaaatcttggttaatcagaagcaatcggagaaccaattggactcgaatcaaatacgatctaatatcgacatgatcaatacatacagcgtaatcataaaaagccctgccattttggagaaagtcattgatgagctagaactagatcaaagcgtagaacaattaagtgaaaaaatcacgatcaacagccaagaaaattcacaagtcttttcattaacggttcaagatagtaatccgtcacaggctgtagaaatagcaaacacggtttctggaactttccaaaaagaaatcaaggatataatgaacgtcgacaatgtcagcgtattagccaaagctgaaattaaggtgaatcctatagctgtaaaacctaatccactattgaatatagcaattgcaatcgtagttggattgatggctggtataggcttggcgttcctattggagtttatggacaatacgatcaaggacgaggatgatattgaaagaatcttagaattacctatacttggatcgattcaaaagattaaacaggtaaataataaaggataa

SEQ ID NO: 43 - DNA, 300 bp, Peribacillus Aracenensis
  source 1..300: mol_type = genomic DNA
atgataggttaccgtgttaagtcgcttagggaagaaaggaaaatgtcaattagtgaactctccgcaagatccggcgttgccaaatcctatataagctcactggaaagaaaccttcaaacaaaccctactatattagttttggaaaagatcgctagaatcctttgtattaaggtcgatgctctgttgaatgaacaagcagacaatagcattgatgaagagtggatggaaatcatgcaggatgttatgggatcaggaatatcgaaagaggaaatgcgcgaatttattcaagatagaaagtga

SEQ ID NO: 44 - DNA, 120 bp, Peribacillus Aracenensis
  source 1..120: mol_type = genomic DNA
atgttttgtttgaattattttgattatattcaagcttcagagaatatcatcaaaacgaataattggacttatatgaatagtaatgaagaaatagagaaaaagctaagtacaagaatatga

SEQ ID NO: 45 - DNA, 2067 bp, Peribacillus Aracenensis
  source 1..2067: mol_type = genomic DNA
atgtttaagaactttgatatcgcggtggatacaaaaaaagtaatcagaaatcgtgcaatcactgtcaacaccaatgatttacagactgttaaattttctataactatcacccaatcaggggaaccggtctatttaacaggatctactgttcgtttggctgttaaaaagccggataaaaagaccgtattacaagattgtgcaattatagatgcagcaaacggaaaatgcgaaattatcttggatacgccagcatatatcgactatggtcttcatcatgctgaagtaatgatttattatgcagcagataaggtatctgttacaagtaggttttcatatacggttaacaaagggattctcgatgaagggacattcgaatgtactcatgaatttcaatccaatacaaaatctattgcggacgttgatggtattgttgctgatttaaggtataagggaacaggaattgacgatcaagcacaatccgaattggaagccaaagctgtacagtcagcttatattgctaataagaatgaggtaagcataactgattttgaaagtgaaaaagttggtgatgattggtatccagcatttcaagcagcattgacttctataggtaatacagggagcataaaatttcctggaaaggtaacgtacagcgtgtattctcctttggttcttccattaacagggcatagaataaggatattttcaaacgatggagctaccattttggtaaaacataacggagacggcattgtgctaaatgcccaaaacgagaattactcgtcccatattattgagggtcttggtattcaaggaaccaacacatcttatccatcagatgggtatataccaccaagtacaggagcaggtattcgcatgaattcagcatattattgcacattgcgtgatgttcgtgtttcagggtttcaatatggaattcaccttaaactcgcaataaaaaataattttgaaggaaacacttacattcgacataatcaatatggaatttattttgatgggggtgcaacaaatgtaaacaactttgatggtattggtatacgtgagaatagaaaagctggagtttatttcaacgttggtcattctccttttcctacacataatacattcactgattgtttaatcgagtcaaacattcctttcccttatattacaggaggaaacgctccaaatgatagtataggtgtttatttaggcggggcatattataacatttttgacaattgttactttgaaaatcaacagtatgcagtttatttaactggtagttcagacgggaacaaatttagtaaatgtagattttcaccaagtgcggatttgacaagactggacaaagttatgtttgatggtgctggtgtaagtaataacacatttaccgaatgcttctcattatcacaagataatacctctgctaatgttgaatcaaataatgctacccaattctataatcagtttgttaattgtgaaggatttacctttatacctgctagtattttagctcctatagatgtgattaatcttcgtccaaatcaagcaggttggggaactccattcggggcgttaattattccttctcatggttattataataatcccggagagggagcaactaggggaagaataactggaataggtactgcaaacgcaactctaaatgccgatggttatggtgaacttatgcttggttcattaataaccgcagccacaacgatcacgaatattactaatttgaaaaaaggtcaatatttcactttaagcaactatcagattagatttcctgttactttaaaatcttcaacggatgggattaacggcttggttttgaaaaatttacgagacgcagttctcataagacgttctgacacaatattattctacgtgacacaattaggaaaaattgttgaggttgggcgtaattttaatgaaggagtaataaatcttgtttcatcttcaccttcgtatataggtcaattggctattgtaggtggagttggctatattgcagttgggacttcttcggtatctgattggaaacaaataacaaattga

SEQ ID NO: 46 - DNA, 408 bp, Peribacillus Aracenensis
  source 1..408: mol_type = genomic DNA
atgagtttagcaagttatatcggatgcaatatagaaatacctcttagtaatgaagagtcagacgatttaattgttattggaggttgtttttcgaacaaatataaccgtcgagatgtgaaaaaacatcaatttaccactccttttgttttcgaagtatcaagtgactggggaatagagatttcggaatatatgaaccaaaaaacgtgtgccgaatcaaaagagaagctaattgaactgtgtaaaattatggacagttacattgataaaggtgattattttgaactgtatagttgttgggtcggagaagaagccgataagcgagaaggtgagataactcttcgaatcaataactttgacattgaacagatagaaatgcctgaaaaaacgttagtgagatttgagaaatga

SEQ ID NO: 47 - DNA, 468 bp, Peribacillus Aracenensis
  source 1..468: mol_type = genomic DNA
ttgaagaaagttttcactgtattatttataatgatggttttaacagcttgttcatttaccaacagtaaggaaacacaatcagaaacgaggaccgaacataattatcaatttataggaaatagcgaacattgggaagctgaatattcttatgaagcaaccgaaatatggagggaaaatgaacgcaaacaaacaggtcattctagtaaagatagctatgaacttgtattaaaatacaaaggatctttagaagagttatcttccatgaaaaacctcgaatacagttttgaaacaaccagtcaaagcgcaagtacaaaagaacaattccctgaaccacctagcgaaaaagtatttagaacgggtggaggttcagaaggtggagcaataataggtgaaggcgaagttataaaggtaaatgtaaaatgggatgattctgaagagtcatttgaactgcacaataaggataagtaa

SEQ ID NO: 48 - DNA, 267 bp, Peribacillus Aracenensis
  source 1..267: mol_type = genomic DNA
gtgaaaaaaagatggggtctttggtggactggtaacatattttggattatcgtttttgtgataggggcagctattacttggctaagaaaggttgatggcgctggtgttacacaaacccctgagcttaaatcagtggcattcatagttttattgattgcgtttataattccaataattattcaagttgtatggctaattgttaatttgagaatttccagtaacaaagatcaaacatatcttaaaggtgaagacatagttaagagatag

SEQ ID NO: 49 - DNA, 201 bp, Peribacillus Aracenensis
  source 1..201: mol_type = genomic DNA
atgtatatgaaagaatttggaccgacaatagttatcgattatgcacacactgcggaagccattcaacatatgcttcaaatcgccaaagaatgcggggtcaaaagatttatcatatctttggtttccaaggtggacgagatacaaccaaaagggctgaaatggttaaagtatcatcggaacatagtgatgtttcgattttga

SEQ ID NO: 50 - DNA, 225 bp, Peribacillus Aracenensis
  source 1..225: mol_type = genomic DNA
atgaaaaaaggtgttggtgctggaccaggtgatcccgacttaattactgtcatggcaaccaaatgccacgcggaagcggatgtcatcttgtatgatcgattgtataatcgtgaattgttttatgcggtaaacctgaagctgaatacatttattgcggtaaagcgcctggtaaacattgtgtctctcaagaggagattcatcaattgtttattagtaaatcaatag

SEQ ID NO: 51 - DNA, 147 bp, Peribacillus Aracenensis
  source 1..147: mol_type = genomic DNA
atgaaaggaatatatactaacaaggatatttatcaatttgataatgtcttaacagagaatttagaatcaatcacaataatctatatgaaagaagtaaagaagctttttaataaaaaaactttaaatggtaaatttgtgaaagaatga

SEQ ID NO: 52 - DNA, 576 bp, Peribacillus Aracenensis
  source 1..576: mol_type = genomic DNA
atggaagtctggttagattgcaggttgctgcttggactaactaacttagagaaagaaaatgtattagaaatgactgaagttgaattggtatcgatatgcgaaggcattttaaaacaacttaaaagtgtatataaaagagaaataacactgcgtttcgaggaaaatccaatcaatatctatgcggatttattaaagataaagaaggtaattatcatcttgcttgataatgccattaaatatagcaatgacaaaattgaagtcttcttagataggaatcaagaacatgcaataatccatataaaagattatggtatgggaattccagaggaagaaatagagaatatttttgaaaggttttaccgagtgaataaagcaagaaaccgagaaactggaggttctggtttggggcagcatattgccaaaagtattataaatcttcataagggtgaaattaaaataaaatgtaaagaaggatcagggacgaatgtagaattgtttttaccaattagcaatggaaatgaggaaaaaaatacacagaagagaaatccacgacaactggtatcgttccaccaatga

SEQ ID NO: 53 - DNA, 201 bp, Peribacillus Aracenensis
  source 1..201: mol_type = genomic DNA
atgaattttgaacaaattgaaccctttccccatataaggaagagggttttttgtgttgtgaaaacaggattttcaagcatactcctgtatgtgttgccatttacacaaaaacattggcgtttatctcgttccaatgtcggggctatcactgtaaaaagtcggggtcatcgagaacacaaatttttcattccatttttttga

SEQ ID NO: 54 - DNA, 225 bp, Peribacillus Aracenensis
  source 1..225: mol_type = genomic DNA
atgcataataacgtacttattgataatacattcgaaaatgttaatggaagaagtcacatcagtttatccagttcttcaagaaatggtcgtgtttacaattataggacaataactttgcggggggattttcatctcaggtggagatgtaaaagattcttaagtaatgccttaaacattgaacaaaaagataacgacattgacatcgaagaaattgatctgtattaa

SEQ ID NO: 55 - DNA, 474 bp, Peribacillus Aracenensis
  source 1..474: mol_type = genomic DNA
atggcgctaatcaatagtaaatccgatggcttcagctttactctgaataagattgtttatgatgctggaacagaaataaagcatcagaatctgaataaaatacattacaatccgcacaaaatgaagcgaattatgataaatattttgaagcaattgaaaacaactcggcatatccttgtggtgttggtaatcatggacatacaccagaaagattcattagaaacgttcgtattaaagatcatgcatttgaaggttgtacttttgcaggaattcgaccttacaaatttgaaaatacttggatcaagaataatacccttgataactgtgattagggaatacgtctctaatcctgatggtaaaggtacaaatgacaatggagttccagaagcaggtaaaaacgttacaattaaagataattccacaaatgacacaaccacagaagtagtgtatataaatgacggtgatgttgcataa

SEQ ID NO: 56 - DNA, 282 bp, Peribacillus Aracenensis
  source 1..282: mol_type = genomic DNA
ttgaaaaaggctgaaagaaataaatatgctcaggcaaatgtaggtggaaaagacaaattagcagatgatgatgtcggacatttaacaggagcacaatttaatggacctcctgatattgataatcttgtaccacaaaatagtcaaattaataggaagggtggagtttggtacgaaatggagactgagtgggccaacgcattgaaagagatatgcccaaggaagtctctgttagcattgaaccaatctattctaataattcaatgcgacctgattcctttatag

SEQ ID NO: 57 - DNA, 1671 bp, Peribacillus Aracenensis
  source 1..1671: mol_type = genomic DNA
ttgaagaaaaagtttattgttcctgcagttctatcgtcagcgttgttggtaggttctatcccagccggtaatgtatttgcgaagccggttgattcgaaggtggctagtagtgtacaagcttctaaaaagtggaatgagaaggcaagcgttcctgtttttgtgaaggagcgatttgctgagaaattctcttctagcaacccttccaatgcattaaattatttaaagaaaaacgaaggtaaaactggaattaaaaatccagataaaaacttaaaagtaaaagattcacaaaaagataaactcggtatgacccacgttcgctttaatcaatcaataaatggagtgaacgtagaaggaaccgaagttattgttcattttaacaagaataatgaagtcgtatccgtcaacggaagagtaaatcagacgattgccgatgatgcggtgtacacgactgcctccttaagcagtgatgcagcactaaatcaggcactatcatctgtcaatgcccctgaagagctaacgtatgagccaacttctgagcttgtagtctatccttttgaaggagagaatcatacagcttataaagtgaatgttaacttcatgggggatgagcctggcaactggtttgtctttgtggatgcaaacacgggtgaaatcatcgataagtataatggtttaatgcatgctgatgaaatgaaaacacaaaaaggtgctggaaaaggggtacatggtgctcacagggaattacatattacccaagtgaaggaacctaaatctggaactcagtttgcgttagctgattactctcataatggtcttgatggaatacttacgtttgatgctaaaaatgataatagttccagtaatgatactctatatgtggggaattctgctgcatttatcagcgactatgatcgggctcttgtcgatgcacactataattcggaaaaggtatatgattattaccttaatgagcatgaccgaaattctcttgacggtgaagggatggcaatcatttccaaggtccactatggcaataattacaacaatgcatcctggaatgggcgttggatgacctatggggatggtgacggtgagttctttatttcactatcagccggtcttgacgttgctgcccacgaaatgactcatggcgtcatcactcatacagcaaatttagtttaccgcaatcaatctggagcactaaacgaatcatttgctgacgtctttggtgcacttgttgacgacgatgattgggaaatgggtgaggatattatggcaccagctgctaaagctgacggtgtaacgagattgcgcagcttgagtaatccaaacagtgttgtagtaagtaatgcggaaagagctgcatatggcagtggagtctatccggctcatatggatgaattttatcacatgccaacttcggtagatggcggcggtgtccatgttaactcctcgattacaaaccacgctgcatacaagattggtcaagaaattggaaggcacaagttaggacaaatctactatcgtgcaataagcatttatttaacgccaaattccgattttagtgacgctcgtaaggctattgttcagtctgcaattgatatttatggtgaaggcagcaaggaagaggctgcagctgctgccggatttgattcggtgggaatttactaa

SEQ ID NO: 58 - DNA, 792 bp, Peribacillus Aracenensis
  source 1..792: mol_type = genomic DNA
ttgaatatagtagcgagtggtacaaagttcgtcccttacagcaaggaatttgcgcaaaagcaggtacagtacgcaaaagctacaataacagacatagcgagatcaggaaaaaccacgttaaaaaatataggtgaagaaataggtaaaaatgaaatccctaaacgggtaagtatggaacaagtatccctcggaggacaaccccttcgccaagttatgatggaaaagcagacaattaaggaagcctatcagaaatttacggtgaaggatagcaaagtagagggagtttcaggggagagtatttctaagggtatagataatgttagaaatggtgatcaatacacgaaagtaaatcgtaagaagaccttaaaacccaatgtagagtatacaacaaaagaaggatataaatataccactgatgataacgggcgtattgcaattgctgaagttaaattagaatttggtaaagcaaaacaaaatccttatgcccaaagaaaggttggaggaggcgatagactatcaaacgatgatggtggacatttaattgcaattatctttaaaggttctggtgaaatagataacttagtacccatgaatgctactttaaataggagtgaatataagactctagagaatacatggaagaaggctttagtaaaggggaaagaagtaaccattaaagtaaaacccatatatgaggcacactcagctagaccaagtgagtttaaaatcaactatgtaatagatggtaaaaaatattccgatagattaactaattatttaggaggtaagtag

SEQ ID NO: 59 - DNA, 1005 bp, Peribacillus Aracenensis
  source 1..1005: mol_type = genomic DNA
atggaagattataatgtaactggattaagtattgcagcaattgatggtggtaacataataagtacagaatgcttcggtttacttgaagtggaaacagataaaagagtggaaagtaattccatttttagtgcttgttcaatcagtaaatttttaacctcaattctagtgatgaaattgacggaacaaaggattcttgatctagatgaaaatattaatgaaaaacttttatcgtggaaagttcctcataatgaactaaataaaaataagaaagttaccttaagaaatttactgagtcaccaatctggtgttattgaccccgaaggaagttttattgatctcaattcgaggatggaaaatcccacaatggtcgagatattagaaggaagaacaccctattgtaaagctcctattgaaattaagtatgagcctgggagcacctttcaatattcagacgcaggtttttgcattatacagcttttgatagaagatgttactggaaaaccttttaaggaagtaatgaatgaacatatttttcatccattaaatatggaaaatagcatatttgaacttccaacatcagaagcaaccaaaaaatatttctcttgcggtcacaacaaaagaggagaattagtaaatggaaaatatccaatttatccatatccagcagcttctgggttatggacaacgcctacagatttagctcttttggtcattgaattaatgaatgctttacatggtgaaagtaagcttaagctttcagtatgtaaagcaattgaagttataaatccccaaggttgtaaggagtggactgggctaggagttttcctagataaaaacgaaaagggaattgaaatttcatcacttggttggggtgttggttttcaatgtatgatggtggcttatccttatttagaaacgggattagtcataatgataaataccgatctaggtgttcatcaattagaaggtattattggtgaagtctacaatgcttatcctttttaa

SEQ ID NO: 60 - DNA, 333 bp, Peribacillus Aracenensis
  source 1..333: mol_type = genomic DNA
gtgatcaacaattcaaagttggtcggggtcatgaatgatgaagatatagctgcattaaattggttgaatggtgaggtaaagggaggaataatcgaagcggtccaacacggtaaaccattaagtgttgaagtgatcaataggacaaggaagaaaatcaagacggaattgaacggggatcaattgacgatcaatattaggtgtgtggaaaatcagcatccaaagttttgggagaaaaataagaagaaatgggacgaaattttcggtaatgctgtcattcatcatgaagtggatattagggtcgtagacgtcgtttcaaaaggagggataaagtga

SEQ ID NO: 61 - DNA, 132 bp, Peribacillus Aracenensis
  source 1..132: mol_type = genomic DNA
atgaaggaaattcttcgtgaaattggaatgatagcaagggcattagatcaagaaatagagataaagaatgggagtttgttaaaaagggaaacaagagaaattattgattatatgaaggagcgacatatttaa

SEQ ID NO: 62 - DNA, 405 bp, Peribacillus Aracenensis
  source 1..405: mol_type = genomic DNA
atgaataactttgattcaatttgtgaacaatttgctactctcctaaaaggaaaaagtaacgtaaatcaaggtagttgttctgtatcattacaccgtgattttaaggtgatagttcaagggcgccaaagcagttctgttgtgccggcaggagtcttatttgaatcattggatcaaagtggtaatgcgttaaatttggctgaaatcgctgttttacaagaagagattcctagttttatttattcaattgtccaacagggtttgattgtgagtgccctacataatcactggttatttactgaacctttaattatgtatgttcacattcaatctattgagcctccattaaattttgcaaaaaagatggtacactcattttcatttttacgcagttatcccgttgcttag

SEQ ID NO: 63 - DNA, 834 bp, Peribacillus Aracenensis
  source 1..834: mol_type = genomic DNA
atgaaagatttattaaaccagttgtacgtaccttcacgatttgaaaaagcagataaggttttttggcaagatccttatattgccaaacaattactagaagctcatttaagtcctgatacggaaggagctagtagaagttttacgtttattgataaatctattgattttattcaacaagttgctccaagaaaatcttatcaaaaagtattagacttaggttgtggtccaggtctttatagcgagcgtcttgcaaaaaaaggttatatggtaacagggatagatttctctgaaaactcaattcattatgccaaagaacaagcaaaagaactaggacttgatattgaatatcgctatgagaattatatggcattagatgattcaaatatctttgacttagccctattgatttattgtgattatggtgcccttgcatcagaagatcgcagtaaattaatttataacatttggaatagcttaaaaaatggtggacagttgctattagatgttttctcgcaaaacaaatttgatgagttcaaagaagaacaatattggaaccttaacgaaaatggcggtttctggtcggaaaatccttatatagcaatcggtagaaatcttaaataccctggtagggtaacattagagcaaacaacggtggttaccgatgatagaacagaaacttactacatttggtaccaattcttcacaaaagaattatttatcaaagaggttactactgtagggtttactgtaaaagaaatttacaatgatgtttctggtgaaacttataatgaaggtagtcaaacaatcgccttattgttagaaaaacgagaataa

SEQ ID NO: 64 - DNA, 612 bp, Peribacillus Aracenensis
  source 1..612: mol_type = genomic DNA
atgaactatgaaatatttcaatggattaacggttggtccggccatttctcttatctagataaaggaatgatattcatcactaatagcgttccttatgtggtaatcgcacttatgttgttcctatggtttattgcaaacaaagaaaaacgggcggaaaaacagtacacagctatatacgctgttttttcttgcttacttggattgttcataaacgcaatccttcaccttgtctactatcatccacgtccattcgtggcataccatgttcatcagttaatactgcatcctgctgactcttcgtttgtaagtgatcactcggtattagtattctccatagcatgtacgatggtgctacgaaacgactcgtggaagtatcccgtattagtatgggctattattgttggcatatcgcgtatattcgtcggagtccattatcctgcagacgtgattggtggcgtccttatttcatacggggcaagcatattcgttatgcagtcttccaaaaaattggagcctttggtacaagtagtgttctacatgtatgacagagtaacgaaacatatccctttccttgctaagtacagccataaaaacctaagtcaagaaagataa

SEQ ID NO: 65 - DNA, 1518 bp, Peribacillus Aracenensis
  source 1..1518: mol_type = genomic DNA
atgcaagaaaaccaaagtaaaatgaaaattttacttaacaaagtgccacaagtgacgattttcttttggatcatcaaagttttgtgtacaactgttggtgaaacatttgctgattacatcaatttcaacattggacttggtttaactctcactaccattattatgggagttgcgttttttattgcattgttttttcaatttaaagcaaacaaatatgttccagccatttactgggtaacagttgttcttataagcgtatttggaacacttgtaacggattatttgacagataatatgggcgtaccacttgaggttagtacagctatattctcggtgttgctgggactgacttttctattttggtatcttagtgaaaaaacactatcgatccactcgatttttactagaaaaagagaagttttctactggcttacggtccttttcacctttgcacttggaacagcggtcggcgatttatattccgaacaacttggttttggttatcttaacacaggaataggcgttgttattattattgctcttgtgttcttagcttataaatttttgaaacttgacggagtattagctttctggattgcttatattttaactcgtccgcttggagcgtcaattggagattacctatctcaaccaaaagtaaatggcggattaggactcgggacaaccgttacgagtgtgatttttcttatcgctattttagcaatcatcgttttccttgccgtttcaaaaattgatacaaatgctaaaagtgatatagcggaaacaaaccaaagtaatgcaaataagaaacatgtgctaacacaaacgcttgttgtactcgtaattttcttagttgttggtataggtggttataactggcgcagtaataatattgcatcacaaggtgctgcagagcaagctacattagcgggtcaattaaatgattttgttaaaattgaaaatgatatgctaaacgctgtaaataaaaacgactttgcttcagcaaaaaaaggcgctgataatttggaacatcagtgggatacacaagaacctaagcttcgaaaaattgatagcactacatggacaaaaattgatggaacaattgactctgtgctagcagcggttcgttcttcaaaacctgatattaatcaaagcaaaacagcacttactaattcacttagtgtcttaaaaggtgcaaataaatcaacatcaaaatctggtgcctcacaaactacattatctggacagttaaacgattttgcaaaaatcgaaaaagatatactaaacgctgtaaacaaaaatgactttgcttcagcgaaaaagagggcagatgaattagaacatcaatgggacacacaggaaccaaatctccgaaaaatcgatggggctacatggacgaaagttgatggaaccattgatgttgtattagcagcagttcgttcatcgagtcctgatgtaaacaagtgtaaaacagcacttaacaattcacttcgtaccataaacgcagcaaataaataa

SEQ ID NO: 66 - DNA, 120 bp, Peribacillus Aracenensis
  source 1..120: mol_type = genomic DNA
atgcttggagtccgcaatataaaacgtgaaataggctacgggattcatccgtattattggagaataggatatatatcggaatatttctgggaggtagaaaaatggcgaaaattactgtag

SEQ ID NO: 67 - DNA, 126 bp, Peribacillus Aracenensis
  source 1..126: mol_type = genomic DNA
atgaccaaaaccattagccttatttgtgctagtttacgcaataattcttataatcgaatcattgctgaatcattggcagtcatggatggttcagcccatttcgttgttacaaaaaagagaaaatga

SEQ ID NO: 68 - DNA, 801 bp, Peribacillus Aracenensis
  source 1..801: mol_type = genomic DNA
gtgacagacaaaaaaatcacagtacaatttacgatgctgacattttgcatagcctatcttgtgtcaggtgctttgattgctctcgggcaattcggatattcggttcacaattgggttcactcgttacagcaattcgggatgaatatcccttttgcaatctatattttgtcgccggctattgcttcatatatcgttctgaagaaaaataacaaaatagcaggtttcaaggaatggttgagaactgttttttatgccaaaaatagcatatctctctatttgttcgttgttgcaggacttacactgtattttttgatacatattgcagtttcaggccgcacggaaatggtgcttccattttatatgttcttcctttccctgcctggtaatcttattatcggtggcttggaggaagctggctggatgtacatattgcagcctgagcttgacaaaaaatacggttttgttttgtcttctgtttttgttggaattatttggattttatggcatatccctcttttcttcattccggggacgaatcacggagagggactcattaacttttggatgtttgcagttcaactcattgcgtttcggtttttcaacgggacaatctacaaaatatcaggaaaaggcagtgtgtttatgtgcgtattattccacaccatgttcaatgcggcatcccccatcttcggaaccatgactatgacttgggcgggaaccattgccgcaaatgctgtgattgttcttgtttcaattgtaaccgttttgatatacgacaaaaagaaaaggcgaatagtataa

SEQ ID NO: 69 - DNA, 819 bp, Peribacillus Aracenensis
  source 1..819: mol_type = genomic DNA
atgtccgatggaaatgtaggcaaatattttactactggcgaattcgccaaattatgcaatgtaaaaaaacaaacgctcattcattatgatgagattgggcttcttactcctgatttaaaaaacgaaaagggctatcggtattactcttatcaacaattcgaagttttttcggtcatcacgcttttaaaagaattcaatatgcctttgaaagagatcaaatggtttcttaccaacaggtcacctatggaactaattgagcttttcaaagaaaagaccatagaattagaaaaaaagataaagaaccttcacagagtgcagaaaatcattgaaacgaaaatatacctcactgaaaaagcgatttgtatggatgactctcaaatcaccttgaaacttcaggaggaagaacagctcttccttagtgaatccatcctgaactcttctgatgccgaattcttaaaatctacatctgacttcattgatttctgtaatgaaaatgaattttacacaggattccctatcggggccatgattagtaaagaaaacatcatcgacgggaatcatgatgactattcatttttgtacacgaaagtcatgggaaaagcccccacgttctattcaaaaccgaagggactctatgttattgcctatcataaaggcagttataaaaatatctccgaaacgtacgaaagaatattacaattcatggcgagtgaaaacttgaacctcaaatcgtttgcatacgaagaatacatcttggatgaagtcgcggtaaaggggtatgaaaactacctgacgcaaatcatggttgaagtggaatga

SEQ ID NO: 70 - DNA, 549 bp, Peribacillus Aracenensis
  source 1..549: mol_type = genomic DNA
ttgtcaactttattatttagaggaattcggagatctattcagcttcggagatatatcctggttttttcgtcgatatatcgcagatttcggagatctatcacggtttttcgtcgaaatatcgcaggtttcggagatatatcctggtttttcgtcgatattttgcaggtttcggagatctatcctggtttttcgtcgatatattgtagatttcggagatatatcctggtttttcgtcgatatatcgcagatttcggagatatatcacggtttttcgtcgatatattgctattttcgaaaatatatcctggtttttcgtcgatatattgctattttcgaaaatatatcctggttttttcgtcgatatatccgcaggttccggagatctattttagtttttcggagatatatcgcagcttccggagatatatcctggtttttcgtaaagatattgcaggtttcgaagatatattctggtttttcgtcgatatatcgcggatttcaaagatatattctggtttttcgtcgagatatcgcagatttcaaagataa

SEQ ID NO: 71 - DNA, 567 bp, Peribacillus Aracenensis
  source 1..567: mol_type = genomic DNA
atgttagttggatatgcaagggtatcgacagttggacagtcgcttgaaaaccaagttgaacaattaaaagaatatggttgcgaaaaaatatatatggaaaaagaaagtggaaagaaaacagatcggcaggaattagaaaatgcaagaagagctttaagaaaaggtgataaattagttattactaaaatcgaccgcctagctcgttctgttagggatctacataaaattgctattgaattggaaactgaagaaattggcctggtatttttaaaggagcaaatagattttagtaccgcagctgggaagctcatgtttaccatgttaggggcgattggagaatttgaaagggatttaattgtaagccgcacttctgaaggcagagagcgggcaaagaagcaagggaaacacctgggaaggaaaggccaggacgaaaaggaagtaaaaaaagccttgcagctttatgagactagagaatcaaacggaatgagcgtttcagatatttcaaaattaactggtgttccccgttctacgatttatgcaaaagcaaaggaaataaaaaataaataa

SEQ ID NO: 72 - DNA, 351 bp, Peribacillus Aracenensis
  source 1..351: mol_type = genomic DNA
atgtccaacacaacaacagaaccatggagacaactagtagaagtattaagaacttatgaaaatgaaacattacaattccaaatagaatcaaaagataaatccctatacatgctgcaaacaatcccaagtatgtgtctcggagaaaatgaagaattcgaagaaataagtcatctcatcgctatatcaagtgacgatattaaatttgctcaagtaaatataacactacagaaaaaagatatacttaacgttgaaagtatctatactccagatgaagttgaatggagaaaagatggtttcaaaatagaatacaaaaacgatgtcacatttactttcaatgtattattagactaa

SEQ ID NO: 73 - DNA, 150 bp, Peribacillus Aracenensis
  source 1..150: mol_type = genomic DNA
atgagtgaccaccgaatttggtggtcctttttgagttggcatagtaaatatgggaagcgtgtatatgaatatatgatttggaaaagtacggaatgtttgcacaaatgcaggattcctttacaatatttgttaggtggaaagggggattga

SEQ ID NO: 74 - DNA, 561 bp, Peribacillus Aracenensis
  source 1..561: mol_type = genomic DNA
atgtttcttattatcatattcatcattataggctgtacatatggaggcatccatttttggaagagaaaaagggtagtatcgatattcttgtttagtcctttactagcagtcatttcatttataggatacttcatttatcatacgttgtaccacacaacacctgactcattacaactaactgtccataaagaaaatgaagcatacatcgtggggggagtttggaaggatcggttagatgcgtatcgatttcctgctgattttcttgtgttctatgtccctaataatgagaatgtctccaatgttaaaagaaatagagttaaatcctataatgaaatggatgggaagtttttagagaaagaagtacaaaattggtttgggcaaaaaactcatctcgagtgggaaccgcaaatttttgatttacatacaaatagtgaatttgaatttacattcgatctcccaaggaacgtaaaaccaagtgatgtggaattgtattatatacacacaagagaagagccaatggaggcattagagttttggtccaagaaaattgaattaaagtaa

SEQ ID NO: 75 - DNA, 159 bp, Peribacillus Aracenensis
  source 1..159: mol_type = genomic DNA
atgcttgcctttttgttgcatttagaatggttgggaaagagcctgattggcaacatcgacgtcattttgaagcaattggttaaagtcgtatgcaggatagagatttctttcataaaggcagtggaatatcttggcgtgggtatcgatggctccatttaa

SEQ ID NO: 76 - DNA, 111 bp, Peribacillus Aracenensis
  source 1..111: mol_type = genomic DNA
atgttagtagcaattactcatgagttagagcgttttactcgtgagttagtagcaattactcgtgagttagagcagtttactcgtgagtcagagcaattactcgtgagttag

SEQ ID NO: 77 - DNA, 150 bp, Peribacillus Aracenensis
  source 1..150: mol_type = genomic DNA
atgaaaaagcagaagaaaataatgagaaaagcctgtcacataagcggcaggctttttctattcagccagattaacaaagagtataaaactaatcctaatttgaatttgaaaatgttagatacctatgtgatagtttgggtagatcaataa

SEQ ID NO: 78 - DNA, 126 bp, Peribacillus Aracenensis
  source 1..126: mol_type = genomic DNA
atgatgccggccttctttttgttgactaagcttatcgaacagggaattgcagccaattatgagtttaaaataaaattgaaactggtatattcgttttgtataatgagtaagttgaggggtgaataa

SEQ ID NO: 79 - DNA, 2289 bp, Peribacillus Aracenensis
  source 1..2289: mol_type = genomic DNA
gtgaaaattcatatagtccaaaaaggcgatacactttggaaactcgccaaaaaatacggcgtcagttttgaagaacttaaaaaagttaacacgcaattgagcaacccggacatgatgatgcccgggatgaaaattaaaataccagggacatccggagcagtaattaaagaaacgggtaaaccaaacgtgaatattcagccgggaatgaaagaatcccaaattcaaccgcaaccgaatcagtcagcaaatatgaaagagcagcaaattatgaaaaaaccggccgttaaagaacagccgaaatttcaactgccgataaaagagcagccaaaatttcaacagcctgtaaaagagcaaccaaacattcaaaaaccagtgaaagagaaacagatcgttccacagccggttaagaaagagaagcagatcgttcagccaaagccaatcattaaagagaagaaagtaatcgttccaaaagaagtgccggtgcccatgccggtgattccggagatcgacgtcaataattattatatggtcaacatgaccaatatgagtgtgcaaaagcctccagcaccaccacctttaccgaagaaaaaagaaaagcctgcagtgaccaaaaagaagaaaaagccagctgtacagccagctcaggaatatagtgagccggtggatgattgtattccagtaacgccaatcttgcctggaagcggttattgcattgagccgccaccatgggcgcatatgcatggcatgcaagcaccatatcaaggtgcacaagggtatcaggcggctccggaaatacaaggttatccaatgatggaagagagctctgaaagtttggaggaatcttctgacatgcaaatgatggatcaaggattcgtccaaggggcgagcatgaatgtaacagaccagcaacattatccatatcaagcctccgcaccggttccgcaccattattatggagggatgaatcaacaagctcaagcagcaggttcatatatgcaacaaggttatgagtcaccaggcgaattgccttcttcatacaatcaaaatttccctcagcattattcccagcctgctggtgaggaggattgcggctgtaataaggggttacttggaacttatgggccggaagtgaaggggcagtatcaagggaacaagaaaatggatgcccatgcacatcaccatccagattatcacgaatatcaatccgttcaatcacaagccccataccaagggttgtcaccaaaagagtctcagatgggaatagcgatgccatcccaatatgaagatgaagaagaatcatatgatggattcatgatgatgggtggccaaaacccaggtcagccgggtatgatgataggcggccaaaacccaggccagccaggtatgatgggcggtcaaaacccaggtcagccgggtatgatgatgggcggtcaaaacccaggtcagtcaggtatgatgatgggcggtcaaaacccaggtcagccgggtatgatgatgggcggtcaaaacccaggtcagccgggtatgatgggcggtcaaaacccaggccagccaggtatgatgatgggcggtcaaaacccaggccagccaggtatgatgatgggcggtcaaaacccaggtcagccaggtatgatgatgggcggtcaaaacccaggtcagccgggtatgatgatggacggtcaaaacccaggtcagccgggtatgatgatgggcggtcaaaacccaggccagccaggtatgatgatgggcggtcaaaacccaggtcagccgggtatgatgatgggcggtcaaaacccaggtcagccaggaatgatgatgggcggtcaaaacccaggccagccaggaatgatgatgggcggtcaaaacccaggccagtcaggaatgatgggcggtcaaaacccaggtcagccgggtatgatgatgggcggtcaaaacccagaccagccaggaatgatgccgggacagtttggtggtcagtcaggaatgatgccgggacagtttggtggtcagtcaggaatgatgccgggacagtttggtagtcagccaggaatgatgccgggacagtttggtggtcagtcaggaatgatgccgggacagtttggtggtcagccaggaatgatgccgggacaatttggtggtcagcgagacatgatgcgcggccagcttggtggtcagccggaagcaatgttaccgggacaaatgggaggccagccaggccaattcgggggcgtccgtgcgcctgaaacatttgggataccgacatatgtagatgaaagcgatgactactaa

SEQ ID NO: 80 - DNA, 198 bp, Peribacillus Aracenensis
  source 1..198: mol_type = genomic DNA
atgagtgtcgttccttgtatcgtttggaccctatttattttttatatttataaaaaactagataaagaagatataaacgcttttctaaaaaaatggtctacacctttaagtgttgaaatcatggaccccactgcaaaaatcatcgtgttggaacaggaaaagaaacctttatatgatttagaagttagagcagtatag

SEQ ID NO: 81 - DNA, 315 bp, Peribacillus Aracenensis
  source 1..315: mol_type = genomic DNA
gtgtttgtgccttttactcgtgagtttgcgccttttactcgtgagtttgtgtcatttactcgtgagttcacgctgtttactcgtgagttcacgctgtttactcgtgagtttgcgccttttactcgtgagtttgtgctgtttactcgtgagtttgcgccttttactcgtgagtttgcgccttttactcgtgagtttgcgctgtttactcgtgagtttacgctgcttactcgtgagtttgcgccttttactcgtaaaatcaaaaaagacagttccccatgtatcagggagctgtcttttttggttttatcctcttag

SEQ ID NO: 82 - DNA, 219 bp, Peribacillus Aracenensis
  source 1..219: mol_type = genomic DNA
atgttttttacagtaattcttaatggattgaaaattcttaatggattgaagaaatttgcgacactcctgccgaataactggctagccgagaccccggtgacgcttgcgtcgaggaggcttggcagacagtcggaggaaagggagcggatttctgaaatcaactcggatgtttttaagaaagaaaaaactgaaggcggtctcatcccgaacctagattaa

SEQ ID NO: 83 - DNA, 213 bp, Peribacillus Aracenensis
  source 1..213: mol_type = genomic DNA
gtgcgagactcctgcggggatacgcgtccaagggagaccccacaggcgcaaaagcgcctaggaggctcccggaccgcccgcggaaagcgagtgcctggagaggaaatcaacgttcccattttacaaacccacaaaaaaaatgttggcaagagaaatcatgttcgttcgcctttttcagcttcctgccctgtagcggattttccatcaaactga

SEQ ID NO: 84 - DNA, 201 bp, Peribacillus Aracenensis
  source 1..201: mol_type = genomic DNA
gtgaattatgccgatttactcgagaaaggagcattactcatagaatgcagctgcaaactcacgaaatataagcgtttactcgtgaaattagagcaaatactcgtgagtttggtcgatttactcgtgagtttagatcaaatactcgtgagtttggagcaaatactcgtgaattatgccgatttactcgtgaaaggagcatga

SEQ ID NO: 85 - DNA, 1440 bp, Peribacillus Aracenensis
  source 1..1440: mol_type = genomic DNA
atggctgaattagataatgaacaaggtctcaaaagggtaatgaaaagtcgccatttatttatgattgctttaggtggtgtaatcggtgcagggtttttcaacgcttcaggttttacgattagtcaggcaggccctataggcgcagttttagcctatatgatgggcggacttattatgtatttagttatgctgtgcttaggggaattgacagtggaaatgccagtatccggatctttccaagcttatgcgactaaatacattcatccatcgacaggctttacagttgggtggatttattggattgggtggtcttctaccgtagcctatgaaattatcattataggttcgctgatgcaaagatggttccctgatatttctccatggatctggtcgttaattgcaggaattgtactattttctgtaaatgccctttctgcacgcagttttgctgaaacggaattctggtttgcgagtatcaaggtaatcgctataatctcttttatctttattgggttagccgtcatttttggtattgtaccaattgagggtgaaccagcggctccttattttacacacttaacagaatttggcttctttcctaatggaatgtttgcagtagttattgctatgatggctgttaattattcattaggcggtacggaacttataggaattgcttctggtgaaagtgaaaatcccgagaagacgatccctaaggccataaaccaaactgcttaccgaataatattattctttgttttgtcaataatcatcgttgtttctatagttccttggcaacaaatccagccagctgccagcccgtttgttacagcactagataacatcggtataccatatgcagccgatattatgaattttgtcattattacctcattactatctgttgctaactctggtctttatactacaactaggatgttatactctctttctagttctaagatggcaccaagatcctttcaaaagttaaccaaacaaggtgtgcctttacttgctttaacggctagtatgggaatctcctgtgtgtccattcttgtttcaaaagtagcggctgaaactatttatacctggatcctttctgtagcaggaatggcatccatgttggcttggatgagtattgcggcatctcagtattttttccgcagacgatatgtagctgaaggaggaaaagttagtgatctaaaatttcggaccccacttttccctttagttcctatcttggcatttgtctttaatctagttgtattaataagtttagtatttgacgaaggaactaagttgactatttatattggtgttccagtagccattgcttttcatttgatatatattttatttttgcaaaaacgcgtaaagaaagatgttgggtcatcagttcaagaggagtatgaaaaggtgcgtttaattaataaaagttaa

SEQ ID NO: 86 - DNA, 1275 bp, Peribacillus Aracenensis
  source 1..1275: mol_type = genomic DNA
ttgcagttaatcaaagaacaaattcaaacatggttaaaagagcattatgaagaaggtacagaattattacaacgacttgtacaatctcctagtatttctaaaaatgaggcaaaagcgcaatcaataatcactgaagtattatcgaatatggggttaaaggtggatgcctgggagccatgtggagaagaattaaccgaaagtccctacttttgctcgtcaagggatgattttacaggaagtcctaatgttgtaggtgttctacccggaacaggcggtggccgttccataatcttaaacggacatattgatgttgtccctgagggtgatcatgaacaatggacagatgatccctatagtggagcgattaaggaaggaaaaatgtatggtcgtggtgttacggatatgaaaggtgggctagtttcattccttttagccttacaagccattctgcaactcgacattaagcttagaggcgacgttatttttcaaagtgttatagaagaagagagtggtggaacagggactttatctactattctaaaaggctataaagctgatgctgcactaatcactgaacctactaatatgagggttttccctaaacagcaaggatccatgtggtttaggatctttgtcaaaggacggtcagcccacgggggaacacgatatgagggagtaagtgcttttgataaagcaatggtactagcggagcaaatcagggctttggagtttaaccggaatcaacgtattaatgatcctttatacgagcagacccctatccccattcctattaatatcggagttttttcaggaggaaactggccatcttcagtacctgatttgctgaaaatagagggaagaatgggtgtagcacccaacgagaagatagaagatgcacaacatgaaatggaggaatgtctacaacaactatcagtcctggacccatggtttaaggaaaatccacctgtcttagaatggtttggtgctcgatggctaccaggggaaatcgatcttgaacatgatttgatgaatacgttagttcatcaatatagagaaactactggtgaagaacccgtgatagaggcctctccttggggaactgacgggggattacttacagaagtagggaaaattccaacggtggtttttggaccagggacaacggaaatggcacacttcccggatgagtatattgaattggataaagtttttaaatctgcagaaattattgcattaactataattcagtggtgtagtatcaaggacaatatctga

SEQ ID NO: 87 - DNA, 1182 bp, Peribacillus Aracenensis
  source 1..1182: mol_type = genomic DNA
atggaagatgccgtcatcgtatcaggagttcgtactggagtgggtgcatttggaaagtcccttaaaagtgtttccgccactgaaatgggaagacaaatattggagggtttaatggataagaccactcttaccaaagcggatgtaaatgaagtgatatttggacatggatatgtacatgggggaggattgaattcagctagaatatcatcgcaattagctggattcccaacgagtgttccaggacatgtagtgatcaaggcatgtggttctagtttaaaagcaattactaacgcggccttaacgattaaggccggtcaagaagaggtggtaattgcaggtggggtagagaatatgagtcaggtcccatatttagttaaaaatagatgggggacaaagtttgggaacgtagaaatggaagatgccctattaactgatggtttaatttgttcgttggaaaatgaacatatgggaatgacggccgaacgcttaacgcaaatttacggtatctcccgagaggaacaagataaatttgcctttgatagccataaaaaggcagttcaggctattgaaaatcattattttaaagatgaaattttaccagttcaggtcaccggtacgaaaggaacttacctattcagggcagatgagtctgtacgctcggatattcagctagaaaaattaatcaatcttccacctgtttttaaatcggatgggtcaatcactgctgggaatgcgtgccctatgaacgatggagcagcagcagttttaatgatgtcaaaaaagaaagctatacaaaaaggtattaaacctttgttaaaagtgaaagcattttccagtgctggtgttgaaccaggcattatggggattggacctgttccagcaacaaaaaaagcactggaattagccgggttaactttagatgatattggtttgattgagcttaatgaagcctttgctgcacaggcattagctgttattaaagaactagagttagactattcaaaagtaaatgttaatggtggagctattgcattggggcatccagttggagcaactggtgctaagctaactgttagtctaatgaatgaaatgttacgtaccaaaacaaagtatggaatggtgacgctatgtatggccggaggaatggggcttaccgtcatatatgaaaacctaacattataa

SEQ ID NO: 88 - DNA, 660 bp, Peribacillus Aracenensis
  source 1..660: mol_type = genomic DNA
atgggtttgggagtagaagaacgccatcgtatcgctaagcgcgctgcccaagaaatagaaaatggaatgattgttaatctaggaataggcattcctacattaattgctgattatatcccatcggatatttctgtccaattccatgccgaaaatggagtgttgggcactggtccgacaccaaacaggagtgatattaatcctaatttatgtaatgccggtggttatccctgttcggtggttcaaggagcctccttttttgacagtgctactgcatttggcatgatccggcgaggccgtttagatgttaccattttaggagcccttgaagtaagcgaggaaggcgacctggcaaattggatcgttcctggaaaacttgtccctggtatgggtggggcgatggagttggctcaaaagtctaaaaaggtaattgtattgatgaaccatacaaacaaacaaggtaaatcgaaaatactgaaggaatgtacactaccacttaccgctaaaggttgtgttagtttgatcatcactgaaatggctgtgatcgaggtaacgccacaaggattagagttaaaagaagttatggagccttacacagtggaagatgtaattaaacatacagatgcacaattgaaagtattaaaaaccacaggaaaagtttag

SEQ ID NO: 89 - DNA, 699 bp, Peribacillus Aracenensis
  source 1..699: mol_type = genomic DNA
atgctactgtccaagtctaaacaaggaaaggtaagtactttagaggctgcccttcaaagaatttccgacggatgctccttaatgtacggaggatttggcggcattggtactccccctaccattgtagaagggatattgaataaaggatgtaaacatttaagtttaataggtaatgacgcaggtttcccggacgttggggttgggagattgattagttcaggaagggtgaagaaactaattacttctcatattggctccaacccaatagccggtcaattaatgaacaagggggaaatggacgtaacattttctccacaaggaacgttgattgaacgtattcgagccggtggtatgggattaggtggtattttatccgatgtgggattagccacggttgtagaggaaggaaagacacatattactgtaaatggacaggtatttttgattgaaacagcattaactgctgaagtatctataatccatgcttcaaaggctgattatcttggaaatctcatatttgataaaagcgcacgtaattttaaccctttagttgccatggcgggggattttacgatagttgaagcagatgagattgttcaagttggtgaacttgatccagaatcgattataacccctggaatctttgtggatatggtaattccaagtgaaggagtgaattggaaatgggtttgggagtag

SEQ ID NO: 90 - DNA, 1368 bp, Peribacillus Aracenensis
  source 1..1368: mol_type = genomic DNA
atgaaggaacgagattatttaattaaaccggtattaggacagcaatatccaatagctgcatctgcaaaaggcatatatatatatgatcagggcggtaagaaatatatggatgggtcgtctggagctgtaacggtaagtattggacacggtgtacaggaggttattaaagaaacccttgcacaggcagaaaaaatttcattttcttatagatcacaatttaccaatgaaccggctgaaaagctagcagaaaaattgagtcaattggctccgggagatcttaattggtcattctttgtaaatagtggttcagaagcgaccgagacagcgatgaagattgctatacaatattggcaagaaaaaggacaaccacaaaaggatcgcattatatctaggtggactagttatcatggcattacaatgggagcattatccatgtcaggacatatattaagaagacagaggtttgcagcgatgttagctgattatccttcagtagctgccccttacacttatcgtcgacccgatcatttaactgaagaagaatttggtcttctttgtgctcaagaacttgaaatggagattaggcgtattggggaagaacgtgttgctgcatttattgccgagccaattataggagcttctgggggggccatcactccaccagctaattactatcaaaaaatcaaggagatttgtgagcgttgtaacgtcctatttattgcagatgaggtaatgaccggaattggccgtactgggaagatgtttgcaatagaacattggaatgttactccagaccttattactctaggaaaaggaatgagctcagggtataccccaatggcagctactctagtcagtgataaagttatggaacctatattaaatggatctaagtccattatgggaggccatacttatagcgccaatcctcaatctgcagcagttgcactaaaggttattaaatacgttgagaagcatcaattggtagaaaaggcagaagaacaagggatatatcttatgagtaaattgaaagcgcttttaaagtcttgcgaaatgattggggatgtaagaggaaagggccttttaattggaatggagttcgtagccgaccgtgaaaagaaaaacccgtatccacctgaattaaatgtaacaaatagggtaattaaacaagcctttgaaaaagggttacttatttacccagcgtcaggagctattaatggaatgggggatgccattatcatttcgccacctttggttattacaaaagatgaaattgatagtttggtagatattttagaagaagcaatttctgaagtgcaatgtgaactcaacatggagggcaagatcaatgctactgtccaagtctaa

SEQ ID NO: 91 - DNA, 1560 bp, Peribacillus Aracenensis
  source 1..1560: mol_type = genomic DNA
atggctattcggatttctgaagctttgcaactgcctatcatgaaacaaacaaaattaaaggctggaaaaaaggggttacaaaattggatcaaatgggtaactattgtggaggtaattgaagatatctatcgtttacaagatggagagtttttgatcacaacaggattcggattaggagaaaatacgaaggaacgcaaggaattcgaaaagcttttatccatcggaaaactatctggaatagctatatatacaggattttatttaaaggaaattccaaaatcatttattaccatcgcagatgaatatgccttacctttaattgaaattccagcaaacataaacttttctatgattacaaaagaactactggtacaaattgttaacaaacaaagccaaacatttgaatattcactacggatccatcaggattttacacggcttgtattagaacaacacggatttgatcccattacaaaaacccttcatgaaataattgatgcaagtgtaatccttatagcaaaagatgaaataataagttcctacataaaacatgacttcattgatattaacaatttaaaggatctaaatgaaaaacaaatggataactacaaaattaatagtcaacctattatagctaataaaaatacctatggaagtctactcattataaaggaaaaaaggttatcggaagaattggattcaattgcaattgagcatgccactactgtatttgcgattgaatttttgcggaggaaagcagtagaggagacacaattgaggctcactagtgacttcctggaagaagtattaaatcctataatcccaaataataaagatatgatcgagagaggacgtaaactgggagtagaccttacaaatccacaaagtatcatatatatttattttccattattgaaagaggagaaaataaaggaaaaatacattgagttaaccgaaagtattcaatacaccatgggaaagtcaaaaatcccctacctcatgaggacaaaatccgatagtgtcattattttggtggaagcaaaacctggattaaatattttagagttagctgagaacctcttaaataattggaattcggcattatcaaatgaacaaatagctataggtattggtaaaacaactgccgacgtttatcaattacacaaaagtgctgctgaatctgagcaagcagcacgattttcccaaattctatttaaaccaaaatccatagtccattataacgattttggcgtatatcaattactcattgaaatgaaagaatcaggggtagatttagaagaattttaccaaaaatacattggaaatctgcttgattcaaaaggtatagacctcattactacacttgaagcttatctttttttcaatcaaagtattaaagaaacagcaagcgagttatatattcatcgccatacactgaagtacaggttagaacagatacagaaaaaaactggattagacctaaacaattatgataatggcataaagttatacttagctattttggcatataagttattaaaatacattcaaattcagtaa

SEQ ID NO: 92 - DNA, 99 bp, Peribacillus Aracenensis
  source 1..99: mol_type = genomic DNA
atgtggattggtgcagtaaatcaagagttagcggcaattttgggtgctattgcacgagatttagagatgttactcacgggtttagggcattactcgtga

SEQ ID NO: 93 - DNA, 354 bp, Peribacillus Aracenensis
  source 1..354: mol_type = genomic DNA
atgcccttcatgatgttttgcaattcgaaaatatgggggaaccggcccatcgttaacgatacggaatggaaccattattatattgtcttagatgtacccgacaacagtgccatcatttcattcggggtccttctatcagggcgcggaaaggtatggatcgatgaactggaattcgaggaagtcagtaaagatacacctacgaccaatatagattacggctgtgacctttggatggaccggcaaatctatcttttgaagaatgaatgcgcagcagcatgcctttgcaaaaatattatcaaagttttcttaataattgcaatcatccgcttaaggaacccgccattcagcccatga

SEQ ID NO: 94 - DNA, 984 bp, Peribacillus Aracenensis
  source 1..984: mol_type = genomic DNA
ttgaacatgatagataatttttggcgtgaattaccacggcctttttttatactggcaccaatggaagatgtgacggatgttgtttttcgccatgtagtgagtgaagcagccagacctgatgtgttttttacagagtttacaaacacggagagttattgtcacccagaggggaaacaaagtgtgcgtggacgtttgacttttacagaggatgaacaaccaattgtagcccacatatggggggataagcctgaacactttcggcaaatgagtattggtatggcgaaactaggttatcggggtgtggatatcaatatgggctgtcctgtacctaatgtgacccagaatgggaagggaagcggccttatccgtcgtccagaagttgcagccgatttaatacaagcagcaaaagcaggaggattgccggtaagtgtaaagacaaggcttggtttcacggatgtagacgagtggcacgactggctgacacacatattgaaacaagatattgtcaatctatccattcatctgcgtacaagaaaggaaatgagcaaagtagatgctcattgggaactaatcccggagatcaagaaacttcgtgaccaggtggcaccagatacactcttgacgatcaatggggatatccctgaccgtcaaactggcttaaagctcgctcatcaatacggcattgatggagttatgattgggcgcggtattttcaataatccatttgcctttgaaaagcagccgaaagatcatagtagtaaggaattgcttgatctattaaggctgcatctggatctccatgataaatactcaaaattaggactacgtccgttcaaggctcttcatcgcttttttaagatatatgtccgcgggtttcgcggggcaagtgaattaagaaatcaattaatgagcacagagtcaacagatgaagtgcgtgcattgcttgataactttgagtcaaagaatcttgatggaatgggataa

SEQ ID NO: 95 - DNA, 321 bp, Peribacillus Aracenensis
  source 1..321: mol_type = genomic DNA
ttgaaacaattagacagttcccttatagaagtaaaagaagaatccgaatggtccagtaatattcttgctgatggtgaaaaagcgtttgtttactattatcatacagattcctctgctaaagccattatattggatgcgacaaactccttatatgactgggtataccctcaattaccagaggatctatcatttttcaaaaacggaaaagaatggttggcaacgaatagccatgaacaggaatgctatattctgaccgaagataaaaatgaaattgatgaagttatgaatattaaaggaataaaagcaagtttagaagaatag

SEQ ID NO: 96 - DNA, 525 bp, Peribacillus Aracenensis
  source 1..525: mol_type = genomic DNA
gtgaattcgcacgctttactcgtgaatttgctcggtttactcgtgaattcacacggtttactcgtgaattcacacggtttactcgtgaattctgcgtttactcgtgaattcgtgcgggttactcgtgaatttgctcggtttactcgtgaattcgcacgctttactcgtgaatttgctcggtttactcgtgaattcacactgtttactcgtgaatttgctcggtttactcgtgaatttgcacgggttactcgtgaatttgctcggtttactcgtgaattcgcacgctttactcgtgaatttgctcggtttactcgtgaattcgcacgctttactcgtgaattcgctcggtttactcgtgaattctcgcggtttactcgtgaatttgctcggtttactcgtgaattcgcacggtttactcgtgaattcgcacgctttactcgtgaattctcgcggtttgctcgtgaattctcgctatttactcgtgagttcagtcattctattcaattggttcatttgttcgcatag

SEQ ID NO: 97 - DNA, 198 bp, Peribacillus Aracenensis
  source 1..198: mol_type = genomic DNA
ttggctcttttcgtaaagattgttgtttttaaaatgaaacgatttaaggttgattggagcggaagtgcgagactcctgcgggagcagcgggacaggcgagacccgacaggcgtgtacgccgaggaggctcaccgcccgccccgcggaaagcgagcatctggaggggaaatcaaccacacctcactacttggtaaatag

SEQ ID NO: 98 - DNA, 207 bp, Peribacillus Aracenensis
  source 1..207: mol_type = genomic DNA
atgttatgtgtgattaggcttccttttaatttttgttttaagtttcatgaagaatgtcagcaccgttcatttatccgtcattgcacctggagcaggattggagcaatcgtgattacatttgtcagcaaaaagtattcggaggcaattttaaaaaaacttgcaaatagtaatgattacgttttattattaaagggtgtttttacttga

SEQ ID NO: 99 - DNA, 447 bp, Peribacillus aracenensis
  source 1..447: mol_type = genomic DNA
atgaacggtttaaagggaaggcgggaactcaaacatgcaatcaccaaagcggattgtcattcattaagaaaaaatctgcaaaacttcatgaggcttgatccccatgggctagatgggaaatatttaattcgtagtgtttattttgataaatttgacaataaactcctgaggcaaaaaacagagggattctatcacagggataagttcagggcgtttacgccgaggaggctcacccgcctggcggaaagcgagcatctggaggggaaatcaaccacaccgctttacttggtaaatagcaacaaagtatgcgaaacagcctttaaagaaaacggtaggcaaactgcttttcttcgaattatctatagtctgaggtatcccaaaatattcgggataccctttttattgaattggcgtatggcttcttccgggttattcctccacatttga

SEQ ID NO: 100 - DNA, 276 bp, Peribacillus Aracenensis
  source 1..276: mol_type = genomic DNA
atggattcctttcctgatttaagatgtttagttttcttgatcattatcatggacaaagtaaaatggcacccatgtagtgcgttactcctcgcctccgtcgttttagggattatcgcacgtatggatattccagatgttgcagatgctgttcagacaggggcaggtaaaatagcactcattgtcggtttaggtgccaagcttggaaaggcgatggccgagtgtgtaaataggaattcccatgtttactggacctgtttttggttcctgaatatctaa

SEQ ID NO: 101 - DNA, 354 bp, Peribacillus Aracenensis
  source 1..354: mol_type = genomic DNA
gtgggtttggacgttactcgtgactttcgcaattttactcgtgaatttggagcgaatactcgtgagtttcgcgcttttactcgtgagtttggagcgaatactcgtgagtttcgagcgaatactcgtgagtttcacgcttttactcgtgagtttcgagcgaatactcgtgaatttggcgaaatcgtatgggtcaaatcggggcgggccatgccatgctcttcgtggtcgatgcttcgaggccataaacaaaaagaaggaatccccgctattaaaaagcggggcttcccgatattcgatgcttgcgttgcggaaggatttcattcgaacaaatccacatctccgagcttctcatga

SEQ ID NO: 102 - DNA, 105 bp, Peribacillus Aracenensis
  source 1..105: mol_type = genomic DNA
atggctgatgggaaaatgaagagagcgttgcctgttgttctattttcgttcatggcgtcagcgacttgtgttagtgcttatgagcaagaatatgtcacttggtag

SEQ ID NO: 103 - DNA, 270 bp, Peribacillus Aracenensis
  source 1..270: mol_type = genomic DNA
ttggtcaaatgcatgatttccctcgtgactgtgaatgttacgcaagatttagaactgtttttgcatgaaattggagcgaatattcgagagattgagtgtttactcgtgaattcatgccatttactcgtgaatttggagcaaatactcgtgaaattcatacatttactcgtgaatttgccgcatttactcgtgaattcaaatatgacacaaaattttgagcggtttacgcatgaatttgagtgtttgctcgtaaattcgaatattacgtaa

SEQ ID NO: 104 - DNA, 369 bp, Peribacillus Aracenensis
  source 1..369: mol_type = genomic DNA
atgtcaaaatgcagagcgcaacgcgcgctgaacaatcactttgttccaaaacattggctgaagaggggcagaatcttatgcagagatcctaacggaaaagatacaaaccttgttatcttcatgaaaaatgttgaagaaaatctcgttttattaaaccagtttttcctaagcattaccgagtttgttaagcttgtacagggtttagactaccaggcaaatttactatcattgaactcagccatcaaggcgccacgtgcaggcgaacatgatggatttgcagttgtttcaaatgaggtcaggaaacttgcagaacagactaaaaaaacgatagctgaaatagatgcaatcgtgcaaacatcaaataaataa

SEQ ID NO: 105 - DNA, 138 bp, Peribacillus Aracenensis
  source 1..138: mol_type = genomic DNA
gtgactgggagaacaagggaagagtttgaggcaggtgatcatgtattgttcatcggtgagatccaggagttacatttcgaagatttggaagcgcttactttcatcaagggaaaatggggtctgctaaacaacttgtaa

SEQ ID NO: 106 - DNA, 903 bp, Peribacillus Aracenensis
  source 1..903: mol_type = genomic DNA
ttgcatgttgttataacgggaggaagcgggtttgtaggtcaagccttgactcacctgttgactcaaaaaggccatcgagtaaccatattaacgcgtcttcctgatcataaaagtacaagtgaattcgttcattatgttgattggctttctgcagatcatcaacctgaaaacgaacttaaggatgtcgatgcgatggtcaatttagccggggaatcaataaatagcggacggtggatccaaagtaaaaaggaggctattttgaatagccgtcttacagccacaaaagaggtcattcgaattttgagacatcttcatccaaggccaaaagttcttgttaacgcttcaggtgtaagttactacgggatgtcagacttcaaaacgtttaatgagtcctccgaaagtgatgcaaacgattttttggccagtgttgtaaagagctgggagaaagaaggggcaatggcgaaagaattaggcgttcgaacggtcttcgcgcgtttcggcatcattctgggtcaagagggtgcctttccacgaatagtgctaccgtataaattaggtattggggggacaatcggcagtgggatgcaatggatttcctgggtgcacattcaagatgcggttgagatggtttacttcgccataattaattctgaagtagatggaccgttgaatgtgacctcgcctcatccaatacgcatgtcatcatacggacagtccattgcagacgtccttcaccgcccatattggcttcatgttcctggggttgtagtaaaattagtacttggtgaaatgagtcagttggtattaaaagggcagcgggtactccctcaaaaagcactttaccacaattactcctttcaatttccaaacgtacaaagtgcacttactgatattctaggctaa

SEQ ID NO: 107 - DNA, 546 bp, Peribacillus Aracenensis
  source 1..546: mol_type = genomic DNA
atgcttgaaactttccgccaatttttcgatcttcatacaattatttggttgtgcccaatcatttttgttttccatgacttagaagagatcataaccattgaatcttccatgaaggcaagtaaaaataggtttcaaaaatcttctttcgtccaactaatattaaatatgagggaaaaactaggttcgaccgctgcccagctttctgtttcggctacatggattttgttgattatttcattcactacagtggtgactgcccatctcacattaaacggagggggctttcttttatatacagctattctcaatttatttattctgcaagcgatcatgcatattgttcagtccatctttttcaaaggctacacacctggcatcataacggcgctattccttctcatcccttactgtcttattgcctatgacagtttgttcgaacacggtctgatagacgggcatttacttattgcaagtctcccggtcagcctgctcatgatcccgatttttcttgttggcaatcttttaggccgttattttattcactaa

SEQ ID NO: 108 - DNA, 1869 bp, Peribacillus Aracenensis
  source 1..1869: mol_type = genomic DNA
atgggacatcgggtaaatgaggaaatgaaccgaatcgtcgatcagttcattagggaccaatcagatgacgggtcctggcaatatccttttgagaccggcatcggaacagactgtcacatgattatcttattgcggacattggagataaatgatgaggcgttcataaaagaactggtggaacgtattgcagggaaacagcagaaagatggttcatggggtttgttttatgatgaaggaaaagggaaccttacgtccactgtggaagcttattatgcccttctttactccggttaccgggatcgggatgacccggatatccaggcagccaggcggtttatccttgccaacggaggggctacagaagtccatatgttttttaaagtcctgttggctttaaccggacagtgcgagtggccgcctttccccattaagattgaagtgctgcttataccggactcctttccaattaatctttttgacttctccatgtttggcagaacgaacatcatcccgttactgattctggccaatttgggttttagcaggagaacgctgcggtctcctgatctctctgatttgtatctcaaaaaagaaaatcgcttttttacagaagatccggaattccgctcggttatcgattcgattcaaaaagggataaaaggcctgaaagactaccccggaaatcttcgcgagttagctttaaatcgcgccgaacaatatatgctggatagaatagaaccggatggcaccttatgtaattatttcggttcaacttccatgatgatttttgccttattggcgaggggatattcgaatacacatccggtgattacccgtgccttgcaaggcttaaaggagatgacctgccggattgatggagaactccactgccaatatgcgacggctacggtctggaacacgacgttaatcagctatgctctgcaagaatccggaatcccttattcatcgaataccgtccagaaggcaaaccgatatatcctctcccggcaacatgtcaaatacggggattgggtcattcatgaaccagacctgttgccgggaggctggggctttgaggacatgaatacaatccatccggatattgacgacacaacggcagcactaagagcgattcgaacgttagccattgaaagggtggattgtcgacaggcatgggatcggggaatcagctggctcatttccatgcaaaacaatgacggtggatgggcggcattcgaaaagaatgtaaataagaaaatattgaacctgttaccgatcgagggcggaaaagatttgttgattgatccgtcgacggttgatttaacgggaaggacattagagtttttcgggaactatacccatttggattttcatcatccaatggtgaaacgcgggattcgttggctgttaaagaatcaagagtcagatggttcttgggtagggcgctggggcgtctatatttatggcgcatgggcggctgtaacgggaatggttgcggttgggatttccccgaagcatcctgccattcagaaggctgtaaactggttaaaagccattcaaaatcaagacggagggtggggggaatcctgtaaaagcgatatcgaaaattgttatgtgccgttgggcgaaagtacccgcacccatacagcatgggcccttgatacacttatctcagccgcggctgaagtcacacctgacattaaacgcggcgcagcttttttagtagatggaaaagaaaaagattgggcaaaggcctacccgaaaggaaggggaatggcgggagccttttatatcaattatcattgttacgaatacgtttttccgttattggccttggcccattatcaaaaattagctgaagggagctaa

SEQ ID NO: 109 - DNA, 1131 bp, Peribacillus Aracenensis
  source 1..1131: mol_type = genomic DNA
ttgcttgattcctattcggatgtaaagaaggatttgaaaaaaaaattaaaaagtaaatcttccggcctcctgccctttttatccgaaaacgataaacaacgcattcactatataagagaacagacaaaacaacataatcaaaacaatgttacacggactcgggcttattataatttttatctcgagcatccagaaatccattgggccctccttggacatatggtatcgaggaacgttggctggaacatgaccgatttaaaaggggatttgctgacaaaacttctgccagaaagagatcagatggcgatttattcttttttggaacgcggcagctggttgatttttcaggatgtgtatccccagtgtttgatttatgacctaagtgtgaaagccaaccaggaaatgttccaccttttacacttttttcacatttccacctttatggaaacgatgtggcgttatttttggaacagcggggattcctacactcttgcgattgcgactgtgataaatgaacaaagttatttggaaaaaagagtgatccaaaatgatcattttaaaaaaaccgtaaccggtacggccagcttcaagttgtatgattttttgcgtttcaatcacattctttttccatactgtgcagagggaaataggcaacgagccttactagccggcgctacctcgcgccatttcacttcacttcacgaacgaattttattcggaaaaagattgtatgcccttctttttcagcgtacaaatatttcagcgggcattttgaaatgggcgaacgatcatccccatacgggttcacgaaaagattattggccagatttgtttaacgatgtaaacgaatttttcccccgttccctttataaacctcgggtcaagaattgtaagttgagaaaaggcgccgccgaccggttgtacagtccactgttaaaatacgcctggccgaatacttctcatgaagatgcggaaggtggtgactggtttgaggattggcatgttctggactatattcataaggaagtcgatgtgaatggagatatattcgggaattattgcaaaacgcttgaaataattgagcttgcggtcatgggaaaggaagcccttctgtttcgggaagaggaataa

SEQ ID NO: 110 - DNA, 357 bp, Peribacillus Aracenensis
  source 1..357: mol_type = genomic DNA
atggaaaacgttaattaccatgatttctttaagaaaaaaatcggaattatatccccagccaaatgggaattttctttcatcataatagtcccgaacaaagcaacaccttcaaatctcaggtatggttttcaccaaaattttgtagctgaagtggattggagaggaaggtgcgagacccctgcgggaaagacgcgtctaggggagaccccgcaggcacaggccgaggaggctcccggaccgcccgcggaaagcgagtgcctggaacggaaatcaacgtccaaaggtacaactcataaaaaaactgaagacaaacttgattttcatcgagtttgtcttcagtctgagcccttcaattga

SEQ ID NO: 111 - DNA, 1194 bp, Peribacillus Aracenensis
  source 1..1194: mol_type = genomic DNA
atgattatcaatcacaatatctcagctctaaacacgcaccgtcaattatcaagtgcaacgaacgctcaatctaaatcaatggaaaaactagcttctggtatgcgtatcaataaagctggtgacgacgcagctggtttagcaatctctgaaaaaatgcgtggacaaatccgcggattggatcaagcttcccgtaactcacaagatgcgatttctttaatccaaactgctgaaggtgcattaaatgaaacgactgatatccttcaacgtatgcgtgaacttgccaaccaatcagcaacagctaccaatacaactaacgaccgcggagagattcaaaaagagattaactctttgacttctgaaattaaccgaatcggcaatactactgagttcaacactcaaaagttattaaacggtgataaaaatggtgcgggttctgccgaagtagttgctgttcagggtgaatattcaataggagttactgatgcagaagctggaattacaatagatgatgttgtaattgctggtgctacaggtgataatgtagctgatttggctgataaaattaacgcagataccactttaaaccttaaatatctagcagcagatgataatgggaaattaaaacttactcaattagcagatgctgaatctgcaagtgctccaaaagttgcgggtgggaatgttacaaccactactgcaggagtagttggtaaagcagctaaggaagcagatgatagcaagagtctaaaattccaaattggtgcaaacgaaaatcaaagcttaacacttgatatcgctgatatgagagcgaaagctttaggtcttactactacaggtacaggagataaacttgcagtaacagacggaacaaacaacacaacgactgaacaagctttagatgtgactactcatgaatctgcagctgcagcaatcacaaaaatccaaggtgcaattgataaagtatcagcagagcgttctaaattaggtgctaaccaaaaccgtttagagcacacgatcaacaacttaggtacttcttctgaaaacctaacggctgctgaatcacgcgttcgtgatacagatatggctaaaacaatgatggagcaaactaaaaactctatcttggcgcaagcatctcaagcaatgctcgcgcaagcaaaccagcaaccccagggcgttcttcaattacttcgttaa

SEQ ID NO: 112 - DNA, 183 bp, Peribacillus Aracenensis
  source 1..183: mol_type = genomic DNA
atgcccatcaagttaacaacgacggatactaatagttggactgtttctacaattgagttggttttaattattagatatagtgaaacatctatcatagggaaacacttaccatcaaggacacattcaagaagaaataaatcaagatctcaaaaacagtgtaaagaagccctttccaccagataa

SEQ ID NO: 113 - DNA, 438 bp, Peribacillus Aracenensis
  source 1..438: mol_type = genomic DNA
atgaattactcatactctgaatggacaaagaaggattgtccatcttccctgcctcctaaaggttgcccatccttgtttcctccaaaaccccctgcccctaagcctgaattgttcctaacaaccaatgaattttgcggcaattttaatctcccatgtggttcttcaaactttacagtatggaatacggaagaagtttctccatcaggtacggtaagtgtattttattcagatggatgttcaggaaatctcaccgtttctgttactgattcatctgggtttactgatacatttgatatccctcctctcaatactatctcccgaacatacagtgatctggttatggttagattgacgtgtccatctggaactggaaatggtatatgttcaggaaaatattgtattactattagttatccgatagatatcctgacagaatga

SEQ ID NO: 114 - DNA, 327 bp, Peribacillus Aracenensis
  source 1..327: mol_type = genomic DNA
atgtgcaattcaaatagttgttgtccttctgcagaaatttttaaagaggaattttgcgggaattttgccggaccattagctgccgaagtagtatggagtgcgccggctggtagttatatagctggaacttttcaacttttcaacgccaattccagtacaggtattgttactgcggcagggaacgcaattccactaatagccttatctgctactccagggaatacggatactcaatctgttaacaatccgacttcctttacgattaccgcagctgcgggtgacagcgggacatactgtatcacgttgtacaagcgtgtgttagcgtaa

SEQ ID NO: 115 - DNA, 1287 bp, Peribacillus Aracenensis
  source 1..1287: mol_type = genomic DNA
atggttaattctaaaagatgtaatcgggcttgttgccctccccgtcaaattatccaagaggaattttgcgggaattttaccggaccattagctgccgaagtagtatggagtgcgttgactggtagttatgtttcgggaacgtttcagattttcaactccgcttccagttccggtactgtaacggcagcaggaacagcaacccctgctattgatttaaatgctgacccagggaatacggatactcaatccgttaacaatccgacttcgtttacgattaccgcagctgagggtgacagtggaacttactgcattactctctttcgcaatctttcccacgtgccaactccacctattccttcttgccgttttcttgtttacgttacaaatgctggtcaaccagttagtggtcaaaatgatacagtatccgtcattgatacggggacaaatacggttactgctactattaacgtgggagatgctcctcttgaaatagccgttacaccggatgggacgcgagcttacgtaccaaatttcttttctgacacggtatcggttattgataccgtgtcagatacggtgattgcaaccattaatgtgggagagggaccacttggtgtagcgatcacgccggatgggtcaactgcttatgtgtcaaatcatggatttgtctcaccgatggttgacacggtgtcggttatagatacggcaacgaatacggtgattgctacgattaccgtcggggacggccctcaaggaatcgcttttacgccagatggaaccattgcttacgtagcaaatgaattggacgatacggtatcggtcattgatacggcgtcgaacacggtgattgataccattaacgtaggggaccgccctagatcgatcgtcatattgccggatgggacaagagcttatgtcacaaatcaaggtgataacacggtatcggtcattgatacggcgtcgaacacggtgatcgataccattaacgtagggatcgctcctgtgggaacagacatcacaccggatgggacccgtgtttatattgtaaataaaggaagtaacacggtgtcggttatagatacgacaacgaatacggtaattaataccattgccgtgggacaatcacctgatcaagtagccattttgcctgatgggacccgtgcttatgtcacaaatcaaggtgatgatacggtatcggtcattgatacgacaacgaatatagtaattgatactgttgccgctggggaagctccaactggtatagcaagcggaacaatctgcgaataa

SEQ ID NO: 116 - DNA, 906 bp, Peribacillus Aracenensis
  source 1..906: mol_type = genomic DNA
atgcatattgagcaattggaatatatcgtagaaatatcagaaaccggttcattttctgttgctgcagaaaaccttcatgtaacccaatccggtatcagtaaatcaatcggaaaacttgaagaggaattagggatcaaaatatttaaccggtcacggtcaggggctttgccaactgaggaaggaaaaactgtaattgaaaaagcgtatgaggtaataatcaaacttcaagaattcaggaaaacagcaaaaatacaatcgagtcaagtgcttgaagatctgaaaatatctgtatatccacttcttatagaatctatatttaaaagcctgtcgtcctttaaagaggacaacccacacatccaaattgaaataaaagaagctccttcacatatcattattgaaaaaatcaaaaaaaaatcggttgatattgggctcacgtatatcactaaacagataatagaggatgaggaattagattctgaggtattattaaatagtaaagcgaaaatatgtgtaagtaaagactccccattggcttctaaagattacttgacgccccaaaatttactcaatcagtctatcattttatatgattcaaaggaaatgagagaggaaatgcataattttttaaaaaattacgggaaaatgaatgtattgtgtgttacaaataacgttaatttgattagacaatttgttgcagaaggatcagtcatttccgctacttctgacatattcttaagaaacaatccttatatatcatctgggaagatcatcccaattgatttattgcaatattccaatacatcaatatccataggatgggtaagattgaaagaaagaatgattacgaaatctactaaaacattcttaaaacatttgaaagatcagttcctaataggtaactattag

SEQ ID NO: 117 - DNA, 471 bp, Peribacillus Aracenensis
  source 1..471: mol_type = genomic DNA
atgaaaattacaaataacatactggcgtctaattatgttgaccccaaggagttgccttgggttccgactggattaggtggtatggaaacaaaattatgtaaggtaaacccaataacaggtcaatatattgtgctttccaaaagccctggaggtgatcaagacgtgcctgcccatcttcatcatggcactgtaattgtctatactattcaaggtaaatggaagtatattgaagatgaatgggtatcaggaccaggggacgttgtatttgaacctgctggttcactgcataggccagtggctatgtctcaagatgaagatataataacatttgttgtcattgatggcgcactggaatttaaagatgaaaacggtaacaccttatttaccagcaattcgcaaacagtattggagaaatatcacgaatattgtgcggaaaacggtatcaaaccggttgatgtaacaatatattaa

SEQ ID NO: 118 - DNA, 240 bp, Peribacillus Aracenensis
  source 1..240: mol_type = genomic DNA
atgccttcaaaaatcgtgtacaagaaagtgcgagatgagtactcaattatatatgtaaatatattaattcaattttatcgtatcagtagcattgcattaattaaatcagaggacgagaaacactgggaatgttcaattttaaaccatatagacaatagaaaaggccaggcgatccctttccaaatccaatataaagaactatacattaggacaagtatactaatttcatttggtaaatag

SEQ ID NO: 119 - DNA, 897 bp, Peribacillus Aracenensis
  source 1..897: mol_type = genomic DNA
atggaatatatggatataaccattgctggtagtggtgttttaggaagtcagattgcctttcaaacggcgtttaagggattcaatgtaacagtatatgatattgatgatgaagcattagaacgtgcaaaggtaagaatcagaaatttagaacagcgttatcaagaagatttaggagctttagaggaagaagtgaattcggcttataatcgcatttctttttgcagtgttttatcgaaagctgtgtccaatgctgacctcttgattgaagccatttctgaagtagttcaaattaaagttgatttttataaggagttagggaaagttgcacctgagaagaccacatttgtgacaaactcctctacattattaccaagccaatttgcggaagcgacaggacgcccagaaaaatttttggctttacattttgcaaatgaaatttggaaaaacaatacggcagaaatcatgaaacacaaggaaaccgacatgaaagtgtttgatgaagtgattgaatttgcaaaagcgattggtatggtggctatacccctatacaaagaacagccaggatatattctaaatactttattagttccgtatttggaggctgctacgtgtttggtgatgaaagggattgctgatcctgaaacggttgataagacttggatgatagcttctggttctcctataggtccgtttggtgcttatgatgttattggttttaatactccatacaatgcccttcttgaaaaagaaaaagctggtgataatcaagctgctgaagttgctgagtggttaaaaacagagtttatcgataaagggaaatttggaaaagaatcaggagaaggattctacaaatatcccaatcctaattacatgaaaccagattttttaaaaagttaa

SEQ ID NO: 120 - DNA, 336 bp, Peribacillus Aracenensis
  source 1..336: mol_type = genomic DNA
ttgggcgcagaatttggagataccagtctgacatgggaagacttaaagtttctccgtgatcacacgaaattaccaatcttgttgaaaggaattcttcaccctggagacgcagaagtggcgttaaactacggcgtggacggtttaatcgtatctaaccatggtgggaggcaggtggatggggcgatagcggcactagatgcgctgccaaaagtgtgtgacgttgcccagggaaaagtttctgtactatttgacagtggcattagacgcggtgcagatatagtaaaggcattggctctgggggcgtctactgttctcctgggaagatcttatgcctaa

SEQ ID NO: 121 - DNA, 762 bp, Peribacillus Aracenensis
  source 1..762: mol_type = genomic DNA
atggtaacaaaaaattttaaagaaccaccgactttcagttctgttgaagaagaacggaaacataccaaacaacgtcttgcagctgcttttcgcttgttctccaaatttggatttgatgaaggcgtagccggtcatttcacggcaagagatccgggagaaaaagattgtttctgggtgaacccgttcggcatgcactttagccaaatcaaggcttctgatctgatcctggttaatcacaatggtgatgtggtagaaggggagaggcctgttaatcgggcagcgttcactattcactcccaagtacattctgcacgtccggatattattgctgcggcccattcgcattccgtatacgggaaaacgtggtcgaccctgggacgtttgctcgaccccatcacgcaggatgcctgtgccttttacaaggatcattcggtgtttgatgattacacaggtgtggtccatgaccttgaggaaggaagacgtataggcaaagcgcttggtcctcataaagcggttatcttgcgtaaccatggtttactcactgttgggaaaacggtagatgagtgtgcatggtggttcatcacaatggaacgttcctgtcaagcgcaactaatggcggaatcagtcggtaatcctgtactcattgacgaacatcatgcagagcgtacaagtaactatgtcggatctccgcaaacgggttggtttcagttccagcctctatggagtcgaatcgtcaaagaacagcctgatttattggaatag

SEQ ID NO: 122 - DNA, 1233 bp, Peribacillus Aracenensis
  source 1..1233: mol_type = genomic DNA
atggtaataaataactggcatcaaaaattagaagacttgtacgatcaaatggtggaatggagaaggtatttccaccaatatcctgagctttcttttgaggaggtagagacaccaaaacttatcgcgaaaattcttactgatttaggaattgaggtaagaactagtgtgggcggccgcggcgttgtcggcatcattcgaggggggaatcctgggaaaacagtggcgctaagagcggattttgatgccctgccgatacaggatgaaaaggatgtaccttataaatctaaagttcccggtgtcatgcatgcctgcggacatgatgggcatacagctacactgcttggtgttgctaaggtattaagtgaggttcgggaagaattgtctggaaatgtcgttttaatccatcagcatgcggaagaaaaggcacctggaggagctgttgagatgatcgccgacggatgtctggagggagtagatgcgatttttggctatcacctggcatcacctgctcccctcggatttgtcggaacaagaaaaggaccggtgatggctgcagcagattcctttgaggtaacgatttatggcaagggcggacacggatctgccccacatgaaacggttgactccatcattgttgcaacacaagtgatcaatcaacttcagctgttggtcagccgtcaagtagatccaataaaaacagccgttctttctgttggttccttccatgctggtgttgctaacaatgtcatttctgacaaggcccattttactgggacggtacggtcctttgatccggaagtcagagattatcttgaaagagagttcaaaacaatcgttgaaggagtttgcactgctcttcacgcaaaggcagagattcgatatgagcgcggatattctcctgttgtcaaccatgacaaagagacagaccttttctttaaagtcgccaaggatctattaggagccgacaaagtggcggaaatgcctccgataacggggggggaagattttggagcttatcttgagcatgtaccaggagcattctttcatgtaggggctgctaatccagatggccgcgaaatgttcacacaccatcatccgaaatttgatatagatgagcgagccttggtgattgctgggaaaacgatgttaagtctgacttaccattatcttaacgaacaccagaaaacgtttcttgatgattcaaaaaatggtttactttcgcaaattcaatag

SEQ ID NO: 123 - DNA, 249 bp, Peribacillus Aracenensis
  source 1..249: mol_type = genomic DNA
atgacttccttaaatcctgttttcactataggtaatcaaataatcgaaggaatcaaactccatttaaaaatgaattcaaaggatgcaaaagaatacgcaatagaaatgttaaacaaagttgggattcccagaacggacgaaatgttgaaggagtacccttatgcattatctggagggatgaggcaaagggtatcttatccatcagtttgtggaagaggtaatcccgggaggggcaatgcccatgattga

SEQ ID NO: 124 - DNA, 1647 bp, Peribacillus Aracenensis
  source 1..1647: mol_type = genomic DNA
atgtttgctgatgttgtatttgtaaatggacaagtcatttccgtcgattcagacaatcggatcctagaagcagttgccgttaaacgtaaccgaattgaagctgtcgggacgaacgaggaaatcaaacattggatcggagagcggaccaaggtgatcgatttacaaggtaggagtcttttgcccggatttatcgattcgcatttgcatctgatcggttatggaagaacaaggttggcgattaattgcaaagacgcttctatccaatcgaatgtagatattatcggtaaattgcaaaggaaggcggtgtctactcctgcgggaagttggatcgtagcaacaggctacaacgaaagggctatgttagaaggacggtatttgacccgccatgagctggatgatgaggtgtcgacggaacacccgattctaattatacgaacatgcggccacattatgattgcgaacagtaaagcgttggaattggcaggcgtaaacgaacagtcggtcgatccggaaggtggagtgttcggtcgggacgagtccaggagattaaacgggctactcgtggaagcagccatggatccggtaaaacatgccatgaatccgacggaacaggacttggccagagcggcggaaatcgcttcgcgcgatttcgtatcgttaggcattacgacaattcatgatgccggtgggttcgagccggtcaatatgcgcatcctgcagcaatcggttcgttctggtcgcttaaaggttcgggtgtatgcaatggtcgttcacgagcctaactttaaccgtatgagacagacgtgcctgtcgactgggctcggcgacgagcggtttcgtatcggtccggcgaaaatttttatagacggcgcctcaagcgtgccgacgcttgcgacgcgtcagccgtatgagaccaatcctgaagacagcggcattctgtattacacgcaagaaaatatgaacgatgctctcatcgcagcccatcgcgacggttatcaaattactgctcacgcccagggtgattgggcgatcgagatgttactgaatacgttcgaagaagcgcttaggcaatatccgcgagacaatcacagacatcgaatcgagcatgcgggtttagcaatgcccgatctcatcgagcgaatggctaaattgggcatagtgaccgttcctaacccgaactttttcaccgagttcggagatatatacattaagcacttcggcgctcgcagggactatttttacccaattggatcctgcttgaaagcgggaattgttgtagcaggtgcctcggacagcccggtctcgaactgcaatccgcttatcggcattcatggggcggtcaacagactgacgccgtccggcacggtagttggggaagagcagaaaatctccgtcatggaagcgattaggatgtacacctggagcggagcctacgcaagcttcgaggaagatcgaaaaggaagcatcgaggtagggaaattagccgatttggttgtgctaaacgaccgaatattagatgtaacaatcgacagtattgatcaattaagggttgaaatgacgatgattgacggggaaatcgtttacgagctggggaaatccccggatgcagatgatgagttggaagaaaccgttaatttcattatgtaa

SEQ ID NO: 125 - DNA, 1215 bp, Peribacillus Aracenensis
  source 1..1215: mol_type = genomic DNA
atgaacaagaaatggtttattttagcactgttattttttggttgggcactcgggaatctcgatcgatttgtcatgagctatgcgattgtcgacatctcggcagatttatctttaaaagcaacaacacaggggtttgttcttagtagtttcttcttaggatacgccattatgcaaatgcccgggggatggctagcggataaatttggttcaaggaaagtaatcacgagttcaatgttattattgtccctatttacaggtctaactggtgctgtaaattcattcatgatgataatagtgattcgcttcttatttggtcttggggaaggtggctttatgccagcgtctacaaaagcaatttcgactgtctttcctgagcaagagcgttctcgggcacaatcgattctactatcaagcggtgggataatagggattttaacaccgatttttgctacctatttaatggtttctattggttggcgctggatgttttttctcatgggaggctccggtatattgtttgtaatactttattttttctactttaaagttccgcacgtgacaacaacagaaacaggacaaccactgcaacaaactgaaaatccgttaaaagttgtacttaaaattccattattgtggagtttgtttttttcgtcttttgcaatttatactatttcttggggacttatttcttggctgccaagttacttatcaaaagagcgaggattagatttagtttcaattggttggattcaaattattccgggcattgcttcatttgtcggtatgttagctgccggttacattatggatttaatgccaaaaggtaaagagaaatatcttggaatcgttattacaggtattatggcaatcctaacgtttttcatgttttctgcttcaagcattgtggtttttatcatttgtgaaactgttgtaagcctgtccggtgcaatagtcattattttattaaatgcactattactaaaaaatatacctactgcagttgctggttctgctatgggctttgttaatgtgggtggccagttagctggttttattgcacctatggtcatcggcttcattgttgacaaatcaggaagcttcgatttagccttctggatgttaatagcggccgctgtattatgtatgattacaatcagcacaattcgtacaaagaaaaaaatagaaaggccagcctttcaagaggcaggattttaa

SEQ ID NO: 126 - DNA, 276 bp, Peribacillus Aracenensis
  source 1..276: mol_type = genomic DNA
gtgaaagaaataattgagcaaaaaaagattcatttcgttcgtgtagcgattacatttggggaaatccggaaattcactttggagaaaaaatcatccaaagcactagctgaagcattaaaacaagaaggcttcactgtagaatatggcgttgcgggactagacactgagtttatcgccttgtatggttcaggacatccaattatcggtattttaggcgaattcgacgcgctttcaagtctaagccaacaaaaggagcaacttcacatgaaccagtag

SEQ ID NO: 127 - DNA, 342 bp, Peribacillus Aracenensis
  source 1..342: mol_type = genomic DNA
ttgtatggattccaagatatcattgttgagtaccgtgagtattcacaagatactgcagaatttgtaacgaagttttctttagagggaacagatcgaaggtttgctagtattggttcaccaaatgttacaacaccagtagggtgcccgccatttaatgattacacagcaaaacacgaattatattttgatgagggcctatctgagaagtttaatttttcaacagatatattccaaccgctgcaagctgtatatgttaaaacaatactaaaaacagcaggggatcaagtacccaccttaagagaaattgagttaccttaccgccatgaagaaataatcgaataa

SEQ ID NO: 128 - DNA, 138 bp, Peribacillus Aracenensis
  source 1..138: mol_type = genomic DNA
atgattaaaacaaaaaagaaaacaattggtgaaatgacaaatagccggatgcgttgggcgtttgacccctccactcgtgttattaaaaacaaaaaaggcaaaggttcttataaccggaaaaaagagcaatcctattag

SEQ ID NO: 129 - DNA, 273 bp, Peribacillus Aracenensis
  source 1..273: mol_type = genomic DNA
atgatgttgggagttccacttcttattgcatgtgttccagggatactggtgatacttttatcttggtggtttaggaaattaaacctctctttatttgtaaggctattaccaggcatattaaccgttataacttcaattattttgttttacattggttttgtgtacattagagggtttgtaggagctggatatggaatactggctttctttttacttccctttgcagttgtagcttcgattattgcaagaaaaaacaaaggtgtgcaaagctag

SEQ ID NO: 130 - DNA, 102 bp, Peribacillus Aracenensis
  source 1..102: mol_type = genomic DNA
atgaagaaaattattgaagttgctatagtgaggaatccaaatgtgttggttgaaaatataagtgaatattatattgctgatagtgtcatttacgatgaatga

SEQ ID NO: 131 - DNA, 774 bp, Peribacillus Aracenensis
  source 1..774: mol_type = genomic DNA
atgaaccaaagtgtaattaaagcacttaagttgctggatttttttttagaagaaaaaaaagagttaacactaagtgaaatagcaacaaaatctgatatgccaaagccatcagcctatcgattccttacctctctggaggtatgtggttttttgataaagacaaagaataccgaacaagatgttcgctaccgtttgggtctaaagctgcttgaattaggtaatatagtctcagaacaattagatttacgtaccattgctttgccctggatgagagaactttgtgctgacattaatgaagctgtacatctggttatactcgatggagatgaagctgtatacatcgaaaaagtagaaagcagccaagcggtacggctgcatacaagggttgggaaacgttctgagttatatatcggttccggtccaaaattgttgcttgcttatttgcccgagacagatcgtgaaactcttctggaaaaaatgacttttactaaattcacgccgtatacaattaaaaataaagaaattctgtataaggaaattgaacaaatacggtgtaatggttattccattagtaagggtgagcaggatgaagaaacaataggtatttcctatcctgtacttgactatacggataaggttgtcgctgcgcttactgtaagtggtccgaatacgagaatgcaggagaaagttgaagaaactattcgaaagaaaacaaaagaaactgccagtcaaatttctcatgaactaggatatatagaaacggacgttctatag

SEQ ID NO: 132 - DNA, 1173 bp, Peribacillus Aracenensis
  source 1..1173: mol_type = genomic DNA
atgtttataaaaccgaagcgtgttaagaatgtccccccttatttgtttaatgagattaataaaaagaaacaaaatttaattgagcaaggagtagaaataattgatttaggcattggatgtccagatctgcctactccacagcacattgtagatcgattaattgaggaaatgaaagacccggataattttaaatatcctggatacagtggttgtctagaattccgaaaagcggtggcccaattttataaagatcgttttaatgttgacttggacccagagacggaaattcttgcactaatcggttcaaaagagggaatctctcattttattactgcatcaattgatccaggggatgttgtattgcttccagacccgggatatcccacatatcgaacggctacttatctggccaatggcattccttatagtatggcgctattaaaagaaaatggatatctaccggattttacatcaattcccttgcaagaagtcgaaaaagcgaagctaatgtttttgaattatccgggaaatccaacggccgctacagcggatttagcttttttccagggagccgtggattttgctcgacgtaatcaaatggtcgttgcacatgatgctgcatatcaaatggttacatttaatggatatacagctccaagcattctgcaggtagaaggcgcaaaggagattgccgttgagtttggttctctttcaaagacatatagcatgacagggtggagaattgggtacgcagtaggaaacaaagaagctcttcaatcgctatcggttgtgaagagtaatatggatacaagccagttccttcccattcaaaaagctgctgccactgcacttgtgtctgaacaatattgcgtagaagattacaatcagatatatatagagcggatggaaggaatgcttgcggcgcttcgggaaataggaattgaatccgatacaccgaaaggaagtttttttatctgggcatctgtaccaaaagggtacacttctagcgaatttgcaaccaaattacttgaagaagccggtgtaattgtaacgcccggcggagcatttggagaatacggagagggatatttcagaatctctttatccgtaccaactgaaagattgtatgaagcaatacatcgaattaaaacaaaagtaacgattactgattag

SEQ ID NO: 133 - DNA, 1662 bp, Peribacillus Aracenensis
  source 1..1662: mol_type = genomic DNA
atgggaaaatcgatgaacggagcacgtgcaattgtagaatgtatgaaactagaaggtgttgagcatgttttctgcgttcccggagaaagttatttacctttaatggatagcatttatgaaacggaaagcattcaattgatttctacacgtcatgaaggcggtgccgcttttatggctgaggcatacgggaaagcgaagcgtaaaccgggtgtcgccatggcgacgcgggcggtaggtggtgccaatttagctattggtattcatactgcttaccaggattccacgcctatggttgttttcttaggccaagtccatagtaaattccggggcagagaagggtttcaagaggtagacttggatcgttttttcggtcacattgccaaatggaccgtggaaattaatgatgtagaacgtatgccagaacttgttcagcgggcgttccgcatcgcaaagagcgggcgaccgggacctgttgtcattgctcttccggaagacgttctcgtagcagaagcggaaatgagctttggacctgttaccccagttccggcaccacgtccaggtacgcaagagatcgtatccgttcaacgactactggaacaatcagagcgtccggttattcttgctggaggaggcgtaattgcagcaaatggagaacaggcgttgcgtaaactggcagaaaaatttgagattccagtaatgtcgtcattccgtcgtcatgatgtgtttcctaatgatcatgcgttgtatgtcggtcactctggacttggcacatttgtgcctatactcgatacgcttcgtcaggctgacctagtgctggcaattggcacacgtttatctgaggttacaacacaggattatagcattctaaaccaggaacagaaattggttcatatcgatattgaagaggagacactcggtaaggtgtatagtccacatgttggtattgttgctgatgcaagggaagcactagaagaattacttgatatgaatgtggacaaaagctggtctaaatgggcaaaagagaggaatgaaatatataagcatgctggagacggagtggacgcggagaaggagcatagtgtagataataaggaaattattcgaattcttcaggaaacacttccagaggatgcaattattacgaatgatgccggtaattttgcaagttggttacacaatttttattcctttaaccgttctaaaacatatattggtccaacatctggtgcgatgggatatggtttaccagcggctttaggtaccaaactggcaaatccagataaaacggtcgtttcattatcaggtgacggtggttttatgatgacgacacaagagttagaaacggcagtccgttacaatattccagtgatcgcacttgtatttaacaatagtatgtatggaacgattcgcatgcatcaagaaatacactatccggagcgagtgatcggaactgagttaagtgatgtgaatttttcttctttaggggctgccctaggagctcaagcttttagggtaacaaaggatgaagaatttaaagatacgcttgagcgtgcacttaaatctaaaggagtaacactcattgaaatcatgacaaatcctgagcgtatttctgtacaagcaaccattaattctatacgtgaaaagtcgacgcaaaaggcctaa

SEQ ID NO: 134 - DNA, 954 bp, Peribacillus Aracenensis
  source 1..954: mol_type = genomic DNA
atgaataaaaaaggtttaatatggcaaattgtcgccgggatggtgttggggcttttattgggatttttgtctaagcaatatggtcaagccgtaaagcctcttggtgagatttttattaacatgattaaaattgttattatccctcttgtattttcagttattgtttcaagtattgccggcatggggaacttgaaacggatgggcaaaataggattcaaaacaatcatttattttgagattttaacgacgatagccctagttgtaggattagttgccactaatttggctcaacctggtgtaggtatcgatagtagccaattggaaaaggccgatattcagcaatatacgcaaacagcagaagacaccaaacctattgacgttttaatcggtattttttcacctaatctttttaaatcattagcggaagggaaaatacttcctgttatattctttgctgtgatgttcggtatcgcgctggcttccacaggagacaaaggaaaaattgtgctgcaatttttccaaggggtttcggaaacgatgtttaatttcgtccaccttgtaatgaagtttgctccgttcggtgtttttgccataatggctaataccgttgcgacctttgggtttaaatctctcattccgttgggcaaattactaatcgttaaccacattacgattatagtatttattgtaattatatttggttccctcgcatggcttttaaaagtaaatttgtggacactgattcgcaacctaaaagaggaattaattattggttacgttactgacagtacggaaaccgtaatgccacagcttatggataaaatgaatcgatttggatgtgatcgctctgtagtatcttttgtcattcctactggatacacatttaatttagacggttcagctttatatcaggcaatggttgttcaagtttatcgcacagttatatggtattga

SEQ ID NO: 135 - DNA, 1389 bp, Peribacillus Aracenensis
  source 1..1389: mol_type = genomic DNA
atgtataaaaaatcactaaccgtactattagctgcgggtatggttctatcaactggtacagtatttgcacaaataaacggggcaacaaatgcccagtctgacactgcttttgataacaaagttatcaaaaaaattagtgcggacaatatgtataatacgattgcctatctatcagagcaaccgagggctgctggtacagaaggtgagctccgtgcagtcaaatacatagaaagtcagtttaagagtcttggttttgaaacaaagattcagccttttcccatctatgatacggtgcaaaatgtaaaagtgaaaattggtgacagtgatttaggaggaacaccgcgtgcccttagcggcagtatcagcggaaaggtaacggccgaacttgttaatgttggaaaagcaaagccagaggaagttggagaaaatgtatctgggaaaattgcactagttgaacgtggggacattacctttgttgaaaaggttcagaatgtcctaaacaaaggagcggttggcgttttaatgtacaacaactcaccatcaggaaataatttcggacaagtatcagcggggcaaaatatacctgctgtagccattacccaagcccaagggttagagttggtcgaacagcttaaaactaaacaaatcacgtccactctggaagtgggaaaagctgaaaggatcgaaaagacatcctacaatgtcatcgcttccctaaaaccaaaagccaataaagataatggtcaaatcgtgactgttggagcccatcatgattctgtcccgggcggccctggtgcaaacgatgatgcttcgggtgtatcagctgtcctggaactggcacggatcctggccaaaacgccaattgacactgaaattcgcttcctcacgttcggatctgaggaaagagggctcgttggatcatcctactatgcagattcccttcccaaagaggatgtagaccgcatggtggctcacttccaaatggatatgataggcggacgtgatgctggcgaggataatcctgcaggcggtttgattatgtataccattgatggaaagaaaaaccttgttacggacctgggctcctcagcaggtgccagaacgatggatgttgcgattccttatgggcagctgggcaggagtgaccaccaaccattccatgagcttggcattccatccgccttgtttatccattcccctgtagagccttggtatcaccagcctacagatacactggataagatatcgaaagaaaaattgcagcaagctgctgaaattgtcggtgccagtgtctaccaaattgcccgtccggaaactccggcattaacaaatgcacatgtagctcctggcaaggtagactatgattttgatgaccgtccggtagattaa

SEQ ID NO: 136 - DNA, 96 bp, Peribacillus Aracenensis
  source 1..96: mol_type = genomic DNA
atgtcgatgaattcagaaagtcttgataaaattattgagatcgatctttctgctcatcagacggtgaaagaaagagccatcattcagataaagtga

SEQ ID NO: 137 - DNA, 213 bp, Peribacillus Aracenensis
  source 1..213: mol_type = genomic DNA
atggagaatgtagtattaacagtgaaaggaatgtcatgtgggcattgtataaattcaattgagggaaatgtaggaaaattaaatggtgttcattttgtaaaagtttacttaaatgaagaaaaagtagaggtatcatataattcaaaaatggtttctttaaagggaattactgacgttatagaagatcaaggttatgatatacaattatattaa

SEQ ID NO: 138 - DNA, 144 bp, Peribacillus Aracenensis
  source 1..144: mol_type = genomic DNA
atggagaatgtaatattagcagtgaaaggcatgtcctgtgggcattgtattcactcaattgaagggaacgtaggaaaaatgaagggagtttattttgttaaggttcacttaaatgaagaaaaagtagaggtatcatttgattag

SEQ ID NO: 139 - DNA, 2421 bp, Peribacillus Aracenensis
  source 1..2421: mol_type = genomic DNA
atgagcgataaaaaagaaacaacacttcaaatagctggaatgacgtgtgctgcctgtgcagtaagaatagaaaaaggtctcaaaaaaatagatggagtagaggatgcaagcgtgaattttgctttagaaaaatcaaaagtaacgtttgacccatccaaatcaagtgttaaccaacttaaagataaagtggaatccttagggtataaagtggttagtgaaaaagcggaatttgatatatctggtatgacatgcgcagcatgtgctaacaggattgaaaaacgtttaaacaaagtagatggaatacaaaatgcaactgtaaacttcgccttggaatcagcccttgtagaatataatcctgatgaggtttcggtcacggatatgaaggatgccattaagaaattgggttatcgattagaacaaaagcaagaaactacaggcgaaaaggttgatcatagacagaaggaaattgagaaacaaacaggtaaattcatattctcttctattttgtccatccctttactttgggcgatggtcagtcattttgaatttacatcttttatttggctaccagagatgttcatgaatccatgggtgcaacttgcactagcgactcctgttcaatttttagttggaggtcagttttacgtaggcgcctttaaagcactaaggaataaaagcgcaaacatggatgttttagttgcacttggaacctctgcagcctatttctatagtgtttatttaagcattttgtcaatagggtccgaagctcacatggttgaattatattttgaaacaagtgctgtgctaattacattaataatattaggtaagttatttgaagcaaaagcaaaagggcgttcatcggaggccataaaaaaacttatgggtctgcaagccaaaacagccacagttctaagagacggtcaagaaatcaatttacccatcgaagaggtaatagctggagatatcgtttatgttaaaccaggtgaaaaggtacctgtagacggagaaatatttgaagggagatctgccctggatgagtcaatgattacaggtgaaagtattcctgttgataagaaagcaggagatttagtaattggctcaaccattaacaaaaacgggtttctgaaggttaaggcaacaaaggtaggaaaggatacagccttagctcaaattatcaaagtagtcgaagaagcacaaggatcaaaagcgcctattcaacgcttagccgatgtcatctcaggaatatttgtcccgattgtagtggggatagcgattattacgtttcttgtgtggtactttgctgtaagtccgggggagtttgcagtagctcttgaaaagttaattgccgtattagttatcgcctgtccatgtgctctaggcctagctactcctacgtccattatggcagggtcaggtcgagcagctgaatatgggattttatttaaaggcggagaacatcttgaaacaactcatcgggtggatacagtgattctggataaaacgggaactgtaacaaaaggaaaaccaacacttacagatgttattctctcaaatgggtttaaagaaaaggaatttttaaagttagtcggtactgcagagagaaattctgaacatccgttagctgaggcgattgttgaggggattaaagaaaaagggattgaactaggcagctcagaacacttcgaagccattcctggctttggaatcgagtctaaagttgaaacaaaatccttgcttatcggaacgcgccggcttatggagaaaaacaacattgatgttggaaacatattagctaacatggaaaacttggaaaagcaaggtaagaccgcaatgctagttgcaattgatcatgaatttgccggtgtgattgctgttgcagatacaattaaagatacttctcaaaaagcgattgagaggttaaaaaatatggggctcgaggttgtaatgattacaggagataacaagcagacagctcaagcgattgcaaatgaagtaggaattgaccacgttatagcagaagtactgcctgaaggaaaggcagaggaagttaaaaagcttcaaaaggatggaaggatagtggcaatggtcggtgatggaattaacgatgctccagcgttagctactgcagatattggcatggccatcggtacaggtacggatgtagcaatggaggctgctgatattaccttaatcagaggagacttaaatagtattgccgatgccatctttatgagtaaaatgacgattcgaaatatcaagcaaaatttattttgggcctttgcttataatgccataggagttccaattgcagcactaggatttctggcaccgtggcttgcaggagtagccatggcattcagttcagtttcagttgttttaaacgcactcagattacaaaggattaagttgaaaggataa

SEQ ID NO: 140 - DNA, 879 bp, Peribacillus Aracenensis
  source 1..879: mol_type = genomic DNA
atgaaacaaaaaaacatgttgacctgggcgatttccgccattgtgtatcttggattagtaattggcggttattccatatatgcaagcttgaacagtaataacgaccactcggatacccatacggcaaaaacaaagggtgccgaggataaagaatctattaatgagcaatcacatatcgataatcatacgagcaaaaaaagtgatggtaaggattcagggcaatcagatcataaagctcattctgaaagtgaagtggtcacaaatataaaatataaagaaggtttaattaccattgatgtgaaggataaaaatcaaaattcacctaatttagaaatatcacatgaaaagattatgcatttaatttttgtaagtgccgacttagaaaattattatcatttacatcctgaggaaaaaggaaatggcgtttatactctgaaattcgacctacctgataactcttataaagcatttgttgatattaaacccaaaaaccttgcctatcaggttagtccggtagggctgcgggtagggaaaagtcatagtgaacataaggaaaacccacttaaggttgatacaaacttaacaaaaacaatcaatgaaaaaacagttgaattaacaactacagagctaggaataaacaaagcagtgacgttaagttttgatacgaaagggattactccagagccctacctgggtgctctagggcatgttgttattttggatgataagggtgagaaatttgttcatgttcatcctacatcagaagaaaaggcactatttgaaacaaagtttgataaacctggaatctacaaagtgtggggagaatttaaaattgatggcaaagtcaatagctatccatttgttatagaggtcaaataa

SEQ ID NO: 141 - DNA, 333 bp, Peribacillus Aracenensis
  source 1..333: mol_type = genomic DNA
atgaacttagatggggttagtaaacatctattaatttgcaacgggaaaacatgcacgaaaaatggagcagaagaagtaacagagactattagggaagaattgaaaaacttagagctgcaaaaggagattcacactacaaaaacattatgtaatgggcaatgcaagcatggtccgatcgctgttctatatccacaaggaacctggtataaagaaatgaataaaacaaaaagtgaagaacttattcgtcaattgaaagaaaatgacactgttcatttaggctctgaactttattaccatgatgggataacattcaagaacaatgagagtgaatga

SEQ ID NO: 142 - DNA, 234 bp, Peribacillus Aracenensis
  source 1..234: mol_type = genomic DNA
atgcaggctcctgtcttaatagaatttagtaagcttctcctaccgattggacacctgatccactctaatatcgacaacatcctacacccagacaacaacggcatttgtgcatacactcacctccatgaaatgaccacaccacgtatttatattcgtggtgccggttttgagcatgcccaggataacataaatagccttataactttatatttgaaatttgtcactcgacattaa

SEQ ID NO: 143 - DNA, 393 bp, Peribacillus Aracenensis
  source 1..393: mol_type = genomic DNA
atgaaaagacctttaggtgtgtctttaattagttatttttatattttaggtgctatttttttattattgacatctattttctatgatcctaatgcaaatcagataggtatagctacaagatttggattatcaaatgtccctgagcaattaataagggtgatagtagctctaacatctttgattgttgtttttggatatatgaggcttaaaaaacggggcttttggatgatgcttgcctatactttgttttttcttttaataagtttctctttatcattaacatacaatcaacaaccctttaccggaaatatgatatggtcgattattgtaattttatatacaatctatgtaaataaatatttttataaagtagctcatgagtcaatgatataa

SEQ ID NO: 144 - DNA, 384 bp, Peribacillus Aracenensis
  source 1..384: mol_type = genomic DNA
atgaagcgtattttattagcggaagatgaggaagtgttacgaatgctagtagttgacactttagaagatgaagattatgaggttgacgaagcagcggatggaatggaggccgtacagcttctcgaaagcaatacgtatgatctaataattcttgattatatgatgcccggatataccggattggaaatcattgaaaaaatccagtcgtctgaaattaaaaaccaagggaaaatcttgatgttatctgcaaaaagccaacaatttgaacaagaaaggatattggaagcgggtgcggattatttcatgtccaaaccatttagtccgttaaaattaatagaaaaaatcgaggtcattttgcatgaaactgaatccttactttactaa

SEQ ID NO: 145 - DNA, 201 bp, Peribacillus Aracenensis
  source 1..201: mol_type = genomic DNA
gtgcgagactcctgcgggagcagagggacaggtgagaccccacaggcgtttagcccccgccccgcggaaagcgagcatctggaggggaaatcaaccacacctctttacttggtgaatagcaacaaatgccgcccggcgttgcaggtgtatccaaacctgctgcaaaaacaggaaaaagagaaattatatcatattttatga

SEQ ID NO: 146 - DNA, 258 bp, Peribacillus Aracenensis
  source 1..258: mol_type = genomic DNA
atgctcaaattactttcgccagttttaccagttgagagattacctgaaggaaagatagattccgaatataagaagctcagtttacaagttttcctcggaaacttcattggaaatgcagcgtatcattcaattcaaaacttttccataggcattccgggcactttattatgcggttatatctcggataaagtttttaaagaacatgagggttgtctttatgccaggtgcattaatcgcagtccttgtatactggtttaa

SEQ ID NO: 147 - DNA, 192 bp, Peribacillus Aracenensis
  source 1..192: mol_type = genomic DNA
atgaatgggtgccaggtggtgaaaagaagttttatatatattttttccttgtttggttgtgcagctttaatcaggggcaagccaatcacaccgagcaagattttaaagagagacaatatggttcgaggagtcttgaaacataaaaaaggagccatggaaaaaccaaggttccttttttatgttaaatcgtaa

SEQ ID NO: 148 - DNA, 216 bp, Peribacillus Aracenensis
  source 1..216: mol_type = genomic DNA
atgatagttgaagatggaagttgtgccatagatattgcttgttggatatatgaggtgtatagtgaccttggatatcccgagaagcaactgaaaacagtaagtaaggttcttgttgagctccctaagttaattaacagctttctgggctatggtgattggggtcagtgcaaactagttaatgacatcaggatacgtttccgccaaagtttagcgtaa

SEQ ID NO: 149 - DNA, 531 bp, Peribacillus Aracenensis
  source 1..531: mol_type = genomic DNA
atgtgttatcacgaggattgttctaagaaaaatcactgcgataatgaacatcaccacgattggtgtaaggaagaatgctgcgataatgaacatcacgagtggtgtaaaaagaaaaaatgctgccataatgaacatcacgagtggtgtaaaaagaaaaatcactgcgatgaggaccatcaccatgattggtgtaagaaaaaatgctgcgataatgagcatcatgattgttgtaaaaaggaaaaacgctgccataatgagcatcacgattgttgtaaaaagaaaaaacactgcgatgaggaccatcaccacgactggtgtaagaaagaatgctgcgataagaaccatcaccatgattggtgtaagaaagaatgctgcgataagaaccatcaccatgattggtgtaagaaaaatcactgcgataatgaacatcacgagtgttgttgtaaaaagaaaaaatgctgcgatgaggaccatcaccacgattgttggaagaagaaacgctgcgatgaggactgttgtggtaattggtag

SEQ ID NO: 150 - DNA, 138 bp, Peribacillus Aracenensis
  source 1..138: mol_type = genomic DNA
atgtctttaaaaatgacatactcaaatcacatccctttaagacttgaatttaaaggaacagcggaagaagtagaatatttaacaatcttatattcttatttagatgaagcccttaatgctagtggtgcaatatggtaa

SEQ ID NO: 151 - DNA, 102 bp, Peribacillus Aracenensis
  source 1..102: mol_type = genomic DNA
atgaaaaggataaaagaaattaatctcttctatccttatcaagcaactcaattactctatcaagtttttgttctatgctattggatttgtttgaccttgtaa

SEQ ID NO: 152 - DNA, 1806 bp, Peribacillus Aracenensis
  source 1..1806: mol_type = genomic DNA
atgttttatgtggtaaaacaatggttttggtatgactggttcttattattcattcgcttaatagtctgtatctcattaattttcgcgataatagaagttcatgaacaattacctttgcctttatggagcaatattgtttggggaatcatcgcattttctgttccttggctctgtctgttatataactataactattatttaattaccgaaatgattttatttggaggaatcatcctctacttaagttattggtttcctgaggcatatctcggattcttgatgcctgcctttatgatcgctgcaaatggtttccaaaattcatatcgttggtcaggtccgatgacagtccttgtcattccaattttaatccttatactatctcatcaagtcattccctggttgccgatcattcacataggattggcctatggttttggattttcatttcatttactaattgtcaatcataagcaaaataaagttattcgtgaacagaatatagttttggaacagtatatgtcccagattgaacggataactcttttagaagaacgaaacaggatggcaaaggaacttcacgatacgatagggcattctaatgtgtcaatcatcatggggttagaatcgttgcgtacttactgctcaaatgctgaaggggaaaaaaaacttgagttattgttggatctgacacgtaaaaacatggatgatatccgcggatacttgcatcaaatggagtcaacaacagaattgcttccactgcacgaagcactgcggcagctcattgatgaatttcaaacaaatgcaggagtgaatgttcattataggattctcggagaagtttatcccataccacggcaagtccacatgacattttatagatgcttgcaggaatcattaaccaatgcagtgcggcatggaggatctacggaaatgagggtcgtgcttcaatttgaaccgaggcagactcgattggaagtgcaagacaacggtcgtgatgtagataacctagaggaaggtttcggtttgacagcgataaaaaagagggcttccaatcttcaaggacaaataaatgtctattccaagagtgaagaaggaacgattgtaacctgcacattgccaagacagatggaatcgccaggtgaagtcattcgattgctaatcgttgatgaccagccctttattcgtgagagcctgcgaactatcttggagaaaaatagagacctttcaattgttggtttggctggagacggagaacaagcgatggagatttgtgagcgggtaaagccacaaatgatgctgatggatattaacatgccgaacatggatggtatcacggcaatgaagttaattaagcagagatggcctgacattcgcatacttattttaacttcttttcaggaaacagaaaaagcgatggaagcactgcggagcggagcggatggttatctgttgaagtccatggatccaagtgaattagctgaaacgatacgccttatttataggggctgtaccatgattgaccaagacatttcgaataaacttttcgaagaggtagaaaagcagcacattcatgagcattcagaggataatcccataaatgatatggaccattatggtttaacaccacgtgaaattgagatattaaagatggtttccaaaggatttcgttataaaacaattgcttcgaaattatatttgtccgatggaacggttaggaactatgcctcaaacgtttatgcgaagctggaagtgcgcaatcgagaagaagccgttcaaaaagcaggggagctaggacttctggaatga

SEQ ID NO: 153 - DNA, 180 bp, Peribacillus Aracenensis
  source 1..180: mol_type = genomic DNA
atgggtgtatatatcaccctatttaaaggaataaacagccaacttggtaaaaagcattttattcaagattcatatgaaacaaatgtccatactaagcaggtgctgttgttacaggaggtattagaaatcttgtctaaaatgaagaggaatgcgggtttattggcgcctaaactatattaa

SEQ ID NO: 154 - DNA, 1623 bp, Peribacillus Aracenensis
  source 1..1623: mol_type = genomic DNA
atgagaaaaagaatgtttggaattattatattaattactttagtttcttctattatattaatgggttgcaatcaattagaatccaatcaatctgatgattcaaatggtgacgttaatcagaagaaaaaggatgagcttgtgatggcatttggttcagagcctgaagcaggttttgatccaacggccggatggggacgttatggctcaccgcttttccaaagtactctactaaaaagagataacaagcttaacattgtaaatgatcttgcaacaagttataaagtcaatgaagatggcaaggtttggacagtgaacatacgtaaggatgtgaaattttcagacggcgaaccattaaccgccgacgatgtagtctttacatttgaaacagctacaaacaatgggtcggtcgttgatcttaatggtatggataaagtggaggcgatcaatgattacaccgtaaaattcacgttaaaagatcctcaatcaacatttgttaattccttagtaggaacaggaatcgttccaaaacatgcttatggcgctgactatgctgaaaatcctatagggtcaggaccttatcagctcgttcaatgggacaaagggcaacagctcattataaaggttaatcctgaatattatggcaaaaagtcgtattttaaaaagattacctttctatttctaaacgaggatgcatcttttgctgctgcacaagcagggaaggtcgatcttgcttatataccagctgcatttagtaaccaggaagtgcctggaatgaggttggaatcggtgaaaacagttgataatcgaggaatcgtctttccatttgtaaaatcaggggactttactgaagatggcttaccaattggtaacgatgtaactgctgatccagcgattcgtcatgcgattaatattgcggtagaccgaaaagcgttagttgatggagtcttagaggggcgtggtacaccagcttatacttcagtggatggccttccttggtggaacccggatacaaccattaaagatgctgattttgacggtgcgcggaaacttttgaaaaaagccggatggaaggatacagatggagatgggattcttgagaaggattctttgaaagctgaattcactctttattacttggcgagtgatgcaatcaggcaatctcttgcaatttctgtggccgatatgatcaagccactgggaatccagattaaagtagaaggaggaagttgggatattattgaaaagaaaatgtattcaaatgcagtcctattaggttgggggagccatgaccctcatgagatgtataacatttatagtagcaaatttgcaggggtagacttttataataccggatattatcaaaataaaacggtggatgaatactttgataaggcccttcttgctacaagtgaaacagaagcaatcgagtattggaaaaaagcacaatgggatggaacaacgggcttaagtgcaaagggtgatgctccatgggcctggttagtgaatattgatcatttgtacttagtgaaagatggacttgatatcggggaacaaagaatccatgtacatgggcatggttggcctgcaacagataacatagttgaatggaaatggtccaactaa

SEQ ID NO: 155 - DNA, 969 bp, Peribacillus Aracenensis
  source 1..969: mol_type = genomic DNA
atggtcacattattgattgccatttgtttaatttcctttctattaataaaaaactctccgattgatccaatccaagcctatatcggagccgatatgttgaaggtgggtcctgagcaacgggagaagatagctgaatattggggtgtggaccaaccagtcatggtgcaattcttgaattggggatctgcggtacttacgggtgatttaggaacttcaatgatatttcgccgcccggtaatggacattatcggtgaacgattcttaaattccctggcactcatgatatcagcctggatattatcagggataattggattttccatgggtgttatagcggccatgaaaaaagggacttggatcgatcgaataataaaatggtactgtttcactcttgcttcaactcctaccttttgggtggggctccttatccttatcgtttttggcgtttggctaagatggtttccgattggaatgggagttccagctggggtccttgcggaaaatgtcacaatgatggatcgaatcatgcaccttattcttccggcaatcacgcttagtatagttggggttgctaatgtggccttgcatactcgccagaagctgattgatgttctttctagtgattatgtcttatttgctagggcgagaggtgaacaaggatttgtcttgttttggagacatggattgcgtaatgttgctttgccggcgattaccttacaattcgcggcttttagtgagttgtttggtggagcagtgctggctgagcaagttttttcatatcccggtttaggacaagctacggtagaagctgggcttaggggagacgtcccccttttattgggattggttatatgtagtacaatatttgtttttgcaggaaatttactggctgatttaagctatcgtttattagatcccagaatgagggaggggagaagttatgattccaggcctcaaaaacaaaaataa

SEQ ID NO: 156 - DNA, 867 bp, Peribacillus Aracenensis
  source 1..867: mol_type = genomic DNA
atgattccaggcctcaaaaacaaaaataaagataatgttaaacgatttgctctaaatcgaaagcagcggacactttatatgatcctaatcttacttgcttttttagtacttgtcatagtaggtggtatctttattgatgaggggagaatcgagacgaatcttaatgagcgaaatgatcccccatcattagctcatccctttggtacggattggttgggtagagatatgtttacacgtacggtaatgggactttccttaagtatgggggttggattgattggagcgatgggaagcgcgtcaattgctctattcttagggatggcagctgcaacaatgggaaaaatggcggatcgtctcatttcatggctcatcgacctatttctgagtgtaccgcatctcgtaacccttattctaatcgcttttacattagggggaggatttaaagggattgtaattggtttaactttaactcattggccaagccttgcccgagtcatccgggcagaggtcatgcaagttcgttcagcagaatatgttcaggtttctcagaaaatggggaaatctcgatggtggatcgctttccatcatattctgccccatgttttcccgcagcttttaattgggttcatgctattgtttcctcatgttattttacatgaggcagctgttacatttataggtttgggattgtctcctcacgagccggcaattggaattattctatcagaatctatgaagtatttatcttcaggtatgtggtggcttgccttttttccagggctatgtttattgattatcgtgagaacgtttgatcagataggagaaaatatccggttgcacttggatcctaatagggctcacgattag

SEQ ID NO: 157 - DNA, 921 bp, Peribacillus Aracenensis
  source 1..921: mol_type = genomic DNA
atgcctattcttgaagtagaaaatttatcagtatcctttaagcaatataatggatttaaaaagcaaaatcataaagttatatcaagtttaaatgtcactcttgaggcaggtgaggttcttgccgttgtaggagcaagtggatcggggaaaagtctgctcgcacatgccattttagggatattgccaagaaatgcgagtattagtggacggattaaatatgcaggagaggatctcaccactgctcggcaaaccgcattaagaggtaaggaaattgcccttgtaccacaatcggtaaactttcttgatccactgatgcgcgttggaaatcaggtccgaacatcagtaaaatccggtgatgctgtatcggtccaacgagaggtctttgagcgctatcacctacggccagaggtggaggatatgtatccatttcaactttctggaggtatggcgaggaggacacttctatcaactgccatggtaagcggggcaaaggtgattattgcggatgagcctactccagggctcgatcccgttgtcataatggaagcattaaataattttagagaggttgcagacaatggttgtgcagtgatgctgatcactcatgatattgaatcgaccctaaatattgctgataaaattgctgtattttattcaggaactacagttgagatagccccggcggagaactttacaggacagggtgaggaactgcgtcatccatatagtaaggctttgtggagagcgttacctcaaaatgattttactccaattccgggtgctcaacctcatccaagttcattgccagcaggatgtttatttgcgccgcgttgcgaaatggcgactcccgtatgccgacaggaacaacctgaaatgcgaggccttcggggcggaatggtgaggtgttttcatgcaacttga

SEQ ID NO: 158 - DNA, 624 bp, Peribacillus Aracenensis
  source 1..624: mol_type = genomic DNA
atgcaacttgaagcaagagatatcggatttcgatatggagatggaccatggttgttccaaggagtcaatttgacgctaaaaccaggggaagtcgtgggtatcaagggccccagtggacaagggaaaacaaccttttgccggatattggcgggttttgaaacacctattgagggagaggtactcttaaatggagcatcattgccactgaacggatatcatcctgttcaaatggtccttcagcatccagagaaggcaatcaatcctaaatggaagatgcataagattcttaatgaaggatatcaacctgataaagcgttgttagaattactggggattgagcaggaatggctagcacgctggcctaacgaactatctggaggagagctgcaacgattttgtgttgcccgtgcattggggcctgatacacgttttttaattgcagatgaaatgacaacaatgcttgacgcaatcacacaagcccaaatttggcaggcactcattgaaattgctaaaaagagagagatgggaattatcgttgtcacccatgaaacgagattaatgcaaagactttgtcagcgtgtgcttgattttaatgattttagtggagataagaataagaaatga

SEQ ID NO: 159 - DNA, 480 bp, Peribacillus Aracenensis
  source 1..480: mol_type = genomic DNA
atgtctgaagataagaatgcaaaacccgaatttgaagattttgaagtggaaacagtatttgagaatcgtgttcatgagcgacatggattcacttttaaggtccaaggcgatgaattcaagggacattttcatgaagatgagatctattggctccacccacatccgaaacaaaagattggggaaagtaaagtaaaagcaattgaatctaccatacattcattaatgcgacactatggcatttcaaaagagattgcagactttgaattaaaaccagcatttgaagaccggttacatgaacgccaacaattttctttgcaagtgcagggaaaggaattcaaaggctttattcacgaaggagaaatccaatggttccatcctcagccaaagcaaaagcttaaggatgatcttattgaggcaattgaaacagaaatccatcaaaaagcagcgaaacaagtaaatgaaaacaaagaaaatatttag

SEQ ID NO: 160 - DNA, 825 bp, Peribacillus Aracenensis
  source 1..825: mol_type = genomic DNA
atgacggattggactggcactttatctctggaactagaagatcggaaaggaaaaaccgtcgcgaaaagggtgtactttcagggtgcactcaaagttatgcggccgatttactttgatgattcagggcaggtttgctattaccttctaaatcccggtggcggctatttagatggcgatcgatacaagatggagatatcagttgatgaaggatccagagttactttaactacgcaatcggcgacaaaagtatacaaaacgccaaaaagccatgcctatcaggaaaccaacatatccttacaaaaaggtagttatttagaataccttccagatccactgatcgcttatgaaaatgctcattataagcaaaaaaatgtggtttatatggaaagcggagcaactttcatttatacggatattcttactcccggctggtccccggggggcaaaaagttcagctataatactattcaattaattaccgaagtttttttggatggagcgcttggtgtgtttgaccatattaaattaatacctgaaaaacaatcgatatcgggtctaggtttcatggaaggctttacccatcttgggtcaatgatcgcaatcagcgaatatacgaacgatgcccttctcgatgaattgtatgaaactattcaaatggaagaaacgagttttaaatttggaatttcaaagttggcagtgcccggccttagcatacgaatccttgcgaactctacccaggtcattgaacgaattttgaatcagtgccataaggtcatcagcgagaagtggaataatcgtacaccaggctcattacgaaaatattaa

SEQ ID NO: 161 - DNA, 612 bp, Peribacillus Aracenensis
  source 1..612: mol_type = genomic DNA
atggaaccaattagaatcggtgttggtggacctgttggagcaggtaaaacaatgcttgtagaaaaattgactcgccatctcgaaaatgaaataaaaatggcagttgtcacaaacgatatttacacaaaagaagacgctaaatttttaatccaaaatggagtacttccagaagatcggatcattggtgtagaaacgggcggctgtccccacactgccattcgagaagatgcttccatgaacttcgccgctatcgatgaattaatcgagcgccacccagacgttgaacttatttttgttgagagtggcggagataatcttgcggctactttcagccccgaactggttgacttctctatttatattattgatgttgcacaaggggaaaaaatcccccgtaaaggcggacaaggtatgatcaaatcagatttgttcatcattaataaaacggaccttgctccttttgtcggtgcaagcctcgaagtaatggcaaaagatacaaaagtattccgtggcgacaaaccattcgtttttacaaacttaaaaaatgatgatggccttcctgaagtaattgactggattaagcagcatgctttattaaaaggtttagattaa

SEQ ID NO: 162 - DNA, 687 bp, Peribacillus Aracenensis
  source 1..687: mol_type = genomic DNA
atgaataatcatattctctctttgtttcagctttgtgactctaatttacctaccggcgccttcagccattctttcggtttggagagctatatacaagaaaatcaagttgtagacaaggagacatttttccagtggctgaaagtgtatttacatgagcagctcatctacacagatgggcttgtctcgagtctcgtttatgaagccctaatgaaagaggatattcaggaaatctggaaattggatcgcctgataactgtccagaacttgccgagggaaacacgggaaggaacgcaaatgatcggggaccgaatgcttaaactcactgaatcactttatgatatgcccatactctcgcattacagagcggaaattaagaaaaagagttcatttggccatccagccattgtatttacgatggcagctcatggacttggggtaacaaaacaagacaccctcctctattatttatattctgccatatccagccaagtacaaaatgcagtccgagccattcctcttggacaaacagcaggccaaacgatcactcacaatttcatacctgaaataacacaagcagcggttagaatcatgcaactgacgaaagacgactttggcattgtttcaccaggtattgagctgtctcaaatgaaacatgagcgtgttaacattcgaatattcatgtcatag

SEQ ID NO: 163 - DNA, 456 bp, Peribacillus Aracenensis
  source 1..456: mol_type = genomic DNA
ttgattattgaaaaaatcgtcactaatttagaaaagatggatactaacgaaattaaaaagcgtcacatagaaaaagtatacttggaaagtgcacatttaatgaagcgcatccaaagggtcaagacggatcacggtaatgaacttggtattcggttaaaagagcctcgagatcttttggctggggatgtattatatatggacgataaaaatatgatcgtcatagatgtgctgtcagatgacttactagttatcagtccccgaagtataaaagaaatgggcacaatcgcccatcaactaggcaaccgtcacctccctgcccaatttgaagaggatgaaatgctggtccaatatgactacttggttgaggaattacttctggaactcggaattccttttaaacgggaggaacgaaaagtgaaacaagcgttccgtcatataggccacagtcatgaataa

SEQ ID NO: 164 - DNA, 1716 bp, Peribacillus Aracenensis
  source 1..1716: mol_type = genomic DNA
atgagttttagaatgtcccgaaagcaatatgctgaaatgtacggaccgactacaggggactctatccgccttgcagacacagatttgtttattcaaattgaaaaggattacactacatatggagaagaagtagtgtttggtggcggtaaagtcattcgggacggtatgggccagcatccccttgccacccgcaaagacgacggtgttgcagataccatcataactaacgtcgtaatcttggattacacaggaatttgtaaagccgatctagccattcgggatggcaaaatttttggtattggtaaaagtggaaacccgctcgttatggacaatgtggatattatcattggcgcatctacagaaatcattgccggtgaaggcctgattgtgactgctggagccatcgatacccacgttcattttatcaatccggaacaagtacaggtcgcactgacgtctggaacgacaacattaatcggcggcggtactggtcctgcagctggatccaaggctactacggttactcccggcgagtggaatattcatcgcatgcttgaagctgcagaaggcctccctattaacattggctttacaggtaaaggtcatgctgcttccattgaacctttaaccgagcaagtgaaagctggagttatcggattaaaagttcatgaagactggggagccacaggttcttctcttgactatgcactaagggtagcagatgaatatgatattcaagttgccctgcacgcagatacattgaatgaaagtggattcatggaaaataccatggccgcagtaaaagaccgagtccttcacatgtaccacaccgaaggggcaggcggtggccatgcacctgatctaatcaaatcggcaggttatcataacattctgccatcatcaacgaaccccaccctcccttataccgtaaatactatcgacgaacaccttgatatggtaatggtttgccatcatttaaatccttcagttccggaagacattgcatttgcagactctagaattagaagggaaacaattgcagcagaagatattcttcacgatatgggcgtatttagcatggtaagctcagatgcccaagcaatgggccgtgtaggagaagtcgtcctacgcacatggcaagttgcagacaaaatgaaaaaacaaagaggcaccatgcaaggagatagcaaatattccgacaataaccgggctaaacgctatattgccaaatacactattaatccagccattacacacgggatttcagagcatgtaggttcaattgaagttggaaaattggctgatttagtcctttggtctccgaagttttttggagtgaagccagaaatggtgcttaaaaacggcttagcggttaccgggttaatgggtgatgcaaatgcttccatcccaactccgcaaccttatattcatcgtccaatgtatgcccagtttgggaaagccttatcaaaaagttcggtgactttcatttctcaagctgcctatgatgctggtgttcatgagaaacttggattacaaaaaatgattttacctgttggcggaatacggaccctgactaagaaagatatgaaattaaatggggaaacacctgatattactgttgatccgcaaacatatgaagtgaaagtaaatggtgagctgctgacatgtgagccggttgataccgttccaatgggtcagcgatatttcctattctga

SEQ ID NO: 165 - DNA, 324 bp, Peribacillus Aracenensis
  source 1..324: mol_type = genomic DNA
atgctgcctggagaatacattttaaaagaagaagagattatttgtaatgaaggaagcactgttttttccatttctgttacaaatacgggagaccgacctgttcaagtcgggtcacactttcatttttacgaagtaaatgaagcactccgttttaatagaaaagaagcttacggtaagagattgaatgtccctgctggagcagctgttcgttttgaacccggagatgaaaaagaaatacaacttattaattttgcaggagagcgtcgtgtatatgggttcaataataaaatagacggcaaattagaaagtgagggtgaatcatga

SEQ ID NO: 166 - DNA, 303 bp, Peribacillus Aracenensis
  source 1..303: mol_type = genomic DNA
atgcatttattgccgcgggaaattgacaagcttatgatagtggtggcagcagaccttgcaaggcgccggaaagataggggattgaaattaaatcaccctgaagcttgtgcgctcatcacttatgaggtattggaaggcgcaagggacgggaaaactgttgctgaacttatggaatacggggctaccattttgacgcaagatgatgtcatggatggaatacctgaaatgattgatgatattcaggttgaagcaactttcccagatggaacgaagttagtgactgtccacagccctataagataa

SEQ ID NO: 167 - DNA, 321 bp, Peribacillus Aracenensis
  source 1..321: mol_type = genomic DNA
atggatgatgcaaaaacgattttagttacaggctacgccaaagttcctaaagcactaccaatgttggacattcacaaacgtgtagggattgttcttgagattaatgaagtaacacatatcatagaaaatgcagatgtcactttcatcgcaaagttgccttgggacttttttaaaaaattaatgataggatatgatttatcccaaggagtcaatccattaattaaaacaattcgtcaatatcatgaatctccatcccgacaagttattattatggctttacaagctgtcgaacaacgatatggagactttcttaaacaatga

SEQ ID NO: 168 - DNA, 189 bp, Peribacillus Aracenensis
  source 1..189: mol_type = genomic DNA
gtgagtttgcactttactcgtgagttcgatgcatttactcgtgagtttgaggcatttactcgtgagtttggcgcatttactcgcgagtttgtgccttttactcgtgagtttgatgcatttactcgtgagtttgatgcatttactcgtgagtttgaggcgtttactcgtgagtttgcgctttactcgtga

SEQ ID NO: 169 - DNA, 477 bp, Peribacillus Aracenensis
  source 1..477: mol_type = genomic DNA
atggctaggcagcttaataagagtgatgctaaaaaatacttaacccctttttataggaaagatctttgcctaaaatcattagcttttttcacttctgctgcctccaaagtattaacacattctcaaattttaacaatgaataaagaatccgtaaacgctccccgccaatgtatgaatgcactccccattagttccaatacttctatttttagcgcatttattagtgaattcacgctgtttactcgtgaattcacgctgtttactcgtgaattcacgctgtttactcgtgagtttgcgctgtttactcgtgagtttttgctgtttactcgtgaattcacactgtttactcgtcaattcacgctgtttactcgtgaattcacgctgtttactcgtgaattcacactgtttactcgtgaattcgcactgtttactcgtgagtttgcgctgtttactcgtgaattcgctgtttactcgtga

SEQ ID NO: 170 - DNA, 1017 bp, Peribacillus Aracenensis
  source 1..1017: mol_type = genomic DNA
gtgacgacaatttacgatattgcgaaaaaagcgaatgtatcaacgatgactgtatcgagagtcattaataataaagggaatatcagtgaaaagacaagggaaaaagttgaagcggtcattaaagagcttaactatataccgaattccgctgcccaaagtttgaatattaaaagaacgaagctgctttcattaatcataaccgatatcacgaacccctttttcacccaggtggcgagaggggccgcggataaagccaatcaaatgggatatcagctcattttatgcaataccgatgaggattacgaaaaagagagcgaatatatcgatgcattgatttcaaaacgggtggatggcgtaatcattgcaccaacaggcgatcaatcgatgaaaaatttaaagaaattaataaaaaacagggttccatttacattgatagataggcaaattcaagatgtttcttgtgatcgggtacttggtgataactatgaaggaacgaaaaagcttcttcagcatctcatcgattttggacacgaacgaatcgctatggttcatggtccgctaacgatctccacttcgaaagagcgttatcaggcctatattgaaacgctgaaaataaatgatttgaccatcaatcactctttcgtcatagagactcattacaaacaggaaaagcaatggaacggtattgacgggttgatgaatgtcccgccctctgagcggccaacggcgatttttgccgccaacaatttcattgccatcaaaattataaaaagtttacgagaaaaacagattaaagtgcctgaagacattgccgtcgtttgctttgacgacttagaattattctcggacttcgatccttttttaaccgtatcttcacagcctgcttacgatttcggatatctaggaacacaattagtgatcgagcgagtggatgaagtcggtcctgccgactatcggacgatcaatttaaagcctgaattggtaatcaggaaatcatctggagctcctattaaataa

SEQ ID NO: 171 - DNA, 867 bp, Peribacillus Aracenensis
  source 1..867: mol_type = genomic DNA
atggtgattgatgcacatcagcatttttggagaattgaccgaggtgattactcttggcttacacatgatatgggagtcctatatcgggattatcttcccgatgatttatcacccttaatgcataagaatgatatttcggggacgatcctggtacaagcggctccaacctatgaagagactctatttctattatccttgtatgaccgccatgactggatatatggcgtggtgggctggcttgacttatctgctccagcattcccggagcaattggattctttgatgaaacgaccgggaattgttggtttacgccctatgttgcaggatttggaagacagtgcctggatcttacaagaacaagtggtggaaaatctgaaacagcttattcgatatgatcttccgctggatttgttgattaatcataaacatatttcaactgttttaacattaatgaaaacgcttccggatttaaaggctgtcatcgaccatatggctaaaccgaatatatcagctggggaattatgcaaatggcaagaagagatgaatgctttgtcacagtttccgaatatgtggtgcaaaatgtcgggtttattgacccaagcggctcctgaaatgtggaagatggatgactttaagccatacatacaacatattgttcgggtattcgggccgaaccgtttacttttcggcagtgattggcctgtatgtttatcagctgggagctatgaagaggcagtggcggtcataaaagggaatttaccggaaactttgacactagctgaaatagatggaatatttcatggaaatgctaaagccttttacaagctaaaggaaaggggagaagaaaatgggcaagctagtttatga

SEQ ID NO: 172 - DNA, 330 bp, Peribacillus Aracenensis
  source 1..330: mol_type = genomic DNA
atgggcaagctagtttatgaacaggacattacaagcatcgtcatgtctgatcaggataatgttgcgacatcattgaaagatgtagaagaaggggaaacattactctatgtcatcaatggtcaaaaagaggcagtggaagcaaagcgttcgattccatttgggcataaaatcgcaatcaaaccgattcagcgatcggcggctgtcatcaaatatggagaagtgatcggtgcagcgacgatggatatcgagcctggtgaacatgtccatgtacataatattgagggaatcagaggaagaggtgataaggcggaaggggagcaaaaacaatga

SEQ ID NO: 173 - DNA, 1164 bp, Peribacillus Aracenensis
  source 1..1164: mol_type = genomic DNA
atgagcatgataaaagggtatcgccgttcaaatgggaaatttggaatccgtaatcatctattgatcattcctaccgtcatttgcgccaatcatgtggccaacagaatccagcaagctgtaccggaatcagtggccattccgcatcagcatggatgcagccagattggtgatgataaagaacgtacacataaactacttggcggaatggggaaaaacccgaacgttggagcggtcctgttaatcagcttgggctgtgaggtgattgatgccaaagtattgaaacaggaaatcgaagaagaaacgggaaaaccagtggagtggctagatatccaagatgcaggcgggacgataaacgcgattaagaaggggactgaagtggcgaaggggttatttctggaactcgaaaaagtgccgcaagtggatgcccccatttcagaattgatagtaggcgtgaaatgcggcggttccgatgctacatccggattgtgcagcaatcccgctttagggaggacggctgatcagctcctgaaaaagggaggtacgatcgtaatgggtgaaaccacggaaatcatcggagctgaacatcttgttgcccaaaaagcagtgagtgaagaagtggcaaataaactatatgcatatgttgatagattcgaaaaagaagtggaacgcatcggggccgatatgcgcggcggaaacccgagcccgggcaacattgagggagggctctcgaccatcgaggaaaaatcgcttggctgcataagtaaagcaggtacagccccattgaacgatgtcttatcatttgcggaagcaatcccgggtaatggctattacttcatggattccccggggaatgacatcgagtgtgtttcaggcatggcggcagccggtgtacatatggtctgctttacgacgggaagagggacaccgacagggaacccaattatcccggtcatcaaaataacgggaaatgaacatacggccatcaagatgatcgataacatcgatatggatacaagccctgtcatgaaaggaaaagaaacgacagaggaagcgggaaatcgcatttacgaaacgatcgttaaaacggcacagggtgagctgacaaaggcggaaattctagggcatcaggaattcagcatcagccggatcagcatcagtctttag

SEQ ID NO: 174 - DNA, 816 bp, Peribacillus Aracenensis
  source 1..816: mol_type = genomic DNA
atgggtaaattgaataatcgaacagcacttgtcacaggaggcagcaggggaatcggtgcagcgattgtcatgagattggctgaggaaggtgccaatgtggctatcaactatacatcaccaggttcatttgaaaaagcgaacgctttaaaagaaaaagtagaatccgagtttcatatccaagcgatcgtcgtgaaagcgaacgttgggttgaaggaagatgtcgatgccatgatcgatgaagtggaaaaagaattgggaacagtggatattttagtgaataatgctggcattgccccgtttgagccttttttgagcctttcggaagaaacatgggatgatacgtatcggaccaatgtgaaatcgatctttttgacgacgcaaagagtggcgaggagaatgattgaaaataaatatggcaagatcatcaatattacatcaacggctagcgtccttgtcacgagtccggtcattccccactatatttcatcgaaagcagctgcctctcatttaacgaaggcattggcggtcgagctaggaaaatacaatatcaatgtgaatgctgtcggcccaagcaccgttgcgacggatatgtgtgaggaatatttggaagatccgcaaattctcgcaaaagagattgaagccaatccgatgaaaagacttgggacggaaaagcaaattggtgattccgtcgtatttttggcttccgatgaagctatgcaaatcaacgggcatctgttaatggtggatggcggtttaacggtgaaagcggcgcagcctgaagatcatatgaatcatgaacaggaggtaacgtcatga

SEQ ID NO: 175 - DNA, 774 bp, Peribacillus Aracenensis
  source 1..774: mol_type = genomic DNA
atgagactgcaaaataaaatcgctgtcatcactggcgggggaagcgggatcggaaaggaatcagcccgtttattcgctagtgaaggcgcatttgtcatcattaccgatattcatgcagaaaatgggcagggcactgtttctgaaataaagaaagctggcgggaaagcggcattttatgaggtggatgtaacgaatccggaagcggttcaatctgcaatctcccaaatcatcgaaacctataagaaaattgatatattgttcaacaatgccggaatctcgaatgtgggcagggtggacgaagtggaaccggatgtgtgggaccgaatcatgagcgtgaatgtgaagggggtatatctgccttctaaatacacgattccttatatgatggaacaaaaaagcggggtcgttatcaatatgtcatcatgtgcagcggaaatgggtctcgtgaaacgcgccgcatactcagcaacgaaaggcgctgtacttgctttgacgaaagcgatgcaagtggactatgcgccttataatattcgggtgaacgctttattgccaggtacgatcctgactccgttcgtcgaagattacttgaaaacttcctatgacgatcctgaggtagccatcggcacgatcaagaaaagacaattgagcggagatttgggcagacctggtgatgtggcaaaagcggcactgttcttagcttcggacgagtctgcgttcatgatgggatcccctttatatatcgatggcggggttgtttttggaaaaaatgcataa

SEQ ID NO: 176 - DNA, 915 bp, Peribacillus Aracenensis
  source 1..915: mol_type = genomic DNA
atgaagttagctacttttataaaaggtgaacagcaaaaactggctgttcacattgaggatcagttaatagatatcgaagaaacggcgaagagaaatgaatggaaccaaatcgtgtcggatgtcatgcaagtgataaatttcagccaatccgaacgggacgaatttgaaaggaagatccatgaggctgtcagagaaggaatggcagctacaatggaagagaaagggctcgcattcggtcccagtgtgacgaagccgcataaaatcatttgcgttggattgaattacaaaagacatgcggatgaaacgaatgcaccatatcctgaagtgccaattttatttaacaagtttgataatacattaacgggccatggatgtgagattgccattccaagcgtaacgaacgagctggactatgaagtggaactcggaatcgtgatcggcaaaaagacaaagaacgtttcggaagaagcggcactgtcccatgtgttcgggtattgtacggtcaacgatttgtcggcaagagatctgcaaatgagaacgccgcaatggctgcttgggaaaacgtgcgatgatttcagccctgttggaccttacttggtaacagcggacgaagtgggaaatccaaacgacctgcagttgaaaacgtacgtaaatgatgaaataaggcagaattcaaatacatccgatatgatcttttcatgcgcggaaatcatcagttatatttccaagcatatgacattggaaccgggtgatcttatattgacaggtacacctgaaggagtggtattgggcttgccggccgaacagcgtgtgtatattcagccaggggatgtggtcaccgttgaaatcgaaaaactgggagcactcacgaacacattcgtgactgaaagcgaagaggccatgacgaatgcttaa

SEQ ID NO: 177 - DNA, 426 bp, Peribacillus Aracenensis
  source 1..426: mol_type = genomic DNA
atgcttaaaggaattccgcccatactttctcctgaattgatgaagatcatgatggagatggggcacggtgatgaaatcgtacttgcagacgggaattacccggctgcaagtcattcaaaccggatcatcaacggtcatggacatggtgtggccgacttcctgcaagcgatattggcgttttttccactcgatacgtatgtcacacatcccgtcatactgatgaaccctgtggaaggcgatgaaaaaagccctgtaatctggaagagttatgaagatataataaaaaaatcgaaccatatccccatcaacatcggaaaactggaacgaatggacttttacgaacgaagtaaagcggcctatgccattatcgcaacaagtgaacgggcacaatatgcgaatctcatattgaaaaaaggtgtactttaa

SEQ ID NO: 178 - DNA, 1341 bp, Peribacillus Aracenensis
  source 1..1341: mol_type = genomic DNA
ttgcaaaaaattccgaatattatgtatgtttatgcgatctttggcggcttggccggactattatatggttttgattccggggccatttctcctgcaatcccattcatcaccgaggagtttggactaagcccgtcaggtcaaggattgatcgtgagtttcctgctattgggggcattgcctgccatagtcctctccacttcactatcaaaggtgcttggaagaaaatcgctcctgattggagcaggcatcacattcatcgtcgggtcgattggctgtgccttcgctacaaatgtaagcgttttaattgcgtcgcgattcatccttggaatcggctgtggaatagccaatatgtgttctcttatttatctggtggaattggctcctcctaaaatcaggggattgatcggtgctttatatcaattaagtgtaaacgtcgggatcttgagtgcttacatagtgggggcttccttctccgctagcggatcttggagaatcatgctcggaatcgggatcattccagcagcaatcttcacatttggaatgcttatctcaccggaaagcccacggtggctcatgactgcaggaaaggaggaccgtgcaaggaaagtcttgatgaaactaaggggaacgaagctggaagtggaagatgaaataaacgatatcaagcattctcttaaacagcaaagcgtagggttcaaacatttagtacaccaatataaaaaaatattgaatatgaatttcattctaacattcttccaggtcttcacgggaatcaatgccgtcgtatactttgccccaatcattttcgacggggttgaaatcaacggatggagcggttccaatatagcaaacttcggaatcgggacggccttggtcgtttccactgccatctcgttattcatcgttgataaactaggcagaaaaacgctgctcatctacagtattggcggtcaggtcctgccgctgatcggattggcactactttcggattatacgatcttcagcatggtttgtgtgttcttatatgtcttcgcattcggaatcggccttggacccgtcttctggctattcattccggaagtgctgccattgcaggcaagagcgatcggaatgggcgtcatcacctttttacaatacacattgaacttccttttttcatacacgttcccgccactgttaagtgtcattggcaataacgtctttctcatttatgcggtcttatcagtggtcgcttgcgtattcatacactataaaactcctgaaacgaaagggaaatcattggaggaaattgaagaatactggcgtgaacaagatttggcaaaggccattaaacctgcttga

SEQ ID NO: 179 - DNA, 132 bp, Peribacillus Aracenensis
  source 1..132: mol_type = genomic DNA
atgaaaccagcagatgttcttaaggaaaataattgtgcaagtttaatgaaagcaatagcagaaaatgattttcaaatggctcaactgcttgatgtattattattcgaggctaactgggaggatgacctatga

SEQ ID NO: 180 - DNA, 285 bp, Peribacillus Aracenensis
  source 1..285: mol_type = genomic DNA
atgaaacagtataaatatcatcatctcaaggatttaggtggagagccttgcaatacgatatctaagattagaagggtgatttggttgaattattctaagttacaagaatttataaaggaatatggtcaaggtgatgattttactggtggagtaagtgaagacaaagtaaaagaaactgaactaaaattacaagtctcattaccggatagctacaagtggtttttaagaaattatggttacggtggactttttggagtgagaatgcccagttattatgtgggataa

SEQ ID NO: 181 - DNA, 153 bp, Peribacillus Aracenensis
  source 1..153: mol_type = genomic DNA
ttgagcacaatgactttatttggtgcgtggttacaggtagctgtcaagaaaggacatcttgaaatggttgcgttgttccgctttacaaagacctttatagaaaattatattaaagtggtagttaaaaataataaaaaccctggaactttttga

SEQ ID NO: 182 - DNA, 693 bp, Peribacillus Aracenensis
  source 1..693: mol_type = genomic DNA
atgtataagatattaattgttgaagatgaaatgcatattgccaatgcattaaaaaaccattttgggaaatacggctatgactgccacattatagtggattttgaaaaggtgctcgatgtttttcaagattttcaaccgcaccttgtcataatggacataaatctcccttactttgacggctattattggtctcgcaaaataagaaaggtatcgaattgtcctatcataattctctcagctaggatgagtgagctggatcaagtgtatggaattgaaaatggggcagatgatttcattacaaagccttttttaatggatgttgtagtggcaaaaataaacggccaaattcgtcgtgtatacggtgaatatgcacaagaatcgcaaactcacattttaaaagagggagacacatctttaaacttggatactgttcgattatatacatcttatggtgaggagctattgactgtaaaggaacttcagctttgtagaatccttcttgaaacattccctaatgttgtcacaaggcaacagttgcttacatctatttgggatgaagaggcgtttgtagaggaaaatacgcttaccgttaatattaaaaggttgagaaagaagctagaagcgattaattcttcgcttgaaattataacaatccggggaattggctatcagttaagggagaaaagcatatga

SEQ ID NO: 183 - DNA, 999 bp, Peribacillus Aracenensis
  source 1..999: mol_type = genomic DNA
atgaagctgtttttacgggatcatttaagctttattatcctatatattatttcatttattagcttgccaattgtcattcagcggctggatggtttggaaaatcattatgcatattttgtctttttatcccttacattcctagccattttcctgttcattcgttatgtacgccgaaaaaaaatgtatctacatttaaatggcaagaatatgacgacagacagccttttgatttaccagccggctgctccaattgaaaaggaatatgcggcacaaatgcaatccatacagtccctcctcctttcaaaagaagccgagcataaagctgtattagatgaacagcaattgttgatttctcatgctgttcatcaaatgaaaacgcccctttctgtcattcaattgctagtacaatccaatcagtcgaaggaaccaggtttacttgtggaatggctaaaagttaaagcagaatgcgataaactgaatttctctttaaatcagctgctgacttatagccgctccacgaaattattagcagatctaaagatagagccgattccattaaaaggtgtcatacaggaagtggttaatgatttaaaggattacttcattgaggaagaaatctttccaaaaattacgatacaagatgacgtatggatctattcggatcgtaaatggacaaaggttgtgatttaccagctattgagtaatgctgtcaaatatggagagaagcaatcttccgttatgattcattatgacaatggtcaactattgatcaaaaacaaaggggaaacgatagctgcaaacgaaataaaccgtgtttttgaattgttttacacaggtacgaaaggccgtactaaggttgaagcgactggtatcgggctttatttagtaaaaaaaattctgtcaacattaaatcatccatacaagttatattccgcccatcatgaaacaacttttatcattgatttttcgggaaatatagaaacggctgccaaaggttag

SEQ ID NO: 184 - DNA, 762 bp, Peribacillus Aracenensis
  source 1..762: mol_type = genomic DNA
atggcaaacacgattttaggcgtaaagcaacttcaaaaagaatacacaggagaaatcacatataaggcattaaaagggatcgattttcatttagctgaaaatgaatttgttgccgtgatgggaccatctggcagtgggaaaacaacattccttaattgcatttccacaattgatcggcctaccaatgggattattaccatcaattccaaaaatccatatgagttaaatgaggatgaattggcaaaatttcgaagaacagaacttggttttgtttttcaagattttaacctggttcatacattaacagtagaagaaaatattttattgccattgacacttgattccatagatgagaaagaaatgaaacagcgtttaacgaatattatcgattttttggggattggagagattttaaaaaagcgtacatttgaaatttcaggaggacagaaacaacgtgtggcgattgcaagagcggtcattcatgaaccaagcttattgctagcagatgagccaactggaaacttagattctaaagccgtaaataatgtgatgggattgtttgaatcgattaacaagtcttttaacacagccatattaatggtgacgcatgatgcttatgttgccagttttgcccagcgtgtcatttttataaaagacggtgttctttttaatgagatacatcggggtaaaagcaaacagcaattttatcaagaaattatggataccctcacgtttttaggcggtggtcggcatgagttttaa

SEQ ID NO: 185 - DNA, 1848 bp, Peribacillus Aracenensis
  source 1..1848: mol_type = genomic DNA
atgagttttaatcatattgtcgtccaaaatattttacgagacaaatcgacgtatatttcttactttttaagcagtgtgttctcgattctcatcttttttcttttttcgacaacagctttccatccgatgatggcggaagttgataccacaagcacactgggaataacaatgatgcttgccagcttctttatttatattttctcatttgtctttatcatttattcgctgtttgcttttttaaaaaagaaaacaaaaacgcttggcgtatttatgatgacgggtgcctccatgaagcaaatccgcaaaatggtttttagagaaaatatgcttgttgccggagcagcaattatcacagcgattgcactcggacttatcatcgcaccgttatttttaatggtggctaaaaggatattacgtgcggatagctttggtatgtatgtacccttacaatccatcatgttaacgattgttttattcggtattttatttattgttgtatcaaaatggatgacacgctttattaaaaaagaagaaatcgtacagctcttaaaatcagatgtgacacaggaaaggctcattgcatcagcaccattgaaactagtgctatccgctattgtcagtgcctttttactcgtgtcaataatcaaggaaatgagttggataaagtcttttgaatcgctcggctatattgctctaattgccagcctattattatccctttatttcataattactcaaggtgcgctgcgggccattcgtctattgcaaagaagaccatcatattttcgaaaaacgaatatgctgtttgtttccaacttaaaggcaaaaggacgttcccatgcgcatatcatataccttttaacggttttactgcttggtgtttttgtatgtacaagcgttctatatagctcctactataatgtgaaggaaaatactgaggccgtatatccttacagcttccaatatatctcccttcctagtaacacatcggaggccgagaaggaagatattacgtttattgaagaaacattaggcaaagaagggaagtatactgccgattattcagccttcaaagccgaggatgaacatcggattggctttatgtccgtttcgaattataatgctcttggtttgcataagccgataaaactaggggataacgagtattatgttgcagccggtaatgagggggtacgtccaaatactgaaatcattcatgattacccgtttggagaacttcattatgccggtctagaagaaaaaaatattttatcaacaggtttacgaaatgcatattttatcgttcctgatgacgtatatgaaaccattgattatccagtttataaagtgtttgcttatgaggcagatcattggacggacaaggtagaagtagctgaaaccattttatcacgggttcatacagagccggatattcgcttaacagcttctaaaattgatttatatgatgcggaaaaatttgtgaagagtatcatgtttttcatcggatttatgttgagtttgatctttttaagcgcagcaatgagtattctttatttctacctgcaaacgtcactcgcagaagaaaaggaaaaatatgcgggcattcgaaaaattggtctttctgttaaagaactatcttctgttgtaacgagggagttggccactttaacttttatcccgtttaccatcgcagctattgttttatttgtagcgatgtttagtatgcgcaactatatttcatctacattctatcaaatgacagcgctcggtgtaggtatatttttactgctatttgttataagttttttcatcattcgacggagttatttaaacaaactggcaaattaa

SEQ ID NO: 186 - DNA, 960 bp, Peribacillus Aracenensis
  source 1..960: mol_type = genomic DNA
atgaaacgaatagatgaattagatttcttgcgtggctttgccctaataggaattattctgattaacattacacaaatgattaactaccttatccctgaacagggaacacttgattatgttgtaagggtcgttttggattatggcgtgggtcagcgatttttcccgattttttctttcttatttggaattggcttttatctgtttctattccgagccaacgcaaatgggaacaatggaagaaaactatttatccgtcggttgctaattttattagctattggatttattcatcatctcttccagccaggggaagcgttacttccttatgccatatgcggctttattttaattccattttataaattcaaacctaaaacaaattttataatcgcagtcattctgttgattccatctctttggatcggctatgtgtttatgatttttacaatgtttttacttggtttatgtgttgggcaattacaagtttttgagagtctaaataggtataaaaagaccattcgccgactgcaattgatagctttggcagctatcccaatatctttatacttgcagtacaggattacatcaaccactggtatgatcgatgtggctggtactgttggcggactcgctgtcagcctgttttatgttacaacgttgacgctacttcttcagcggacaacagtaaaaaaatggctttctcctttgaagaatatagggagaatggcattgacaaattatttaatgcaaactttcttgattatatgcattgactctatatttaatttgaacaatcatgttcatttaacaacattaataatgatttctgcaggaatattaattcttcaaatgatttatagtgccatgtggcttaagcgatttaagatgggtccgatcgagttattatggcgtataggcacatatggaaaagtgcctcagcactacaaaaaaggcgactaa

SEQ ID NO: 187 - DNA, 333 bp, Peribacillus Aracenensis
  source 1..333: mol_type = genomic DNA
atgaaaattattaaatcattagcgatatttagttgtctagcgacttttatgttagtcggttgtggtaaaaaagaagtgatgtatgaaaaagattattatgtgcaaatcgatgaagaagcagaacaaactaataatgaggggcaatatgtttataatgtaaaaggattcgatgagaatgggaaagaaaaggttgtatatttttatgttgaagaaccatacaaaaaaggaacgcttttacgtcttcctagaagtctcgatggatataccggagatcctgaggtgattgaagctgatgatttgtctaaagaggttaaaaagaaattaaatctataa

SEQ ID NO: 188 - DNA, 1830 bp, Peribacillus Aracenensis
  source 1..1830: mol_type = genomic DNA
atgtcgatgatttacgaatctcaaacactagtctctgccatgcaaacgcgtgtcggacaatataaggatcttaaagaacagctcacggaattaaaaaaaggatttaggagtatcgttcatttggatgatgagctgcagggccaaggcgcagaggccattaaaggattttacaaagcacagatcgatgttgtggattcttggctacgtctgatcgatcggcatgttgcctttttaagtggagttcaaggagatacaatcgaagcgaacctgagtgaaaccgtggtcacggtcccttttttagaggaagagctggaaagcgccagtcgaaattccaaggaaatggtcacagcccaaaaaaatgatttgaaaaaaataatggctggaattgatgatatcattcagttagaacccttttccgatgatgcgttctttgagaatatggagaaagctgaaaggaaacggaaccaaacgatagacaaagtaaacgaaatcgatcataggtggacggctgaatatgccaaatcagaagcggaccaagcggcagtgacggcactcatggagcaattgaaagtctccagcacaaggggaggagtagtatcccctctctactttaatgccacagcctataaaaatagtgaagcctatagaaacctggaagtcaggaaaaaagagagcgcgcaatatctgaaggttaagaaagaggaagcggagaatcgccggatcaaggatttgaaggcacaactagaacatgtaacagatccagatgagttcctcaaaatcgccaaaaagatcgggtatgaaaacttagcgcccacccagcagcaatatgtcatgcagctagaatcggctaagcaaacagcagacattgcaaaaggaatcggcgtaggcctttttgatgtaggaaaagacttcgtgacaggagtttgggactttgtcacagaccctggggaaacggtcgaaggtgtagcaaactcaatcatgcacccgattcaaacctataaatatatatcaaaatccatctccgactcatatgaacgggatatggtaaatggcgatgcctattcccggtctcattgggtaacctatgccctcggaacagtcgtcacatcagtagtaggaacaaaaggcgcaggagccgtaacgaaaactggtgtagcgacaaccaaagccgctgcagttaaaggcgttacgaaggcaaaagaactggcctcaattcctaacctattgccatacaatcctaaaaaccaactgtcgttggcagggggtgtaccttataatgtggttaatggtgctggattaaaagaacagttaatttctatggcgaaagtggagtctgagattagtggtaggggaatagttaatcaaggtagtaatttatatagaggggatagtttactacattctcctaaaagacctaatggaataggtaagccttttattgcagagtcaggtaatttggttcctgcaaacccttcgggattgtataaaggacgtcaagttactgttacagagcacattttaggtggttttagaaagggggcaaaatcgaatagcccttataccagttttacgattaacaaaaatataatagaaggttatggggatactttaatagaattagatatctctgcattgagaaaagcaataagaaacggagaagtaaacaatgttgcagtactatctcaaaagcaaattaagaaattaatcaataatgattcttcttctgatttttggaagaaaagagcgttaacttggaccgaaagggataatgaatatttaataagaggagaagttcctagcaagtttataataatttctccaaaggagtga

SEQ ID NO: 189 - DNA, 282 bp, Peribacillus Aracenensis
  source 1..282: mol_type = genomic DNA
atgttcttatatttccgtaatgaatgtttgggtgaaatacagaatgattataaagaaggcctgtggttttatggatctatcatagccaatgaaaatataaaaaaatataaagattttctagcggctcttgttaatgaggagaaagaattcaaggaagatagttttaatgaagattggctgaacgatgataattggtttattattgatgagcatcaaaataaaaagggaatatatttaccggcaatacatgaagatggggagataaattggcggtatagataa

SEQ ID NO: 190 - DNA, 150 bp, Peribacillus Aracenensis
  source 1..150: mol_type = genomic DNA
gtgaaaattgatccagaaaaacaagaattgattaggacatactctttagttgctattgcagcaagccttatagtcattgcctataatataaatgcctacttaggtgatgttgttcaaatgttggccgcacttgtaaacaaagggaattaa

SEQ ID NO: 191 - DNA, 183 bp, Peribacillus Aracenensis
  source 1..183: mol_type = genomic DNA
atgtatagtgtggtcgaaacggcaatggagagcggtttaagtccctatcatcatttccactatttgtatgaatctctaccaaacatagatcttatgaataaagaagagatagataaagttttgccgcggtcatctgatttaccttctatatgcagagtgaaaaatgaaacaaacaaaaagtag

SEQ ID NO: 192 - DNA, 381 bp, Peribacillus Aracenensis
  source 1..381: mol_type = genomic DNA
atgaagcaaatagaacattactttgctactggaggggaatcatttaagccagaaccagaaaagaaagccggggaattgatcgcggaagaattaaaaaccatacgtgaagaaatggcggcacttagggaagaaaataaacaaatgaaagaacagctggataaccaagaaacttttaataaagagtttgttatcccaggtatccaacaaataaaaggtgaagtatctagcattagaggaagtatagaacgcgataaagaactggatgaatccaatagggcagcaaaggaagctaaacaattaatagcagcagccaacgaaaatccggatactaacctggataaacaaaaaaagggcttctttgctcgactttttggaaagtaa

SEQ ID NO: 193 - DNA, 387 bp, Peribacillus Aracenensis
  source 1..387: mol_type = genomic DNA
ttgaataaagtacttttacatctctccagaacacttttaggttttatcttccttattgcaggtctaaacggttattttgtcatttttgactttgaaccatttattgctactagccctgaagcgatggcattattcaaatttgaatatctgttaatatttgaaaagtttttagagatcgtttgtggagttttactattaagtaatcgatttgtcccattagcacttgcaatattgtctccaattgtagccaacattttcttacttcatttgttccttgatcattcgttactcgttttagcagtaatacttgtaatcatgtatagttatttgttgttttgttacagaaaaagctttaaaagtattttggagaaaaagccttctcattaa

SEQ ID NO: 194 - DNA, 555 bp, Peribacillus Aracenensis
  source 1..555: mol_type = genomic DNA
gtgttaatagtaaacaagaacctagaatatcccatcgctatccaagagttaaaagaagaaagacagatgccggaaggtatccaactaaggcaagttaaatatctcaacaatatcgtggagcagggatcatcctttattaaaaaacgaattcgcctgatgcttgggttaaagtccttagggtctgccaaacgaattattgcggggatagaggctatgcacatgatcaaaaaagcagactcttcaaagggagaagtctgtccaaaatcaaaaagaattcatccatcaactgtttggactagttgcttaagaccaggggtcactagaaatcttttgcttttttatattttcttcaagtatttgcaccagaaccctattaatgtagatgttgatatgatccatttttttcggcctttaaaatccattcattttaaatgggaaaatggtaaagttaggaggggattgaagttttctttagaatacggaccctctcttcaatcggttgtacctaccgaatggaaggagggaaatcaaaaaattaatatattaataaattaa

SEQ ID NO: 195 - DNA, 1419 bp, Peribacillus Aracenensis
  source 1..1419: mol_type = genomic DNA
atgaaaaagcacccaatagccaaagtgcaatggaggtgtgtatttttgaatgaaaaaaataataggagtgtaatagaacaaaaaagctttgaatttatatcaatagaggaaaggcagggtgatcctaaacaacttttttttacctggtttggtgcaaatactcatgcattacctatagttactggcgccttagccataacaattgggttggatttttggtgggcgagcttggcgattcttcttggtcatggaattggagcggtggtaatggctctccattccgcacagggaccgaggctgggcatcccacaagttattcaaagcagagcacagtttggttactttggggttatattgcccttactgatagtcttcacgatgtatataggttatggagcaagtaacacgatcataacgggacagggaattcatgaatcattgggcattaaccttaatttgtcaatcacattaagtttactgccaatggtattgttcgcaatttatggtcaaaaattaattcaatatgcaatgaagtattacacgatgatttatattgttatttttattatcataagcctgcttgttataaaaaatgtctcattagagatgctcaatcatggaagtttttctttcaatcaattttttttagtattgtctatttcagtcacttggcaaattacctatggtccttatgtttctgactactcaagatatttccatccggtacatgcaaagaagacatttgttaatacgtatactggcagctttattagctccgcatggttaatgatattaggagctgctatagggtgcatggcagttaatgggactgtcatgtctcaaataaaggatttaggcggaaacttaggttttgttttagcatttttgatagctattggtttaatgctggttaattcgttaaatatttatggagcttgtattgttgccttatcaatcgcaagtaatttcattaaatttaggacgacgataaaattacggatctttaccacaattttagtaggagtcattctagcagtagcagcaaccatcggagcgggaaattttatggtgaatattcaaaactatttaagttttgtccttttctttattgtaccttggagtgtaatcaatttaacagatttctatttacttcgtcgaaattcgtatgatccggaatcatttatgaggaaaaatgattctttcggaaggttgcgtattagttcccttgccatttatcttctctcggtaatttctcaagtgccatttgtaaataatggtgtttatcaggggacaatctctaaatatttaggtggtcttgatgttgcctgggtaatcggtgttttcatttcatttagtctttactattgtttcgagaaattcaaaaaagaatcaaatattgaattaataaatgatatttaa

SEQ ID NO: 196 - DNA, 1731 bp, Peribacillus Aracenensis
  source 1..1731: mol_type = genomic DNA
atggggagcgttcaaccatccataaaaacagaaattgaaaggaagattaaaatgaatagtcaaatgaaccccgctcaaccagctgatattgttctttcaggtaattttgttttctctggattaggggagaagccgaagaaagcttcagttgctattaaaggaaataaaatatttgctgttggcagtgaaaaagaaatggtaccgcttatcggaaaaaaaacaaaaacttataaatttgacaatgagttaataatggcgggctttaatgatttccatattcatttaacactaggtagtttatatgagcattatcctgatctaagcagcgcaacctcagaggaagaagcagtcgatttattaaaacaacactatgaaaaaagcgataataagaagaatcaatggatattaggcttcagatggtaccacttattttgggaaaaaacagaattgccccacagattatccctggataaagtattccccaatcaacccgtttgtctgctgaatgcagatgcccatggagcttggctgaacagcaaaggactagaagtacttggaataaatcgtgaaaccccagatccaccttttggaaaaatcataagagatgaaaacggggagccaacaggagtactggatgaaaccgctcttgggctggctaaaagagcatttgaaattccatatgagcaacgtgtccgtgtttttcaaagttttttaaagatggccgctaaatatggagtgacttctgtgggcgatatgtttcctgtgcctggatttgacatgggggatttggaaatttatgagttattcgaaaaaaaaggagaactttcagtccgaatcgactttttatccactttaaccggagagtttgattatgtaaagaaacttagagataaatattgttcagaaaaattaaatttttctgggctgaaacaatttttggatggcgttcctgctacctacacggcttatttactcggaccatataacgataacccaaatacaatcggtgaaaccttaatgccgcctgaaatagttaaagagtggataactaatgctgataaagaaggatttagaataaggttgcatgcttgtggagatggagctatcagactagctttggacagctatgaagctgctcgaaaaaataatgggataagagactcccgccatacaattgagcatgttgaaacagtctctgccaatgacttagatcgttttgctgaactgggggtaattgcttcaatgcagcctgaacatattgcactgtttgaaacgtttgaagaaaacacctacccttcccgcctggggcctcttcgtgaaccgtattggccgattaaaacattaatgtcccgtaaagcaaatctggcttttggaagtgactttcccattgttaacttaaatcctatgtacggaatatacagagccgttactcgagtgcacaatgatggagagccaaacggaggctggcattcagctgaaataattagcatggctgaagcactgcgtttctatactttaggcggcgcctatggaaactttaaggaaagtaaactaggaacgatagaggtaggtaaattagcggatattgtggtcctcgacaaaaacctgtttgaagtggattcttctgaaataatatcaacaaaagttaatcttaccataatggatggtaaagttgtttatgaaaaagcacccaatagccaaagtgcaatggaggtgtgtatttttgaatga

SEQ ID NO: 197 - DNA, 171 bp, Peribacillus Aracenensis
  source 1..171: mol_type = genomic DNA
atgtattctctttttttattcattggttgtaggattgtagggccttttcaaacaattgattatgtgtattatccaaatgaagacaatgatcaaaatgcatttccagacaataaaatacatatcaattcgacaatccaaaaaccgctggatatggatattctaagccattaa

SEQ ID NO: 198 - DNA, 96 bp, Peribacillus Aracenensis
  source 1..96: mol_type = genomic DNA
atgaaagctgtcacttttcaaggagcaaaagagatacaggtaaaacaagttgaagatccgaaactgcacaaaaggatgaaatcatcgtccgagtga

SEQ ID NO: 199 - DNA, 174 bp, Peribacillus Aracenensis
  source 1..174: mol_type = genomic DNA
gtgacttcaacggctatttgcggatccgatctccatatatatcagggtgctttgtccacgcataaggattatgtcattggccatgaaccgatgggcatcgttgaagaagtgggtccggaagtaacgaaggtgaaaaaaggggacagggttgtcctgccatttaacatttcttga

SEQ ID NO: 200 - DNA, 186 bp, Peribacillus Aracenensis
  source 1..186: mol_type = genomic DNA
atgaaagcagtaggtgcggaaaaattccaagcccaccccggaaaaggtagaatattaatcaaggtgaaagtttttgtgataaatagaacggatattatttcacgagtagggaaatccggttatatggccaatccaatattggtgaatgaagtgtctggggaagtggtggagctaatggcagattga

SEQ ID NO: 201 - DNA, 291 bp, Peribacillus Aracenensis
  source 1..291: mol_type = genomic DNA
atgtttatcgatacaccgttaattcaaattgaattgatcgagccgggcgattcaccgagcacgtggaagcatcaccatgaaaggtatggggaaggcgttcactgtatctcgtttgttgttaaagatatggaagagaaaatgaagatgctagaagaaatgggctatccggtcactcagacaggtaacttttttaacgaaaaaggccgatacgcatatatggacacgacatcgacatataaagtgattattgaactactagaacgtttcgatgtgggaatattctctgtttaa

SEQ ID NO: 202 - DNA, 165 bp, Peribacillus Aracenensis
  source 1..165: mol_type = genomic DNA
atggagaaatgtcataggaaaaatgaaaataaaaagacctgctatagatcgagcaggtataagggtttcagtttaagttggtacggtatcttcatggcacctgatcccattatcctttttggtgttcttgttcagtcaaatggtaagttcgttttgcagctttaa

SEQ ID NO: 203 - DNA, 249 bp, Peribacillus Aracenensis
  source 1..249: mol_type = genomic DNA
atggcgttcggataccacctggtaggtttgtaccacctggagctaatattgattcgcaggaaaaagcggatgcactttcacgagtaccaaagtatagtaaggaatttgcgaatgaagttcaacaagtcaatcaggaattccctgcatcttatcacctgttatttgggaaaaatcgttgctcctgcggaattgcctatgactagtgaaatgcatgctggatcgagttctattcgtaaggactctttatag

SEQ ID NO: 204 - DNA, 243 bp, Peribacillus Aracenensis
  source 1..243: mol_type = genomic DNA
atgaataaagttttgattttcgagagatttagtgactttttgaaaaaaagatggacatcagatcatcaagctactatttcacctaaaagcagtgaaggttcttggaacagtgcagttgtaccagtaaaagctctttttctaattttaacaattactatccatccctccatttttttcagaatattcatttttttcatgagtattttttgtaatatactaattcatgtaaaaggaatattataa

SEQ ID NO: 205 - DNA, 2442 bp, Peribacillus Aracenensis
  source 1..2442: mol_type = genomic DNA
gtggggtatatgactaacaataatcaaccttttaaaggttatcgcctcctggatccatcccatccaaatatcaatgcttgtgttgaaaagttacaaccaccacaaggttgtgacttttttccttttaaatgcaactgtccaacaggagccaccggaccaacgggagccaccggaccaacaggggcaacaggaccaacaggagccaccggaccaacgggagccactggactaacgggagccacgggagaaacgggagccaccggactaacgggagtgactgggccgactggggcaaccggagcagcgggaccaataggagaaacaggaccaacaggagaaacgggagcaactggagcaaccggactaacgggagccaccggaccaacaggggcaaccggagcgacgggagccaccggactaacgggagaaacgggagccaccggactaacgggagtgactgggccgactggggcaaccggagcagcgggaccaacaggggcaataggaccaacaggagcgacgggagaaacgggagccaccggactaacgggagcgactgggtcgactgggtcgactgggtcgactgggccgactggggcaaccggagcagcaggaccaaccggaggaacaggaccaaccggaacaactggagcaacaggagcgactggagcaacaggactaacgggagaaacgggagccaccggaccaacaggagcgacgggagccatgggagaaacgggagccacgggagaaacgggagccaccggactaacgggagcgactgggccgactggggcaaccggagcgacgggagccacgggagaaacgggagccacgggagaaacgggagcgactgggccgactgggccgactggggcaaccggagcagcaggaccaaccggaggaacaggaccaaccggaacaacgggagcaacaggagcgactggagcaacgggagcaacaggagcgactggagcaacaggactaacgggagcgactggagccaccggaggaacaggacccaccggactaacgggagaaacgggagcgactgggccgactgggccgactggggcaaccggagcagcaggaccaactggaggaacaggaccaactggaacaacgggagcaacaggagcgactggagcaacgggagcaacgggagcaacaggagcgacgggagcaacaggactaacgggagcgacgggagccaccggaggaacaggacccaccggactaaccggagcgactggagccaccggagtaacgggagccaccggactaacgggagccacgggagaaacgggagcgactgggccgactgggccgactggggcaaccggagcagcaggaccaaccggaggaacaggaccaactggaacaacgggaacaacgggagcaacaggagcgactggagcaacaggactaacgggagcaacgggagcgacgggagccaccggaggaacaggaccaactggaacaacgggagcaacaggagcgactggagcaacgggagcaacaggagcgactggaggaacaggaccaaccgaaggaacaggaccaactggaacaacgggagcaacaggagcgactggagcaacgggagcaataggagcgactggagcaacaggagcgactggagcaacaggactaacgggagcaacgggagcgacgggagccaccggaggaacaggacccaccggactaaccggagcgactggagcaacaggaccaactgggctgacaggaccaactggaacaacgggagcaacaggagcgacgggagcaacgggagcaacgggaaccacaggaccaacaggagcaacgggagcgacgggagccaccggagtaacgggagcgactgggccgactggggcaacgggagcaacgggaaccacaggaccaacaggaccaacgggggcaacaggactaacgggagcaacgggagccaccggagtaacgggagcgactgggccgactggggcaacgggaccaacaggagccaccggaccaacgggtacatccggaatatcaacgtttggatatgtttataaccaatccgtacagaatgtaccagtaaattcagatgtaacgtttgatacaaacggaccacttgttggcattacccatacacctggaacagcgcaaattattcttccgacaacaggtaattattctgtcctttttggggttacgactgtacctggtactggtaaacaatttgctttattccttaatagtgtactggttccgggttcgatatacggtacctctaatactccccaattgaatggaagagtaattgttaccgtaactaccgctccagcgacgctcactctaagaaacttcacatcccaaactggtaccgttactttaaattcaccagaagggggaacagaaccaactgttgacgcttcggtgcacattatgaaattaaattaa

SEQ ID NO: 206 - DNA, 297 bp, Peribacillus Aracenensis
  source 1..297: mol_type = genomic DNA
atgtttgaagcagatataattgatatagatgaattaattcataaaactgattcccttcgagaaattgaaaaaagaattttatccgaactaaagatgtataaacaaactgagtctgtaaaaattgatgaaattctttatatttctgaaaatattcattcactatgggaatacgctaatgatttcgaaagaaaacaaatgatgactaccttgttttcacagttaattattgataccaatgatgaatataaaataggaactggtaaagcacgtaagattatcattgtttcagaaaaatga

SEQ ID NO: 207 - DNA, 186 bp, Peribacillus Aracenensis
  source 1..186: mol_type = genomic DNA
atgaatgaaattgtgcatgaagtgtgggaaaggaatgcgggaaatgagggcaacccaaacgcatcagccttttccttatctttgtgcatgacttttttgttttttagagcaggagtcagtcaggcatgtttattaaatcatcgggcaagcatcaaaaaaaaacctatgcattcgccgcatgcatag

SEQ ID NO: 208 - DNA, 105 bp, Peribacillus Aracenensis
  source 1..105: mol_type = genomic DNA
atgcacttatcccgaaccatgattttaaaagaaaaactgaatgttcttttagaaaaaaaccgtactcaaactgactttacttcgaatttgataccttctcaataa

SEQ ID NO: 209 - DNA, 117 bp, Peribacillus Aracenensis
  source 1..117: mol_type = genomic DNA
atgattgttagtcaaacctgggatcatgaagtaattgcaaaattaaatcaaaatgttcacaattgcatgcaaaactatatccgaggtattttaaggaatataatcattgtgcaatga

SEQ ID NO: 210 - DNA, 225 bp, Peribacillus Aracenensis
  source 1..225: mol_type = genomic DNA
atgaaattaaagagcttcatagttacctttggttcatttgtattgacgacaggaatgctttatctggttggtcatatgtttactattccttggttaatgttccatcacgaatataccgagaacggaaacggcttcttcatttcagctggttcgtttgttccactaattatcggtctgattgtatgcttttttgcagaaaagatatatatttacaagttccgataa

SEQ ID NO: 211 - DNA, 138 bp, Peribacillus Aracenensis
  source 1..138: mol_type = genomic DNA
atgtggttagttatttatcaggatttttcagtccttactccaaaagaacatttaaagctctttaatgctattaaagaagattatttccctgagcaggaaaaggacgagatactgctgtcgagttggacaaggtgttag

SEQ ID NO: 212 - DNA, 171 bp, Peribacillus Aracenensis
  source 1..171: mol_type = genomic DNA
atggaagaaataatgctttttatgaaaggaaaaaacaaagtgcgaagcgaaagggacagacaattttcaattggttgtgatagatataatgtaacagatgtggaacaggaaagttcagtgatcagtgaatgcctgtttcacagctatgtaacaaatcagagcttgttttaa

SEQ ID NO: 213 - DNA, 180 bp, Peribacillus Aracenensis
  source 1..180: mol_type = genomic DNA
atgatccaaggacaaaaatatttcgttataaacattgagcaacaatttactgttaaagaacaaaaaaatttcatcatagctgttcttttaatccgtgatattattttacatcaatatggatttcttggtaataggtataacggttgtataaaaagtcagaaaaatataaaatatacttaa

SEQ ID NO: 214 - DNA, 489 bp, Peribacillus Aracenensis
  source 1..489: mol_type = genomic DNA
atggtaaaggcacccatcccttggttgtcactttcttttactaatgaaagcaagaatgtatggaacaaacttacaaaagttattatcttgttgactgctggcacatggcataatgaagccaatacaggtaatattccgctaaaacttgctcgatatatgctcctcctaaccatccatttggtactgttcatgaaactaaagcagatgcagtggcttcggaagagggttacggtccatggcaatagtaatacagttatttctggcaggactccagatgaatggataaagcacaagggatttttggtgaatgaagggttagaggatgttaaaagaggaataaatgctacgcatattcttcaagaattttttctaatgggagttcttgcagggaaaggatattctcccgaaaaagcatgtgaaaaagtagaagaatgggaacgtaccggggaatccaaacttcttcagcaaagcaaaaatatgtataaatag

SEQ ID NO: 215 - DNA, 402 bp, Peribacillus Aracenensis
  source 1..402: mol_type = genomic DNA
atgcaattagaaaacggttttgtaattgaaagtaatccagtgtttggaaagtgtgtgtacaacatttacaccgactatgtgaaaccagatattaagttcacaaatgatagtgttatgctctggtgtgatggctggcaaggtatcaagtttggtaactcaaaagagattatgaaacagggcgttccaagttctactttctataaggaaagaagagaacgaataaaagaggttacaataaaagatttagaaacattcaaagacggttatgttaatgctctgtattactttggagaaggtgagcatgttcgaaagaaagttattgaaacgattatgtcatttgatgatgatgaaaggattaaaccttacataatcaaactactaccaagtggtatccaatgctga

SEQ ID NO: 216 - DNA, 1518 bp, Peribacillus Aracenensis
  source 1..1518: mol_type = genomic DNA
atgtccatacgcatgctaaaagggaaggtgatcaaattgttaagatgtgtaacatcggaaaaagaaactttatatgcttcaagttgtgaagaaagcgcaattaggcaactagctaaagataagaaaatatactgcccaaactgtcaaactaatgtaatttttaaaaaaggaaagataatgagtgcacattttgcacattataattcagagtgtgtagtaacaaattcagaaccagaaactaattctcatataaatggaaaggaaattctattcagttggcttaaacaaaatttcccaacagccgatgttgattctgaagttcatattcccgaaacagggcaaatagcagatgtttttatacaacacagagaaaaaggaatggaaggtttacgatgggcatttgagttccaacacagtccactttcatctacggattgggaaaagagacataacctttatcaatctgaagggattcaagatttttggattttagataaagctacatacatgaaattttcaatagcaaaaggtattacagatgctcgtagaagaaatgaattagaaaaggcaatatataatataacaggcctttgttattttttagatttggaaacgtcagagttgaccattgattttgatttcattacgcgtaccgagaaaaaaatgataaaaggatatgaaagaaaaactgactatacttatcacagcccaatacttcattccagccatatgaatcaaattaaaataagaatgaatgaagaatttaggcatggtgtattaatatataaagatatagaaagtcgaatggaaagaagattatcatggattatacaaaagtttaaaagaaaacagaagttgcaattagaacaagaattccaggaacaagctataaaaaagaagacatttgcaaaagacaaatatggacaagaaacagcagatatatttgctaaatttatagatgataataaagaagaactagatataaaaagtattcaaggaattgatatccctcttggatattatgaactagttgaagatatacgaaatatgcaagatcatgattttttcgataaatataatgatttaatcgaaaagctttcgcttaatttacagttattcgaaaaaataaaagatggtgatgatttaataaataaaataattgggaaaataaattattcatttcaattttataaattatctttcttaattgatcaagactctaagactctacaagattatttaattagtaaagaccaagaaaagattaatttggtgggatatgtatataaagaatataaagaagtattagaaaaactagcttctatgaatcctaaatatataaaaaatgaactgggaaaaataaaatcttccttatctgtatgggaggataacccaactgctttagattatgctatagaatatcatcgacttaaatctaaagatgaaatagacgaatgcattgagcaaattaaagagaagattataaactataatccttttgcgggtgaggattggtaa

SEQ ID NO: 217 - DNA, 264 bp, Peribacillus Aracenensis
  source 1..264: mol_type = genomic DNA
atgctattgcacaaaacagagcaacccttcgaggacgatgatttcataactgagctcaagcttgatggaattcgtttgattctttctaagtttgataatcagattaaattgtatactcgtcacaataatgaagtcacaacgaaattttccgaactgctccagttggatattccgaatggaattattcttgatggtgaaataattgtgactgatcaacaaggtaagcctgattttgaacaggttatctttatcgtaaacaactaa

SEQ ID NO: 218 - DNA, 441 bp, Peribacillus Aracenensis
  source 1..441: mol_type = genomic DNA
atgacgttagaaattttacaagcaaaatttgaattaagagaattggttgatgcttatctcaatttgggagatgaaaaaaagacttcagaacaaatgcttttacttacgcctgatcatcggtatatggtttattttggcgaccaattggtatctgatgtttcaggaagagatgaattggaagagcagttcaaaggtcacgcttctcttgtcaaacgttacttctccactaatgcacaacataatgtacaagtggacggcgatactgcaacaggtgtttcgtactcacagcaaaaaatggtgagagatgaagatggcaaagaagttctcagtgattatagtatcaaatacgaagacacatatgtacgtcaaaacggaacttggttaataaagacacgtattgctcatttcataattatagaaacaagagtattacaaggctaa

SEQ ID NO: 219 - DNA, 678 bp, Peribacillus Aracenensis
  source 1..678: mol_type = genomic DNA
atgaaaaatatcgtgatcgtcggtgcaggttcaggacttggattagcacttgcaaagaaatttggagaaaatggctatcgtgcactattagtatcacgtacgcaagaaaaactagatgcattagctaatgaattacaagcaatcggcatcgaaagtaaaggctatgcagctaacctttacaacgcagaagaagtcaaatctgcttttgatgcaatcaaagcagattacggatttattgatatcgttgaattcagtcctacaattggcggtgtaccaacacctgctacgcaaacaacgtatgaaaatgcactacaacaatttgatggatacgttggcagtgcgattcgtgtagttgaacaagtattacctgatatggtggaaaaaggagaaggagcgattcttttcacaacaggtttatctgcactatatccgattccaatgatgggtaatatcggtattgcactagcaggcttacgcaattatgtaatgaacctgcatactgatgttacagataaaggcgtgtatgttgcacatctttcattaggtatgtttatgaaggctggtacagaaacagatccaagtgtagcagcaaatgcatggtatgagatggtagaagcaagagaagtggcagaagctaaatatcctgcagatgtaacacctgcaactattattttttaa

SEQ ID NO: 220 - DNA, 1059 bp, Peribacillus Aracenensis
  source 1..1059: mol_type = genomic DNA
atggaacaacaaagatcatctccatttgaattcgggatttattcattaggagaaagaataccaaaccaagataaagagactaagtctgcagaagaacgtatatctgaaataataacaatggcgaagttagctgatgaagcaggattagatgtgtttggcatcggtgaacatcatcgttcagattttgtaacctcttcttatgcaatgatattagcagccattgcacgagaaacgaagcagattaaattgacaagtacattatctgtgattagcactgctgatccagtccgtgtatatgaggattttgcaacattggatttattgtctaaagggcgaacagaaatcattgtaggtcgtggagcctttttagaatccttttcattattcggtgctgatttaaataactataatgagttatttgaagaaaagctgaagctctttctggcattgcaagaagaagaaaatattagctggtccggtagattccgttcatcactggaaaatgcaagtatttcaccccgcccatatcaacaaaaactgccattatggataggtgtgggcggcactccagaaagtgcagtacgtgcaggaaaattaggggtgaatatggctcttggtttactaggcggtcaccctgaaagtgtcaaatatttatctgatttatattggaaagctgctcgtgaagctgggcatgaccttgataaactgcgtatatctgtaacaggtcatgcatatatcgcagatactggtgagaaagcaattgatgagttttatcctcattatatgaattattttggacattttatgaaagagagagggcagagattttttgttacaaaggaatctctatactcgcaacgggcagctaatcaaattttagcagttggcagtgcagaagaattaactgaaaagatattatatcagcatgaagtatttggtcacagccgtttcatgggtcaattcgatatgggaggtcaatcactttctagagtagaaaaagcaattgatctactggccaataaagtagcaccaattgttcgccaagctctagcaaagtaa

SEQ ID NO: 221 - DNA, 345 bp, Peribacillus Aracenensis
  source 1..345: mol_type = genomic DNA
atgacaattttaacttggattttacaaggtttattagcattaatgtttatcatggccggaatgggaaaaacttttggttcaaatatgcataaagaggcatttgaacaatggagattgccacaatggtttagagttgtcacgggtattgtagaattgacagcagctatctttttaatcattggtttttggtcaacaaactttgcaattattggagccttaatcattgtatttacctctattggtggagttataacacatttacgagtaaaagatggatttaaagaaacttcaactattctatttcttggaattatagctattgcattgttattcattttaatctaa

SEQ ID NO: 222 - DNA, 645 bp, Peribacillus Aracenensis
  source 1..645: mol_type = genomic DNA
atgaaaataactattttcggagcaaacggagcaatcgggaaaatggtcgttcaagaggcattaactaatggagaccacgtcgttgcatatgttagaagaaataatgcattaacaataacccacgaaaatttagaaataattgtagggaatttggataatgaaacaaaaattgaagaagcaattgttaattcagatacagttatcagtacgctgggaccttcattagataaatccagaaaggtaaaagagttaccgattacttcagcacataaatcaataataacagtaatgaaaagactaaataagaaacgtttcattacattagctacacctactttaaaagccaaagaagatacatcacaattaataacaatcttacctagtataatggcgaaagtcctatttccaactggttatcaggaaatgaagcaaatagaaccaatcataaaaacatcaaatttagattggacagttgttcgtatcatcaaccctaatgtcaaatacacaggtcagacttatgatatatcttttggaaatacaaaaggaaagatgaatgtatcacgagaaaatgttgccaaatgtttatatgatgcagttcgtaataatgcatatattcataaaatgccaatcgtatttaataaataa

SEQ ID NO: 223 - DNA, 636 bp, Peribacillus Aracenensis
  source 1..636: mol_type = genomic DNA
atgtcaataaagaaattgttaattagaggagtaaaacaaaacatggtaaaggaaattgataaacaactaacaaaacgtaagtatcaagcaattaatacaaaaaataatcttttactggccgcaaaaaaattaatgacagaaaaaaggtttgatcagattaccattgatgagattaggaaagaagctgatgtttcaattggtacgttttatcatcatttcaagtcaaaagatgaaatcttttcaatcttattttcaaaaatagacaaagaattgtttgatgactttcatcaaggtaataatgatatgcctgctgaggatatccttattaactattttaatacattggcaattactcttactgaatttggatggccaattgtaaaagaaaaatttttccatgacaatattttttatagtaagaatcaaaaattgagaagtgtattgcttgaaatcatcattgacggtcagtcaaatgggtgtataaaaaaaagaatgccctcagaagaactaactgattatttactgaccatggcaagaggaattgttttagagtggtgttattgggaaggaacctattcattaaaggataaaatgaatttttatatggaagaaatgattcatccttacgtaatgtga

SEQ ID NO: 224 - DNA, 567 bp, Peribacillus Aracenensis
  source 1..567: mol_type = genomic DNA
atgacaattaaaacagatcctcgaataattcgtacccgtaaattaattatggattcctttgttcaactttccatgaaaaaagattttaaaaatattaccatcagcgatattacatcaaaagctacagttaaccgtgcaacattttattatcactttaccgataaatatgacctgttaaacaaggtgctaaaagaagatttaatgacaaaagtattaaaagagattgagaagcatgaaaaggtaaatcataaaacaattacgagcatttttctatctataatttccttccaaagttctttatcttcacagtgcaaaaaaagttttgaagcctttagtacaactatcgagaatgtaattaaaaaagaattggaaaaagtattttatcaaatgttgatgaaagaaacctcttctgaaaatgaagaggtagtaagggcaggatctgttatgttaagctggggaatttatggagcatcaatagactggcagcataatagtagtatgagtcccgaagaatatataaatatgatgatgccttcgttaattagtggagtagacaagttgaattga

SEQ ID NO: 225 - DNA, 624 bp, Peribacillus Aracenensis
  source 1..624: mol_type = genomic DNA
atgaaaactcaaggcatcaaaaaaattacgccaaaactacatcatattggtttgactacagggcgtttcgaagaaatggtagattggtataaaaacgtattagaaatggagccagttcattattcggagaatccagctggggatattggagtggaagtaaaaggtgtttgggtaacgaatgatgaagctaaccatcgtatagccatcatgggaattccaggattagtaaatgatgagaacagaagtaaacattctcgacttcaacatatggcttttgagtatgacacactagatgatctattagatacgtatgtacgtttaaagaaaattggtattaaacctcatttaacagcagatcaaggtgttagtattgctttttattatgatgatcccgatggtaacaccgttgaattaacaatggatacttttggagattggaataaatcaacagaatatatgaaaaattcatcaatctttgcgaaaaaacctatggggaaatatgttgacgttgaaaagcttttggaagcacgtgaacaaggtatttcctctaatgaaattcacgaacgtgcatatgccggtgaatatgaacctgatactcccatggatccaacaaaaatgctttaa

SEQ ID NO: 226 - DNA, 765 bp, Peribacillus Aracenensis
  source 1..765: mol_type = genomic DNA
atgacaaaaacatttcaaaacaaagtagctttaattacaggtgcaaccggaggaattggaaaagagacagctttaacactcgcagaacgtggtgtaaaggttgttattagcggtcgtcgtcgagaattagggaaccaagtagttgacgaaattatagtgaaaggcggagaggcgttgtttgtgacttctgacattggaaatgaacaagaggtacaagaacttatcaagaaaactgtttctcactttggaaagttagatattcttgttaataatgcaggaatctatttagagacggtaccagtagctcaagcagatggagagcttttcgaaaaaatgttacaaacaaatgtgatgggtgttttctatacaatgaagtatgcaattcagcaaatgcaagaacaaggacatggtggagcaattgttaacttagcatctactgctggcttaaacggtatcccttacggaggaccttatgctgctacgaaacatgctgtcgtaggtttaacaaaatcagctgcaatcgaatatgcaccagaaaatatacgtgtaaatgcagtagctccaggagccattaagacggatagcattgcgcaatttattgaacaaggtacctatgatgaaaatatgattattcaaatgcatccaatgatgcgtatgggccgtcctcaagaaattgcggatgctattgtttggttaagttcagatgaggcatcttttgccacaggaacgattttaaacgttgatggcggattcactgctaaataa

SEQ ID NO: 227 - DNA, 924 bp, Peribacillus Aracenensis
  source 1..924: mol_type = genomic DNA
atgaaagctatattaatgaaagaatatggaaatgaagacgtactattagaaacggaagtagaactacctgctgttggtgaagaagaagtacttgtagaagtcaaagcattttcaattaatcacgtggatatcgtaactcgtgaaggtgattttaaagcttttggacccttgaccttccctcatttattaggtttagattttgtcggggtagtaaaagaagtaggagcattatgtcagtccatcaaaataggggatctcgttacgggtattaactatggaggtacctatgctgaatatattacgattgctgagcaagctgtcgtgaaactaattcaagacgtcaatgtgaaagaaactgcagcttttcctgtaatagcagtaacggcatgggcagcagtaatggatcatgggttagtaaaaccaaatcaaaaagtactcattcatggtggtgctggtggtgttggacatattgccattcaattagctaaacaagcaggagcttatgtatatacaacaggagcagagcgtaatacagcatttttaaagaagctaggtgcagatgaagtcattaactacgcaacaactgactttacaacagtagcaactgatgtggacgtcgtaattgatacaattggtggtgacgtacaagagaaaagtttccaatcactaaaacaaggtgggcgtcttatttccgttgtgacaaaaccaagtgaagagctatctgaaaagtatggagtgtattccgactttattcgtggaaatgtgtcgaaggagacaatgataaaactcgtaaatgacttagttgcaggacgtttaacatgtcatgtcgaaaaagaatatccattttcattagatggagttcgtaaagcgcaagtagaattatcacaggggcatactcgcggaaagcgaattgttattatctaa

SEQ ID NO: 228 - DNA, 627 bp, Peribacillus Aracenensis
  source 1..627: mol_type = genomic DNA
atgtcaaaggtattatttgttaaagtaaacgatcgtccattggaccaatcagtaagtgcaaaaatgtatgatgtatttttacagaactatagggtagcaaatggatcagatgagattgttgaattagatctatttaaagaaggtttaccattctatggaaacgacgctattacaggtgtatataaacgtaaccaaggttttgaacttacagctgaagaagagaaagcagctaatttagttgagaaatatttagatcaattcctttcaatggacaaaattgtatttgcatttcctttatggaataaaacagtgccagcaccactaactacgtatctttcatatctgacacaagcaggaagaatgtttaattacactgctgagggtcctgttggatatgctggtgacaaaaaagtaatgatattaaatgctcgtggaggagattattcattagatacgatggctcctgcagaaatggcagtaaatttagtgaaaaatattattaatatctggggaataaaaaatccagaagaagtaattattgaagggcataacatgtatcctgaacgttcgaaagaaatcattactactgggttagagaacgtcataagggcagcttcaaaattctag

SEQ ID NO: 229 - DNA, 618 bp, Peribacillus Aracenensis
  source 1..618: mol_type = genomic DNA
atgacaaataaggatagaatcattcgtccagttttgcaccattatgggctaacaactactcgctttgatgaaatgaagaattggtatgctaaggtaataggtatggttcctacttttgaatcttcagaccctacaggtaatcgagctggaatgaatgctacttgggttactaatgataaggcaaatcatcgtattggtattatagccattccgggtttaacggatgattctgaaaaacatcttcatacaaagattcatcatgtcgcatatgaatattcatcactggatgatttattagatacttatgttagattatcagaaattggaatagaacctgtaatctcacatgatcacggtgcgagcattgccttctattatcgagatccagatcagaacattgtggaattaaatacagatacttttggggactgggaaaagtctactgaattcatgcaaaagtctcctcagtttgcagcacacccaaacggagcaactattgaccctaaacttttggtcgaagctcgagagctaggaatttcttcagcagaaatccataagcgagcttatgctggagagtatgagccatccacacctgcagatccacgtgctctaacgtaa

SEQ ID NO: 230 - DNA, 453 bp, Peribacillus Aracenensis
  source 1..453: mol_type = genomic DNA
atgagtgacaatggtgaaaatcaaaaacagaaacttattgaacatctaaataaagtcacgccagaagaacggatgacccagttaagggaaggaataaaaccttcagaaagcgaactagtgaccatcaaaaaactaaaagttaataatcgtttgcctgacggtgtagtaaatgttttgattgagtatatgctattgaaatttaattctaagtttcctgaccatgtggcaatgaaaattggttcccattgggctagattaaaggtttcaacagtggagcaggctatagacttagctagaaaagagcatagacgatataaagattgggctaattcagtaaaaaaagaaaagaatgaaccccataagattactgaattagagtctattaagggcgcaattaaagctggtttaaatgatgaacagctaggaaggtatgtgagagctttattttcctag

SEQ ID NO: 231 - DNA, 1194 bp, Peribacillus Aracenensis
  source 1..1194: mol_type = genomic DNA
atgaaggacattaaattgtacgaaatcttaaagagtaaacagccgatatttgatgtttatcatcaacctcgtcctgataagcatatttcaatcagttcttctcctgtttttgaccatggcggcaacctgattggcgccatatcggtagatcgtgatataacagctaccgtaaaactaaatgataagctttccgttacaacctcgaagctacaagatttaaaacagcaaatcattaatcaggctaaaaacttaccgttctccagcataaaaggcagcagcaaaattattaatcagataaaggcatccgctattaaagtagcagcaactgacgcaacagtgctgatattaggagaaagcggtgtagggaaggaactttttgcacaggccattcatgagtcaagttctagaaaaaaaaggccatttgttcctattaattgtggtgcgatcccttcccccttgtttgaaagcgaattcttcggctatgaaaaaggttcgtttacaggagctgaacagggtggcaaggcaggaaaactagaagaagcaaatggtggtacactatttttagatgaactaggcacaatgcctttagatatccaggttaaattcttgagaactcttcaagaaggagaaatatatagagtaggtggcacaaaagcaatcaaagtagacataagggtaatagcagctacaaacagcatgctggaggagatggtggaaaaaggggaattcagagaagacttatattatcgtctgaatgtggttccccttcatatcccctcacttcgagagagattagaagatgttccagagctggtacatttatttatagaggagttctctattaaatatcaaaaagaaatacaatttcaatcgaatgatatgatggagttattttcctcataccactggcctggtaacataagagaattaagaaattttgtagagagacttgtggtcatgactgatgacgctgtattgcaagccagtgacatattgaatattcttccgcaaaaggcgaaaaaaatagcgtttgaacatgctactatcacatttcaagatgagataagcttaatagaaaaagaacgaataaaaagtgcattagaaaaaacgcacggtaataagacattggcagctaaggaattaggcttttcaagagtcactctttacaaaaagataaataagtatggactttaa

SEQ ID NO: 232 - DNA, 1011 bp, Peribacillus Aracenensis
  source 1..1011: mol_type = genomic DNA
gtgatgatcaatttttctaaatttattgaaacaatcgatacccacacaatgggtcagccaacaagaattattgtaagtggggttccaaaaatttcaggagatacaatgttagaaaagaaaaataatcttaaaaaagaaataccttggctaagaaatttattaatgaacgagccacgcggtcatcaggatatgtttggggctattctttgtgaaccttctcaagaaggttgtgatgcaggcttaatattcatggacagcggtgattatcttaatatgtgcggtcatggcacaatcggcactattactgcaggtatacagtttggcttgttacctcaaaaggaattgttttttcttgatacaccgtcaggcaaggtggaatgtacagctaaatataaagatcagaaagttagtgaagtgtcgttccggaatgtgccatcttttgttcttgaaaaaaatgtgaatattgttattgaaggctatggaaccatcaaattagatattgtattcggcggcagcatatttgctattgtggacgcgtcacaatttaatttgaaattagaaacaagcgaaacccttgtcttatctaaacttggtatgagaataaaacaaatgcttaatgagcaattttattttgagcatccgcaaaacccaaatatttgcacggtggatcttatagagttcagcttaaaaaaggagaagaatcattatcgcaatgttgttgtttttgggaatggacaaattgaccgttccccatgcggcacaggtacttcagccaaattagcagccctggatcttcaaattggtgaaagtattattcaagaaagtattatcgattccagatttataggtaaggtagttgggaaaacgacagtatcaggtttcgatgctatcattcctgaaattacaggttcagcctgggttaccggattacatcgatttgctttagaagaaaccgatccgtatcaacaaggctttactttaaatcaacagtttgtattggaaaatgcttaa

SEQ ID NO: 233 - DNA, 1566 bp, Peribacillus Aracenensis
  source 1..1566: mol_type = genomic DNA
atgactatgaatgctacattacaagaaaaatataagcacgagccattcaccgattttacgattgaagaaaataaaaatggatttaatcaagcattaaaagttgttcaatcagagaggggtaaaggctaccccttaattatcgggggcgagtcgattacaacagatgaacaaatcatttcgattaacccagcgaataaggaagaagtaattggaagtgtttccaaagcaaataaagagttggctgaaaaggcgatgcaagccgcgctagttgctttcgatacttggaaaaaagaagaccctgaagtacgggcgaatattttatttagtgcagcaaagattctccgtgaacgaaaacatgaattttctgcttacctagtgaaggaggccggaaagccatggaaagaagcggatgcagacacggcagaagcgattgattttctgattttttatggacgccaaatgatgcaactaaaagggggggctcctgtagaaagcagagaaggagaagcaaatacttttaattatattccacttggtgtagggatcattatttccccatttaactttccattggcgattatggctggaactgcggcagcggcaatcgtagcagggaataccattcttttaaagccatcgaataatacacctgtaatagcagctaaatttgtagaactattacaagaagctggccttcctgaaggagtaatcaattacattccaggaagtggtgcagaagtaggtgattaccttgttgatcatcctaaaacccgctttgtatctttcactggttcacgtgaggttggctgccgtatttatgaacgtgccgcaaaagtacagccaggccaaatctggttgaagcgtgtgattgctgaaatgggtggaaaagatactgttgtagtagataaagatgctgatttagatttagcggcatcctcggtcgtgtactcagcatttggattctcggggcaaaaatgttcggctggttcacgcgcggttgtacatcaagatgtctatgacgaagttttagaaaaagcagctgctttaacaaagactttatcaatcggtaatccagaaaacatgaataactacatggggccagttattgatcaagcttcttttaacaagattacaaaatatattgaaattggaaaagaagaaggcaagttgataaccggcggtgaaggggacgactctaaaggctactttatccagccaactatttttgctgatgtggatgaaaaagcacgcattatgcaggaagaaatttttggccctgttttggctttctgtaaagcccgcgattttgatcacatgatggaaatagcgaacaatacggattatgggctaactggagcgttactctcaaataatcctgatcatattgaacgggcaaaagaagaatttcatgtaggaaatctttattttaaccgcggctgcacaggagccattgttggctaccagccatttggcggttttaacatgtcaggaacagattccaaggcaggaggccctgactatcttattttacacatgcaggcaaaaacgattagtgaaacaatttaa

SEQ ID NO: 234 - DNA, 1002 bp, Peribacillus Aracenensis
  source 1..1002: mol_type = genomic DNA
atggaggtcactactttgacaataacaaaagatttttttattatgctttctcaaaataagatgcttaatagcggtgcaaaacgatgggggcttaaacttggtgcccagtctgtcgtagcaggaacgaatattgaagaaatggtgaagagtgttaaagaattgaatgcaaacggaatttctgcaacaatcgataaccttggtgagtttgtatttgaaaaggaagaagccttgcaggcgaaaaccaagattcttgccgttattgaagctatttatgagcatcaattagatgcccatatttccttaaagcctactcagctgggccaggatattgattatagtttctgccttgaaaatctatcggaaattgttgaaaacgcgtacaaatataatgtattcatcaattttgatatggaagatcatggtcatcttcagtcatcatttgatttaattgatgaactttccaaagactatgataatattggaacggttattcaggcttattttcatgatgcgaaagatatgattacaaaatataaaaattaccggttaagaatcgtaaaaggcgcttataaagagtctgaaaatgtcgcatatcaagacaaaaaagatattgatcaaaatttcattgagttaatcgagtatcatctcctgcatggtaaatttacatccattgctacacatgatcaccaaatcattaatcatgtgaaaaagttcgcgaaaaagaataacataccaacagagaaatatgaattccaaatgctttacggattcagaaaggatatgcagttgagtttagccaaggaaggatacaatttttgtacttatgttccgtttggagtggactggtatggatactttatgcgccgtttggcggagcgtccccaaaaccttaacttagtagctaaacagacattcaacaaaaaaacgaaaaccctaatcgggatcggagcgggtgcctttctattaggaagattaagcaagaagaaaccaacgaaagtataa

SEQ ID NO: 235 - DNA, 1362 bp, Peribacillus Aracenensis
  source 1..1362: mol_type = genomic DNA
atggataagaaagtgtccttttcacaagtgctgtctattgggttaatgctctttgccatgtttttaggagcggggaacgttatatttgccccgatgttaggtcaacaggcgggaacaaacacctggcttgccatgggaggttttttgataacaggcgttggactggttttactagctatcattgctctgactcgtggaggtggtacggtagaaaaacttgcaggaagggtccacccacgctttgcaacattcttttcaatgttactttttctaacgttgggacctatttatgttattcccagaacaacttccgttgtttatgaaatcggtttaaatcccttaattcaaagtgtagcaaatgaaaggctgtatctgcttgtattttcagtgttatttattctattgacggttctgctctcctgggatgcaaagaaattggtagataacctgggtaaaattattacccccatcttttcaatattgctggcagtattgattataaaatcatttataacaccgatgggcaaaataggggctcctggagaggaatacatagatggcgttttcttaaaagggtttacgcaaggctactatacaatggatgtactagctgcttttatatttggcggcattttcattaagtcaattggttcgttaggaataaaatctgaaaaagaagtttccaagctatttatcaaagcagggatcataactattattgggttagttgctttacaggtttcaatggcttggatgggtgcttccagtgtagatgcaattgggttaaaagaaaacgggggagaagttttagctgcgagtgctattgctctgtttgggaattatggaatttatatcataggaacaattattttcctcacaggaattacaacaaatgttgcatgcctggcagccgtttctgaatactttgaacgaattgttccgtctattagctataaaaaatggattatagttttttctatcataggaacaatcattacaaactttggattgaatactgtattgacacttgcttctccaatattgctgctgctttatccattggccattgctttgattgctttaatatttgccaataatctatttaaaggttatcggtccgtatatgtgagcactgtagcgggagtcggattggtcgctctgcttgatgctttaaaagaagcgcatatcttaacaaatgcaattaaccatacatttggattcattccattattcgagtatggagttggatggattagcacaggattagtgggctttttgattggactaatagtcgcgaaaactaaacaagaatccagcgtaattattgatatagctggacaagtaactgataaagtttcgtaa

SEQ ID NO: 236 - DNA, 171 bp, Peribacillus Aracenensis
  source 1..171: mol_type = genomic DNA
atggggcaatggtatacagatagaaaaagtgtctgtaataggtttcatttgatcaacggttgttatttttacgtaccggggcagaaaatgaatttttttgaggtatatagtattttaatttggaatgaagaaccgaaaataattaaaaataaaaagcagacggtactttga

SEQ ID NO: 237 - DNA, 1005 bp, Peribacillus Aracenensis
  source 1..1005: mol_type = genomic DNA
gtgactaaagtgaaggcgcaaattattcaatcttttggtgaaccctccgtatttcaatgtaaagagatttcaaaacctgaactaaaacctggacatgtacttattcaagtcaaggctacaagtgtaaatcccattgatacgaaagtccgtgctggtgcagttccagccgttgcccccgagtttccggcagtattacatggagatgttgcaggtttggtagctgcagtaggtgaaggagtaaccgagtttaaaattggcgatgaagtgtttggatgtgcgggaggttttagagggactggcggtgcacttgcagagtttatgcttgcagatgtcgatttacttgctcacaaaccgaaaaatttgacgatggaagaagccgctgctttaccattggttgccattactgcatgggaagcattattcaatcgggcaaatcttgtccctggacaggatatactgatccatgcagcgaccggcggagtaggacacattgccatccaactggcgaaatggggaggggcgacagtctatacaaccgcctcttcgcaggagaagctggagatcggcacgcgtcttggtgcagatgtaacgattaattatcgagaagaaagcgttcacgactatgtacagaaatatacagacggaaaaggatttgacgttgtgtttgacacggtaggaggagaaaaccttgatcgctcctttgaggcggccgcagtacatggaacggtagcagccatcgctgcccgttcgacccatgacctctcctccgtgcatgcaaagggactttctctgcatgttacctttatgttgttaaagatattaaacaaggacatgcataagcattatcgggaaattttgaagaaggttgcccggttggttgaggaagagcagctgcgtccgcttgtggatccaaacatttttacgtttgatgaggtttcaaaagcccatgagtacatggagtccggcaaggcgataggaaaaatagttttgaaaaataattggtaa

SEQ ID NO: 238 - DNA, 627 bp, Peribacillus Aracenensis
  source 1..627: mol_type = genomic DNA
atgcttttaaacgattttatgaatgggaatttcccgaacttagaacttagaccgccgttgttttatagttggaaaacgggcatccgttttgaattaggtgtggactatgatagtgaatttgcttatgaaaatagcccatatctacaaggcgtatataaaagggctatcactttattcaagtccttgcattcttataacgatgatatttatatcgtagttgacgtaaacgattatgccgatggttttaaacataaatcaaacactttttcacggtatattaaggagaagtcgatcttataccggttaaaccaaaagacaacccttcatgacgatgatgaagaaggaacatataaaacacatagatttacgttaaagtgcagaacgtctgacttcaaatacattcctatgctaaaagcaatctgtaatcaagatatgggaataaagccaagtatatttaatagggtctattttataaacatcaacaggaaaactatatttcacgtgtatgatgacaggggttgtgatttattggcgacttcacccgaaacgataagagatgtttatgataaatttaacgactggatattagattatgacagaaatgaaatagacgaagtattcaaataa

SEQ ID NO: 239 - DNA, 570 bp, Peribacillus Aracenensis
  source 1..570: mol_type = genomic DNA
atgccatttgagcaatgtcatagcattacttctttaatgtcagggtttaataaaacgtggttctttgcaggtggttgggcaattgatctttttatcggcagagaaacaagagaacatcaagatatagagattgcactatttcgagaagaccaattatatctgaaggaatatcttaaagaatgggattttaaaaaggttattaaaggtaaattctattcttgggaaaatgagtttttagagttacctattcacgaaatacacgctttgaataagtcaaatggagataaattagaagttcttctaaatgaaacaaaggagaatgattggaaattcagaagggatttaaggatttcccatccacttaagtcagtttggagttattctaatacaggcattccttatctaaatccagaaattgtacttttatataaagtgaaaaacacaagagaaaaagaccatcaagactttatggcgataatagacaaactagataatcagaggaaaaaatggcttcattatgctatacaattgcacgaaccagaacacaaatggcttcaattcttaacataa

SEQ ID NO: 240 - DNA, 828 bp, Peribacillus Aracenensis
  source 1..828: mol_type = genomic DNA
atgacatatttatcaataggcgacatgtcaaagttaaataatgtatcaattcaaactcttcgttattatgataaaatcggcctttttaaaccagaatacattaatcccgataatcattatcgttattatagtgttagacaaattttttatttagatattatcaaatacttgaaacacatcggtacgccacttgaggaaattcgccaaatgatcgcactgcctcctgaatcaatgtatgagttcctagaaaagcaggaattgactatagaagaacaaatcaaaaaactagaaaatattcaacatttgctaaatcactacaaaagccagcttcacgagcaaatacttctaaacaatcaggaactcggtgtcgtctatacccgtaaaatagatgagcgcaacgtattaaaagtagattgccaaaacgtagtgactccactagatcaacccgatatatatttcagagaacttgcggatgcacttgagaaagaagggacagttgttgatcttcaatatggctgtatatatccgttaaagcattacgaatcaacagaaaaaattcattacagcagtctttatactcatattactaaaaccgatctaaatccctcaggtgtttatgtcgattccatcccaaaagggacatatatgtgtatcgcctttaagtggtctaaagccgattattatggtcacttcagcaaactaaaaaaagcctactatacgtcaggcttcccaatgaaaaataatgtgaacgaagtttcactgccgaataattatgctacttcaaatgatgaagactttataaccgagctccaaatacacattgattga

SEQ ID NO: 241 - DNA, 864 bp, Peribacillus Aracenensis
  source 1..864: mol_type = genomic DNA
gtgtttattatgagtaaaacaataaggttaatagcccctgattggcaaggggggaataagcgagaatattattttggtgcagaattactgtcatggttagctcctaataatgctaaccaaaaagagataaaattagatattgaggaaccgaaaaatgaagaattagaaaaagaaaatggggtggttgctcaatctagtgttaaacgaaatgtgagtatggcagcagaagtattgaaagaagaattacctgataaaattattacttttggtgggagctgtttagtatctcaagccccttttgattatcttcatggtaaatatggcaaagaactcggaatcgtttggatagattctcatcctgatgtttcaactccaaaagaatatcatcatgaacatgctatggttttggggaatttattaggagcaggagatccagagttatctataagtgttgaagttccttttaattcaaattcatttttatatgttggaatgcaagagccgaatgatttagaagtaaaattattagaggatttaaatctaaattatactgttcaagataaaaggattttaaaatttgaagaaatacaaaagtggattaaagagaatggttttacaaaaatagctgttcatcttgatttagatgtattagacccaaatttatttagatctttatatttctctgagcctggtgtgacagagtttccctcagaatcaggaaagatgactcctaaagaattactgaatatattaaaaggcatttttgaagaaaatgatgttgtgggattaacgattgccgaatttttaccatgggattctataaatttaaaaaatatattatctgatttagatatttttgaataa

SEQ ID NO: 242 - DNA, 981 bp, Peribacillus Aracenensis
  source 1..981: mol_type = genomic DNA
atgaaaaaggggaaattgtctatggaaaaccgttctatactttcaggtgttcatcaagttattggtaacactcccatggttcacctatctagaattacagaaggtcttgatggaaatatttttgctaaacttgaatatttaaatcctggttttagcaaaaaagatagaattggtttacagataattgaagaggctgaaaaggcaggattactcaagcctaatcaaactgttgtggaactgacaagtggcaatactggtacaggactggctattgtatgtggagtgaaaggttataaatttgtagctgtaatgtctaagggaaattccttagaaagagcaagaatgatggaagcactgggagcagaggttgtattagtagaccaagtccctggttcaccggtagggcaagtatctggaaaggatctcgccaaagttgaagaggtcgcagaacaaataacaaaagaaagaaacgcattccgtgcagaccaatttaatcatattggaaatatacatgctcacgaatatcacacaggggaagaaatgtggagacaaacaaatggagaaatagatgtttttctagattttgcaggttctggtggtacttttaccggatgtgcaaaaactttaaaaaagtataaacccgacattcgttgctacttagttgaaccagattctgctcccttttactctggtaaacctgtaatgaatccaaatcataagattcaaggcggtggatatttaatgaacttgcctcttttggataaaaatttagttacaaactatattcatattacagatgaagaggctacacaagttgcaagagatttagcaaaaaaagaagggatatttgcaggattttcttcaggagcgaatgttgctgctgcattaaaactattgaagcaggaagaaaaaggagcaaatatcgtattaactataaatgattctggtcttaaatatctaagcacagatctatataaataa

SEQ ID NO: 243 - DNA, 555 bp, Peribacillus Aracenensis
  source 1..555: mol_type = genomic DNA
atggatcaaattaataaaagtatcagcaaaaatataaaaagtgtccggcaagaaagaaatttaagtttagaaaaaacatctgaattaacaggtgttagcaaaactatgttaggacaaatcgaaagaggcgagtcgaatccaactgtaacaactctttggaaaatagctaatgggttacgattatcattctcttcactaattagtcaagatagaccatctgttactttaataaaaaagaatgaagtagtgccagttattgaaaataatggacaatatcgtgtgtatccacttgtatcatttaatccagaaaaccagtttgaagtctttttaataaccctagaaccaggatgtgagcataaatcagaaccgcataatgcaggtgttgaagaatacatttttgtaaatgaggggactttagaagttgaagttaatgaaaagctttatgaagtcgattgcgaggacactatgatttttgatgcagataaacctcatatttacaggaacaatggaaataagatagtaaagtgttcagtattaattcattatcctatttaa

SEQ ID NO: 244 - DNA, 183 bp, Peribacillus Aracenensis
  source 1..183: mol_type = genomic DNA
atgaaaaatctaattattggtatcatagttttattggtactttggctaatacttccgttattcaatataaactcatcatatttaattcctattgttattgaatgggctacaaagtttatacttccgtggatagtattgtattggattatcagactcattaaaaatttagaaaaaatttattag

SEQ ID NO: 245 - DNA, 165 bp, Peribacillus Aracenensis
  source 1..165: mol_type = genomic DNA
atgagatacaatgaaacagaggtgaaaattatgaacaaagatcaagaaaaatacgctcctatgcccgatgataatgatttaactgaggaaatgataaatgataatggggaacagagacagctcaattctttcctgacgaaagattgcttgcccctttatcaataa

SEQ ID NO: 246 - DNA, 156 bp, Peribacillus Aracenensis
  source 1..156: mol_type = genomic DNA
atggatatagttggccactttgttgccaggtttaacaaaagagtggtttttcttatagggaaagcggttctttttataaaagagaaacgatacaaacaatggtcaccaggactatctggtgaccttatagtaccaatggcaacattagattattaa

SEQ ID NO: 247 - DNA, 216 bp, Peribacillus Aracenensis
  source 1..216: mol_type = genomic DNA
atgacatatgttttttctttattcattatttttgtaataggctttgtttgttatcggatgattaaaaagaaatcaataccttcaaatagatacacaccttatgatgacatcactatgggaattaaagatgacgatatacaacaagataatccaatacatgataccaagcatcataatcaatatgaagagaaatcaaataacgacaagaccgtttaa

SEQ ID NO: 248 - DNA, 288 bp, Peribacillus Aracenensis
  source 1..288: mol_type = genomic DNA
atgaggcttggcaagttggcgggtagggagcgaatttctgaaatcaactggaacgtttttaaaactgcagacaaactcaattattaccgagtttgtctgcagtctgaagctaatagactagccaatgataagctctccattttaactggagggctttttcggaagggatttttatatattgacaattccttttggattggtaatatttactttattattacattaataccggatgtgatttttaatagaaggcggttaaattatggatgggaaaatcatttacgatga

SEQ ID NO: 249 - DNA, 171 bp, Peribacillus Aracenensis
  source 1..171: mol_type = genomic DNA
atgaggaaatgggtggcatactatgggattgaagattttttccatcatttttattttatgtggtctttttgtaatgtggttcgccgtttttggcaaaaagaaagagatcaaagagttcggctccggaataccaatgaatttcatcgatgtaattttaatgatgatatatag

SEQ ID NO: 250 - DNA, 141 bp, Peribacillus Aracenensis
  source 1..141: mol_type = genomic DNA
atgatgagccatactttcattcctctgttaaaaatgctgttaaaaaatatagttggagaaaatgtgcgaagggatggaatcttcactataaatgaaaacagtattccgggggcttatcaggaagtattgaaactccattaa

SEQ ID NO: 251 - DNA, 264 bp, Peribacillus Aracenensis
  source 1..264: mol_type = genomic DNA
atgagaggctttccgaggagagccctacataatagtgagatcattcccttgggaatcatttcttttcaagatcaggggagtgacatacctcaagaactccttccgcgtttaggtgaacccttttacaccttaaaagaaaagggaacaggactcggattaatgatctaccataaaatcattaagcaacacgatggcaatattgtctatcaaagtaaagtgaacgaaggaaccttggtggagattactttgaatttggcctgttag

SEQ ID NO: 252 - DNA, 165 bp, Peribacillus Aracenensis
  source 1..165: mol_type = genomic DNA
atgttaagcttggttgaatcatatcacctcacttatttggctcttgctattataacagaccatttactcaaatttttaacttttaaaaaatttgaatttccaccttcattttcatatgaaaagttcaacattaatattgaggagttggaaccgaactttccttaa

SEQ ID NO: 253 - DNA, 177 bp, Peribacillus Aracenensis
  source 1..177: mol_type = genomic DNA
ttgcttagttatcgtttaatatttcttgctaaaaggcttgtacctgaatcattcacttattttaccgtaacctgttttgtaataggacaaaatataataggaaaaatcataaggatcttgatggttaatgaaaaaaagcaaaaaactcaaacgggaacaatggaaaaagaaagttaa

SEQ ID NO: 254 - DNA, 117 bp, Peribacillus Aracenensis
  source 1..117: mol_type = genomic DNA
atgtctcactttgactttatttcattttctgatgtgaaaattattggtcaattgaaatcttccgctattttctatcgcaagtttgagaaaaaatgtgcgggggtagaaaatacttaa

SEQ ID NO: 255 - DNA, 477 bp, Peribacillus Aracenensis
  source 1..477: mol_type = genomic DNA
atgattattatgaaatttaaggaaactgatattgaagaaattgtttctttattttacgaaacagttcattcagttaatttgaaggattattcgcaagaacaattagatgtttgggcaacaaaagaggaaaaagaatcgaaaatcaattcgtggaaaatttcattaggtcaaaatatatcatttgttgcaaaaattaatcataaagtagtgggctttagtgacttgacctatgacgggtacttagatagactgtttgttcataaagattttcaaggtcaaggtatagcttcagcattagttgatatgcttgaaagtgaagcgaaaaagctaaaccttttagaaatttatacagattcaagcattacagctaaaccattttttaaacataaaggttacaatattgttcgttcacaaactgttgaacgtaaaggtgtcaaattgactaattttaaaatgagaaaaaaattaaaatcctaa

SEQ ID NO: 256 - DNA, 837 bp, Peribacillus Aracenensis
  source 1..837: mol_type = genomic DNA
atgcgttcagaaaaagaaatgatggaattgatattacgagttgccgagaaagatgagagagtacgagctgttgcattgaatggttctcgaacgaattttaatgtacctaaagattctttcagagattatgatattgtttatcttgtatctgactttcaatcgtttctaattaatcctgattgggtaaatgtttttgggaaaagaataataatgcaaacaccagaagatatggcaatgtttccacctgaattgggtgggagattcacctatctaatgttatttgaggatggtaatagaattgatttaatgctgattccgattgaggaaaaagatacttattgttctgaagatggattaacactaattttattagataaagatggaaatatgcctaagctttctgaaccaacagataaagattactgggtaaaaaagccttctgctgaattttttgctgaatgttgtaatgaattttggtgggtttcaacttatgtagcaaaagggttatggagacaagaaatactttacgcttatgaccatttaagtagtgtaagagaaatgttactaacaatgcttgagtggaaagttggtatagaaaccaatttttcattgagtgtaggaaaaaacagcaagtacctaaagtgctaccttgataacgacatttgggaaagattgatgaaaacatatcctaatggagattacgaacaagtttggaattcgttgtttgaaacaattgacttgtttgagcaagtagctattgaagtagctagtattctcgaatatcaatacccttctgaagacgcgaataaggttaaacaataccttactaatcattaa

SEQ ID NO: 257 - DNA, 330 bp, Peribacillus Aracenensis
  source 1..330: mol_type = genomic DNA
atgaaatttacattatttattgaggcaagtaattcagaagaaactaacaaacacttagatgattttaagaaatttactgctaattataaagttttcatgtctgtttccgaaatagaaaagtattggaaaattgatgatatgtacaaggtttttcttgatatagatgaatcatctgaatctaatgtaaaaccaatgctaaataatattgcatctaaatggctggaacttcccaacgaatttttagcttcaaacactatggatggctgtgaaatttatattccaaaccttcatatgataactcttgtgctaattaaaaaccatgcttgttaa

SEQ ID NO: 258 - DNA, 291 bp, Peribacillus Aracenensis
  source 1..291: mol_type = genomic DNA
atgaataatcactgctgcgaaactatgaaagaccaagttaatattaagtgcaagattgattgtccagacattttgattacctatgataaaaagtttgatgaatatgggttaataatccacgatggaggcagctcaagtatagagataacctattgtccctggtgtggctcgaaattacctgattctaaaagagatttatggtttgaaatccttgaacagttaggatttgatgaccctgttgagcaatcgattccagaggaatttaaaacagataaatggtataaaaaatag

SEQ ID NO: 259 - DNA, 696 bp, Peribacillus Aracenensis
  source 1..696: mol_type = genomic DNA
atgaaacgtatatcgattttaattgctgatgatgaggaggaaattgctgaccttattgcaatccatctagaaaaagaaggatacaatgtcattaaagtacataatgggcaagaagccatacatgttatccagactcaatcaattgatttgctaattttggatattatgatgccgaaaatggatggatatgaagtaacccgtcagactcgggaacaatataatatgcctatcatttttttgagtgcgaaaacttctgatttcgataaggtacatggattagtgattggagcagatgattatatgactaaaccatttacccccattgaattggttgctcgtgtgaatgctcaattgcggcgctttatgaagttgaatcaacccaaagtagataataaagctatcttggaatttggtggaatggtgatttctcctgatcaacgtacagtattgctctatggtgaaaacatcgagctaacgccgaaagagtttgatattttgtatttattagccagtcatccaaagaaagtttatagtgtagaaaatatttttcagcaggtttggggtgatgcatactttgaaggtggtaatacggtaatggtgcatattcgtaccttacggaaaaaacttggagaagataaaaggaaaaacaagttaatcaaaactgtttggggagtggggtatacattcaatggctaa

SEQ ID NO: 260 - DNA, 1113 bp, Peribacillus Aracenensis
  source 1..1113: mol_type = genomic DNA
atggctaaatttatacacagttttcgctccaaaataatcgtattatttggtttaagtatgcttcttggtggtattataacttacttaatctttaaaggactgcagctttattatcatacgagggttcgttggggtgacccattggcccaacttcgtgaattcatagacagtattggagactttaacttcttttttgtactatttatctcactttcgatattgtttttctatttactcactaagccctattctacctatttcaaggagatatcaagcggaattcattatctcgctcgtggcaactttaaacatcgggtttatatccaatcaaatgatgaatttggagatattgcacaagcaattaatcttgcaagtgaaaaattagaagaagccatacaaagaggcgatttttctgaaaacagtaaagaacagttagttgtaaatttggctcatgatttgcgtactcccctaacttctgttttaggttatttagatttaatccttaaggatgagaagttgactaaagaacaagtcagacattttttaacgattgcctttactaaatctcagcgtttagaaagactgattgatgaattattcgaaataactagaatgaactatggcatgttaccagttgaaaaaaggcaaattaatttaagtgacctacttcttcaattaaaagaagaattgtatcctgttttcgagaaaaatgatttgatcgcccgaatgaatattcttccccatttacctattttgggtgacggagagatgttagctcgtgtgtttgaaaatcttttaaccaatgcaaatcgctatggatatgatggtcagtttgtagatattaacgggtttgttgatgcaggagaagtggttgttcaggttattaattatggagatagtattcctccgaatgaacttccatatctttttgatatgttttataccggtgacaaagcacgaactcatcaagaagatagcacaggtcttggtttattcattgcaaagaatattgtggagcaacataatggaacgattacggccgaaagtagtttaatacacactgtatttgaagttcgtttaccgcaggaaagtgttacaattgaccaagtttaa

SEQ ID NO: 261 - DNA, 912 bp, Peribacillus Aracenensis
  source 1..912: mol_type = genomic DNA
atgaagaagtggggatttttattgttgttagtattatgtctgagttttgcatttgtcaataaagaatcgtcttttcaagaggttcaaagatatgaaaaaagtaacaatgatcaattaggtaatagagagacctctgaaagtttccaaacgatagaaattacaaaagaacgggtctttcaaggaaatttacttttggttaataatgaatatccgattcacaaagagagtataaaatcagatgttgtaaatttatttacgcataaagaattgacaaagggatacgggttgcttgataacgaaattaaattgtcagaggatattgcacatgaattttcggcgatgatggctgctgcagaaaaagagggggttcgccattttacaattaatagtggctttcgagactttgatgagcaaagtgcactttaccaggaaatggggtctgactatgccttgcctgcaggctatagcgaacacaatttgggtttatcacttgatgtaggatcaactcaaatgaagatggatgtagcacctgaaggaaagtggataggaaaaaatgcttggaaatacggctttattttacggtatccaaaggataaaacagaagttactggaattcagtatgaaccttggcatattcgctatgttggattgccgcacagtgtaattatggaggaaaagaatttttctttagaagaatatttggatttcctaaaagaacaaaagtccatttcaactactatacatggtgaaaaatatgagatctcttattaccctgtaaccaaggatacgaccattcatgtgccttccaatcttcattgggagatatcaggcaacaatatggatggtgtaattgtgacggtgtttcccagaacaatacatactaatctcaaggaagtaaggacggtgaaatga

SEQ ID NO: 262 - DNA, 573 bp, Peribacillus Aracenensis
  source 1..573: mol_type = genomic DNA
atgaaaaaaacgaaattaatgaacagaagggttattgtactagcactatttgtcttttatatgtacgcattgcttagaatcattctatttaagttccgttggagagatatgacctttctctggcatcaacttcagacgaatcttgggaaccctgatattctcatgtaccaattgcaaagaggtaattttttcccgtttaaaacaatattcattaatattcagagtctatcatggtggcatgattttagtaatttggtggggaatatcgcattgttcatcccatttggaatgtttctcgtatttttgtctaaaaataaaggaatgtcattcataggcgtattagctggatctttgagtttaagcttatgcttggaatgcttacaggtagttttttctctcggaatttttgatgtggatgatctaatactaaacacctctgggggattgcttggctattgtgttatcaagctttatgacaaggtttatagtaaatttatagggaatacatcaagcattgtccaagatagagatattgttgaaaaacaggaggcgggtgaaccgtaccataaataa

SEQ ID NO: 263 - DNA, 201 bp, Peribacillus Aracenensis
  source 1..201: mol_type = genomic DNA
atgattcattcattttctaacggagaaatcgattctttagtgacagatacaagcgaattgctgggggaaatagccactgatagtgcggattcagatggccatctaagtgaaaaaatgtttaataaaccattaaggaaaagtaatggcagggtgtttgatgggtgggaagagtaccaaaaagaaatttcctatttctcctga

SEQ ID NO: 264 - DNA, 177 bp, Peribacillus Aracenensis
  source 1..177: mol_type = genomic DNA
gtgcgagactcctgcgggagcggcgggacaggtgagaccccacaggcgtttacgccgaggaggctcaccgcccgccccgcggaaagcgagcatctggagggaaaatcaaccacaccgctttacttggtaaatagcaacaaagtatgcgaaaacagccatatggaaatagtaaggtaa

SEQ ID NO: 265 - DNA, 399 bp, Peribacillus Aracenensis
  source 1..399: mol_type = genomic DNA
atgatttttgaaatgactactcaggttcgggtttccagcataaaagaagggcaaagatggtatggaacactgctaaataagaagcctgaatttactccacacgatggatttgcagagtgggaactcattcctggttgttggttgcaggtcgctgaaggaattcttactgacggtaacggaccattacgattaggggttactaacattgaagctgaaagagatagacttgtagaagagctaaagattgatagttttgaaattcattcaagaccagaagttccagttaaatggggaactttcacagacccgtggggaaatcgacttggattttttgaatacttggataagaacgaagagcaagaacgtattaaaacaatcgttggaacaatagaagtttaa

SEQ ID NO: 266 - DNA, 234 bp, Peribacillus Aracenensis
  source 1..234: mol_type = genomic DNA
atgattgaagagttttgcgcagatttgcaagcaaatggccctgtacgcttttttagagttccaaatagtgatgaaagtcctgtcgtttatcaatccaatgatcgtacggcttttagtgaattatgtgattggtattcaattgaagtggaaagaagaagccaggaacgattaacgtgttttattaatcctggatttaacttattctcacacctagcattaaaagaaacttcttaa

SEQ ID NO: 267 - DNA, 363 bp, Peribacillus Aracenensis
  source 1..363: mol_type = genomic DNA
atgactttggatgatgaggttactaatgacttttctattaatgggctagattcatatacacctatagatgaggtggcgggtggggtcacaccttgtttacctgattctggatgtactttagcaactactcctactagtatactggctactacgtcttcgtcttttattgctgcacctgctaatgtgcctgatcatttcattagtgcactttgggatcgtggttttactgatgggcggtttgtttttggtccttggggaaaagtacagttggcttttaagacgtttagtataccttttaaggctattgcttcgaattctgactttatgggacttagtgattgcggctgttggtgtaacctgtga

SEQ ID NO: 268 - DNA, 171 bp, Peribacillus Aracenensis
  source 1..171: mol_type = genomic DNA
atgcgtaggttagagattcaggaaaagttaagatttaattatgtagattctaagtttctggaagacatgcttttggagattgatctagaatattcggcacgtataagacgtgaagcaactaaagaaaaaaatgtttttagttattttagggattatttgagtttggattga

SEQ ID NO: 269 - DNA, 543 bp, Peribacillus Aracenensis
  source 1..543: mol_type = genomic DNA
atggtaacaataaaaaaggataaccaattaagcttggaagttcatgtaaaccagataaaagaagatgttaaaaaaggagagttggtacttgagcatgaaatatttttaaaacttaaaaaagaagttggttttaaggaagaatacgaaggatacgaaaaattgttggatatcattaaagataatgaagaaaataacatttgtcgattgtcaaaaaagaaaatatccgaattatatgggatgtcctataccagcactcttaataagatgaattttttggttcgttacgatttgataaggcaagttgatggtgggttcgttaggacagaggaaaaactaaacaatgccattccattttttattatgccaaaaattctagccttaaaaatattgagacccgacttacgtacacgtgaacgtaaaaattacaaaaaacaagcagagattctttcagtctctttaagagaaattcaagtcgctgacgggttcatcaactatgtaataggtcaccctgaatgcagtttgtatcaatatggtctaatctag

SEQ ID NO: 270 - DNA, 510 bp, Peribacillus Aracenensis
  source 1..510: mol_type = genomic DNA
gtggaatttttcttgatagaaattaaaagaacagatatagaaagtctcggtaaaatgtttgaggttgaatatgtagaaaacaaaatggagcgtaaaaaaatattctacatatatacttacgaacgtgtaatgtccataaaatggaaaggacaaatcattcacatacaaacattgaatctggattgtaattttaaaatggataacggtagaacctcagaactacctgttgatgaaataagaaacagaataaaaacagttgatggaatgtcaaaagatgaatttgcactttattgcttagatatgttaaagctctatcatgaaattgttgagctaataggagaatacaaaatcggacgaagtgatgatgaatggtcaaaacatacaaaggtatatattgatagcccttattcatctatacaaatagattccgtacaaggaagtatgtctggatgtagtcctcaaataagcagtagtcagaatttatattttgaaaaacttcacatcaaataa

SEQ ID NO: 271 - DNA, 180 bp, Peribacillus Aracenensis
  source 1..180: mol_type = genomic DNA
atgttaatttgtgttactatttacctaaaaagaggtgcttcaatggatataataattactttgtataatgcacttggacaattaatagatgattattacaaatgcgatgatttaacagttaaagaaaaaatacaatgtgagatcattttgttaatagacgttatattaaattgtgattaa

SEQ ID NO: 272 - DNA, 336 bp, Peribacillus Aracenensis
  source 1..336: mol_type = genomic DNA
atgaatatagatagaggaatcttaaagtggcagccagcattaatgctccctaaactgaaaaaattgcataagcaagttaatcaagactactatagggaatctaaacccattctggatgagtaccaaatccaagacatagaagataagattaattattcaatggagtttattttgcctgttaccataactttgtatagtgatggttttccgaaaagtataaaaggtttttttgtttacctggaaccaattaataaaggaagtacatttgagcttgaagatcaaacctttcttaaaattttcttttccgatctcttagatataatggttcatgaataa

SEQ ID NO: 273 - DNA, 1035 bp, Peribacillus Aracenensis
  source 1..1035: mol_type = genomic DNA
ttgaaaactgtcattcttgcagaaaaaccaaatcaagcgaaaaaatatgcgaatgcgctgggaacagtaaagagaggaaaaggttattttgatattgactctaacataataaactgggacgtcagtattatctgtggtgtgggccatttagttgagttatcaagtatggatagatatggtgaacaatataagaaatggaacatgaataatcttccttttcagccatctaatatgctatatgatgttagcggaaaaacaagagatcagtttgttaatgcaaagaagcaattggaagaagctgatttaataattgtggccacagatccagacagagagggcgaaaacatagcatactctattttctcaatgtgttctaagatagtaagaaatacacctaaaaaaagattatggattaactcgatggttgataaagaggtacagagagggttcaggaatttaaaggatagcaaggaaacctataatttttatgtagaggcacaaactagacaaatcagtgattatttagtaggcatgaatttcactcaatattttactctttttgcacaatcaaaaggcttatcaggaatatattcattaggtagagttcaaacaccatgtaatagtttaatcgtacaaaatgacagggacataaaaaattttaaggaagagattttctataaattaattggaatggcaactaaatatacaaataatgataaagttaaattctttagcgaaaaaaagtatagaactaaagatgaattggctagtgctttatatccattccaactagaagcaaagataaaaactaatattttatctgtacaaaaggaaattaaaacgaaaaaagctcctaagttatttaatttagggggaattcaaagctattcgaataaaaaatggaaatatagtttagataaatcccttaaaataattcaatccttatatcaagaaggctacctttcatatcctcgaacagactctgatttaattactactaatgaggggaagaaattctatttacacttagtttag

SEQ ID NO: 274 - DNA, 273 bp, Peribacillus Aracenensis
  source 1..273: mol_type = genomic DNA
atggataggttaggactcggtaccccagcaactagatcatctatactgaaaacgttaatcgatagagaatatgttaaagtggaaaaaacaaagctatatccaactgaaaagggtattttactatatgatcttacgcagaatattcttttaggtagtcctgaaatgacagcaaaatgggaagaatatttgaagagaattgaagcaggggaaggatcacaaaaaacctttttaaataatattaattccttcattagtaaaacattatggatttga

SEQ ID NO: 275 - DNA, 336 bp, Peribacillus Aracenensis
  source 1..336: mol_type = genomic DNA
atgagagggcaagctgaaagtgttgcaagctcagtaaaagaaatgttcgagcagatgaaatctatcaatctgtctgttgacatgggggataaaggagtcaccccattagtatttagcgcgacaaaaattaaagaaatctccactctaattactgatatttcaggtcagacgaatttacttgcattaaacgctgcaattgaggcagctagagccggggagaatggaaaaggattcgcagttgttacagaagaggttagaaaattagccgatcaaacaacacaatttgcaaataatatccataagcttgtttcaatcatccaaaatgaatcaaactag

SEQ ID NO: 276 - DNA, 414 bp, Peribacillus Aracenensis
  source 1..414: mol_type = genomic DNA
atggtagaggcaatccacaaaggaaaattaaaatccctttatctatttggagaagaaatggggcttgtggatgcaaactcgaaccatgttcaaagtgcatttgaaaaattaaacttctttgtcgtacaggatattttcttctcgaaaacggcacaatttgccgatgttgttttaccggcatcaccttcacttgaaaaagatttaaacaatggacgtttgcttgagcacttccatgaaggaaatatgaggtaccggacagaaggacttatccataaggtacctggcacatggctggaggtatcgcacgaattggcggaggaacgcaatctcagtgacggtacattagttagattaagttcaccatatggacaggttaaagtaagggcgcttgttacggaccgggttaaaggttga

SEQ ID NO: 277 - DNA, 579 bp, Peribacillus Aracenensis
  source 1..579: mol_type = genomic DNA
atggggaaaataattgcaaacgtaagcaacacattggacggtatctttacggggccgaaaggtgaagaaaacaacatggtaagctgggcaatgcctggcatcgtggattccacaaatgatggtcttgtcatgttccagaaggctgacgcactcttgatggggcgggtcacatatgaaggctttgcaggatattggccgttccaagagggagattgggctgacgccatgaataaaactcgaaagtatgtagcaactaataataatgagcttacggtaattcactggggagactacgatgataccatttctctgcttaaccatgatgtaatgtcgaaagtaggggagcttaaaagagaaatcaagggagatatcattgttcctgcgagtgcagctcttgttcaaagtttgattaatgctagtttacttgatgaactccgaatcatcattcatccggtcattttgggcagcggaaaacgtttcttcgacaacatagaaacacgtcacgacatgaagttgatagaaaccaagctttacgaaacaagtggttcaatgctgatgcggtatgaaaccgtcaaataa

SEQ ID NO: 278 - DNA, 213 bp, Peribacillus Aracenensis
  source 1..213: mol_type = genomic DNA
atgaatttattaagcttttcaaaagtgaagattttaaaactatctattcatgcattgttaataggtgttttattaacattagttagtttaattgttaatgatgttatttcaatggttcttcatgaaagaatgacattgaatttaatatttattaatgtaattatggctttttgggttttgtgggcaatgcaaaatacaaaatatcagaaataa

SEQ ID NO: 279 - DNA, 939 bp, Peribacillus Aracenensis
  source 1..939: mol_type = genomic DNA
atgaacctttcattaaaagactacattacagaaaatgaaatccaaaattatagcaagacaaccgtcaagaataagaaggctattcttcaacagtttgaaagatggttatgggaaacattccagattgaattagatgatgccaccactagacatgttaaacggtggattaaatatcttctcgataaggaaatcaaagcaaataccattaacaccaaactaaagaccttaaccaacttctataagttctgtattaaagaaaagatactgaaggataaccagttggaagacatagaactactgaaggaagagaaagtcatgattaaaccgttcagccttcaggatattgaaaagatgattgggttttattgtggcagtaactttatggatgttaggaacaaaactattttgacctgcctatttgagactggaatacggtcagcagagttatcagggcctaaattagaggatgtatttgatgatgcccttttgataaggggtaaaggtaacaagcaaagattagtacctgtaagcttagaattaaagcgtcagttgaataaatatagaagggcaagggagaagtacctaaaaggtgaggaatgcccgtttctattcgtctgcacccgtactaaagggggaggtttacggaaagatgataagcctattggaagaatggggcatgatgcagtattaaacgttgttaaacggtcaggaaaagcctgtggggtagatgtgaagcttttagtacactcatgtaggagagaaagctacgcacaaatctctctagggcatacagacctttatacggtgtctaggctactaggacataaccagttagctacaacagagaagtatattcaatcaatggaagataagaccgtactggaaagaggaaggaacgcttcaccgttaacactcttagaaagagatattcataattaa

SEQ ID NO: 280 - DNA, 741 bp, Peribacillus Aracenensis
  source 1..741: mol_type = genomic DNA
atggataaggcttatttggattcacattacattttactcccacatataacattacaagtgacacgtttttatcccgattttttaaaaaatttaaggataatgggaggaaaattcatgggaaagtccgggtttgtccctgataatacaaacataaaaaaaacaagtggaacacctaatctcttttttgattctaaggataatattgagttcgaaaaagacgccgaaaatgtcatatataaagttacttccactcaactccccgcaatagttggaggtgcttttgctgatgtttatcttacaaagggacatattcgggaacctcattggcatcctaactcatgggagttagacgttgtaatttctggtgaagcccaaatttccattattgaccctgataccaataaattgcataactatattgcgaaacctggtcaagttgtttttattccaatgggttggtttcattggattacacctaagtcagaaaaattgcatatgcacctcttttttaacaatgaccaatttgaaactgcattaggttctaatatgctacgattaacaccgccagaggtttatcaactttcatatggtattgatgaaaacaaaatagcagatgtcttaagtccgattaaagaatcagtcgaaattggtcctcctgaacctcgccatcctttcacaccgaatacaagccgtataaaacgagataaagttcccaagcaaaaagggaaaaagaggaaatag

SEQ ID NO: 281 - DNA, 126 bp, Peribacillus Aracenensis
  source 1..126: mol_type = genomic DNA
atgaaacagggagaacccttccaaaagggttttggagggttaattatcataaggaaaatggaatttttagaaaaagatattgacatcccattagctggtttagctgaaaatcagagctgtttttaa

SEQ ID NO: 282 - DNA, 231 bp, Peribacillus Aracenensis
  source 1..231: mol_type = genomic DNA
ttggacatcaaaacagctgaatataacgcaaaggttaaagagcttgctgcagctaacaatacaattaaaaacttgaatacttcacttaaatatgcggaagaaaaggatggacaagctgataaattagtcgctgaacttgaaaaagaaattcaaaaggctaataaagaagtggagaaacatgacaaagaggtgaaaaaccaaaaactaaaactgaggctgctgaaccaatga

SEQ ID NO: 283 - DNA, 552 bp, Peribacillus Aracenensis
  source 1..552: mol_type = genomic DNA
atggaaaaaaaatctttatcaattcaaattggtcaacgtttacgtttttatcgccaacaacgtcaattatccttggacgaccttgctagtctgactggtgttagtaaacctatgctcgggcaaattgaacggggcagctccaatccaactgtggctatactgtggaaaatagctgctggactacaaattccattcggttcatttcttgtaagaaatccttctattaaaattcttcgagaagaggaacaaccaaagtttcaagaatataacgacctttttgaagctcataatacatttgcctcaccaggtgtgccgtttgaaacatatcgtattcgcttgctaccaggctgtacacatttgtcctctcctatagagggactaaaatctataacagtccattccggcactttaactatagagataagcggggaaagttgcaccttacagaaaggagatgccatctcattctctccggccactaatcaggtatatcaaaatctgggtgatgaagtgtgtgaatgtaatcaagtaatcttttataccatccactga

SEQ ID NO: 284 - DNA, 432 bp, Peribacillus Aracenensis
  source 1..432: mol_type = genomic DNA
atgagttatacaattacggagttgtttataggacaaattgcgcgtttgcaacgtacatttactgaacaggacgtaagatcttgcaaggaattaactagagaccatagccctgtatacggactgaatgaagacatatggaaaagttattatagtcaaccaattgttccgggcctgatgacagaagggttaattactcaagtcattagtgaaaaacttcctggaagtgcttgtattttgctgcaaaaggaattggttttttatcatcccgtgtatgtaggagacgttattacagtcgagttggagattattgatttaaatttaaagagaaactgggttacccaaaaggttactgcttacaatcaggctggtaatgaagtgatcaaaggacaagttgtcatttttgttttatccaatgagaaaatggataggtga

SEQ ID NO: 285 - DNA, 1311 bp, Peribacillus Aracenensis
  source 1..1311: mol_type = genomic DNA
atgaagaaacttaatctgaaagaccaaaccgaagactggggttttattgaagttgatgcaggcggaatattgatcgatattagttcggatttttgtcggaattttttgattaataaaaaagattggttaggagtttatgcgaagaaagttatccaaagaacacattacggtaagcatgcaaaggtattatttggagtcgtttttggatattcatgcttaattagagtattgaaaatgaatgaacataagatttatcgggtgattgtacgtcaagaggatgttaatcagtatgaaatgatttcgtttatgaattctctggataccttaaaaacgaagaaaaggtcaacaggtcaaaatcgatacagctttgaggaaattatcggtgaaagttcggcgattgaggagattaaagagttggcagcccgtatcgcaacaagtaattctactgttttgttgacgggagaaagcggaacagggaaggaattgtttgctcaagcgatacacggattaagcacgagaaaaaataacccttttgtggcggtaaattgtgctgccatcccggatgaattatttgaatcggaagttttcggatatgaggcaggagcgtttagtggtgcgaaaaaggaaggcaaaccagggaaaatcgagatggcccagcatggtactctttttctggatgaaatatcagaactcccataccaagcccaaggaaaacttcttcgtgttttacaggaaagagaagtggaacgactcggtggaacagggagtaaaaatgtcgatattcggattatcgctgcaacgaaccgggatttgagaacgcttgttcaggaagggaagttcaggcaggatttattttaccgattatatgtctttgatttgaagattccttcacttcggcaaaggaaagaagatattattccattagctcagtttttcattgaatattttaatgagaaatttggtgctcacgtaaagtatattgattctaagctacaagagaggttaataagttatgagtggccggggaatgtacgtgaattaaaagcctatattgaacgcggaatgaatttggtcttgggagatactctcacgttagacgatttacgtatttcacctaatgtgtcttcagatgtaataaaaagaactctgactcccattcaaagtttagaggaggaagtgaagtgtacggaaatcaacgtaattcaacgtgcattacaagaagcgaatggtgaccgaacattggctgcacaaaagctaaaaattcatcttgctagcctttaccgtaaaattgcaaagtacaatctaaaataa

SEQ ID NO: 286 - DNA, 1110 bp, Peribacillus Aracenensis
  source 1..1110: mol_type = genomic DNA
atgctaaaagaatttgcgaaggaggagctgcttcccaattatacaaaatgggatagagaggggattacgccaagacatttatggaagaagcttggtgagttaggtgtcaatgggctgcgaattccggaagagtatggtggaaccggtgcagattgcgtgacaactggaatagctgccgaagaaattggacgaggtgatttcaaccttacttattctgtcatgttgaatggattaattggagaaattattaataatcatgcacgtgaagagctaaaacaggaatggctgccaaagatagctagcggagatgcaatcgtgggcattgccattacagagccttcagccggaacagatgccggtgggattaagacaacggctgtacataaaggaaatgtgtttgttctaaatggtgagaaatcgggaatcagtgtggccactgttggtgatgcctttatcatatttgcaaaaactgacacagaactagggaatcgtggaattagtgcatttattgttccggcaaatctctctggagtcgaatgcaaaggttatgaagatatggggaatattccgattagtcgaggttccatttacttaaatgatgtagaagtccccgaagagaatttgattggcatggagaataaagggtttgcccaagtgatgaacggatttgatcttagccgcttgttaatcggcttacaatgtgtcggtgcagccttccaaagtattgatgaaacgatagaacatgtgaaaaatagacactctttcgggaagccgttagcaacctatcaaggggtacaattcccgatcgttactcactatacacagcttgagcttgtgaagtggcaggcttatcgaggactttggctccgagatcaaggcttgaggcattccaaggaatcggcttcggttaagtggttaggccctaaatatagtgtggaagcgattcatgaatgtttattattgaacggtcactatgcctatacgaaggaaatgccgcttgagcaacgtttacgtgatgtgattggcttagaaataggcgatgggacagcgcaagcgaaccaaatggtcatcgccaaagatattatcggaaaagaattccgttcttattaa

SEQ ID NO: 287 - DNA, 468 bp, Peribacillus Aracenensis
  source 1..468: mol_type = genomic DNA
atgggaatgatagattgctattttatcggtcaaatcgcaagaatgcagaggacatttactgaaggcgatgtggaacgatggagtttgtttaccggtcatatcaccaaagtgaaaaggacctttgctgaggatgacactgagcgttggaatttgttgacaaaggaattaaatgagcgaattgaacatgagatttccatccaggatgtaagtcaaccttttgtgcctggaattttaagtgagggactgataacagaagcaatcagcaaggtattgccaggcgcaccatgtgtcattatgcaaaaggaaatggtgttcttacagcctgtttatgtaagtaacacggtaacggctgaagtggaaattatcgatgtcaatgttaagcgaaattggattacagaaaaggttcgttgtttcaatgaacttggaattgaattgattaaaggacaaattatcctgaaactactataa

SEQ ID NO: 288 - DNA, 816 bp, Peribacillus Aracenensis
  source 1..816: mol_type = genomic DNA
atggaggtcataatcacaatggaactaacagatgttttatatgaaaaaacgaatgggattgcaaagattacgattaaccggccgaatgtctacaatgcttttcgggcaaggtcgattcaggaattaatctggtccttccgtgatgcatgggatgataacagaattggggcggtcattttgacaggagccggggagaaggcattttgcgtagggggtgatcaaaaagaaaaaggagatgaaggcggatacgattattccggaggtttaggaggcggcatcggtcttgaggtcgaaaacctgcaccaaacgatccgcaatattccaaagcctgtcattgcagctgttaatggatttgcgatagggggcggacatgtccttcatgtcgtttgtgatttaacgattgctgctgaaacagcgaaatttggccaaagtggacctaaggtagggagttatgatgcggggtttggttctgcttatttggctagaattgttggggaaaagaaagcacgggaaatctggtatttgtgcgaacaatattcggcacaggaagcaaaagaaatgggtctcgtgaacaaaatagtccccgcggaacagctgcaacaagcagcggaagagtgggcggaaaagattctcgaaaagagcccgactgcgcttaaaatgcttaaatactcctttaatgcagacagtgcgaacatccaagggatttcacagctatcaatgggtagtctagcgatgttttacaacacagaggaatcagaagaaggaaaaaatgccttccttgaaaagagacctgtagatttcaagaagtttagatag

SEQ ID NO: 289 - DNA, 1692 bp, Peribacillus Aracenensis
  source 1..1692: mol_type = genomic DNA
ttgatactggatacgattttgagtcaaggatatatagagaagtatcaatctatatggccaaatcgaacgattttagattacttgaatgatgccatagcgaaaaatccaaaaaagatagccattgtcgataagaagggccgttatacctatggggaactcggcaagctagtcgatcgagtcgctttgggtttgcttgaaataggtttgggaaagggagatgtcatttcctttcaactgcctaactggaatgagttcattatccttcattatgcggcgactagaataggtgccatcagtaatcctttagtcccgatttatcgcgatcgggaaataggatatatggtgagcatggcggaatctaaaatgattgttgttccagatagtttccgaggatttaattatccggccatgattgagaggctgagtcatcagtggcctggattggaacatgtttatgttatcgggaaaaatgtaccgaaagggatgaaagcgtttaccgatttacttgaagaaccatgggaagagtggaaggatgcagctgtactggatgaaatcagccatgacccgaacgacgtgacagaaatcatctttacgtcaggaacgacagggaatccgaagggggttctgcatacgcataataccctctgtgtttcaacgaattactggattgatggattgggattaacatctgatgatgtcctgttcatggcctccacgtttgcccatcaaacaggtattggatatggagtgcgtttgccgactcattttgcggggacgggtgtttatcaagaggtttgggatgcacgcgaatttatcgagtggattgagaaagagaagattacgattacggcaggggcaacaccattcctgcaagatacgattcaaatcgaaggcatagagaattacaatatcagctcgctccgtacgtttgttaccttaggagccccgattccaagacagctcgtaaaagaagcgtccgaaaaggtgtcattcaaaatattgtcaggatggggacaaaccgaaaatggtctggtgaccttgacgcgtctcgatgattcagaagaaaagctggcgggtacggacggtgtcccttttccaggaatggagctgaaagtagtcaattctgaaggagagatatgtgctcctaatgaagaaggcgatttacttgctaggggacctgctatgtttgttgggtacttaaagcggttggaagatacgattgccgaacataaaaacggttggtttattaccggagaccgggcgatcatggatgaagacggatatatccggatttccggtcggaataaagatatcatcattcgcggcggtgaaaatataccagtcacttatgtagaaaatgtgttgtatgaacatcctgatgtatccatggcgcaaatcattgcggttccagatgcccgtcttcaggaaaaagcttgtgcatgtatcattatgaaaccgggtaaatctcctcttaccatggattcgtttagaggttttttggaagaaaaagggttagcgaaacagtattggccagaacatcttgagattatggaggagtttccagttaaccttagcgggaaaattcagaagttccgccttcgggaaatcatgaacgagaagatgagcagcaaattattaggaccaggtaggctcttacgagaggctgaatataaaaagataagtaaacaatga

SEQ ID NO: 290 - DNA, 750 bp, Peribacillus Aracenensis
  source 1..750: mol_type = genomic DNA
atgatgaatcaacgtgtagcatttattacaggggcaggaagcggaataggcagggagattgctaaaacattggcttctcggcatataaaaattgtcgttgctgatatcaatattaataatgcagaagaaacggtgtctttaattgaaaaagcaggcaatgaagcagctgcagtctattgtgatgtaacggatttggaaagtgtgaaaacggcagtacaggaatcggttagcatttataaaaaaattgatgtattgatcaataatgcaggctgggacaaagtagaaccttttctaaaaagtgagccgagtacatggaagagaattatcgatataaatttacttggacaagttcatacgtgcaaagaaattttgccgattatgattgagaatggttatgggaaggtcgtcaatgttgcttcagatgccgcaagagtcggttcgagtggtgaggctgtatactcggctgccaaggggggcgtaattgcgtttacgaaaacattagcgagagaaatggcccgccataagattaatgtcaattgcattgcgccgggtcctgctgacacgcctttatttcaggaaattggatcttacaatgaaggaattgctggggctttggaaaaagccataccatttagacgtttggcccagccagatgatatcgccggtgcggttgcctactttgtttccgacgatgcgggatatgtaaccgggcaaactctttcagtcaatggcggattaacgatggtctaa

SEQ ID NO: 291 - DNA, 1194 bp, Peribacillus Aracenensis
  source 1..1194: mol_type = genomic DNA
atgaaatctgtatatatacttgattctgttcggacggctgtagggaaaatgggcggaacgttaaaggatgttccagtggattatcttgctgcaaaagtaatcgaagaaattgttggacgaactgaaatcgagaagaatgccgtcaatgaagtgattttcggtcatgtaaaacaaagtgcagatgctccgaatattgctcgtttagctttgctgcgagctgggcttcctgttgaaataccagggtatacggtacataggcaatgtggttccgcattgcaggcaatcaataatgctgcacaactaattatgtgcggactgggagatattgtggttgctggtggagcggaatccatgagcacggctcctttttatcttcggaatgcacggtatggagtgggtaccgggaatactcaattgattgattccaatacggaaagccaatcccgttcgcaaccaatcgaggaatatggaaatttgacgatgggattaaccgccgaaaatttagcggttcaatatgatatttctcaagaagagcaagatgagtttgcattaagaagtcaagaacttgctagtcaggcgatagctgctggtcggtttgaacaagaaattgtcccgtatgaagttcgtgtccgtaagagtgtgaaagcctttgcggttgatgaacaccctcgtttaacgagtttggaaaaactgagcaccttaaaagcggtttttaaagaaaatggaacggtcactgctggtaacagtagcgggcgaaatgatggggcatccgctgttatagtcatgtcagaagatgcagtcaaaaggtatggtgtaaagccaaaagcgaagattatttcgcaagcagtatcgggtgtatcacctgaaattatggggattggccccgtgaaggcgactcaaatagctttggaaaaggccggtttaaccttggccgacatcggcttaattgagctgaatgaagcttttgccgcacaagcactggcggttatgaaagaactaaatcttgatttatcgaaagttaacgtcaatggaggtgcgattgcgcttggtcatccgttaggagcgacaggggctattctcacgacgaagcttcttcatgagatggaacgaaggggtgagaagtatggattggtgacattgtgtattggcggcggacaagggattacaacgattgtcgagaactgtcaagtatag

SEQ ID NO: 292 - DNA, 813 bp, Peribacillus Aracenensis
  source 1..813: mol_type = genomic DNA
atgggacgcggaattgcgtataccgctgctttggctggatttgaagtaacgctgcaggatatttcagaacaagcgattgaaaaagcaagagagtatatagaatcccttttaaatacaagcgttgaaaaagggtatatcccgagtgaacaacgagttctggttcatcggaatcttacgtatacaactcagataaaggaagcagtgcagcatacagatttagtgattgaagcagttttagaagtgatggagttaaaaattgaaatttttaagcaaattaatgagtttgctccacctgaggccatttcggcaacgaatacatcgacgatgagtccgaccgaaatcggcgcaacaacgaaaagaccggatcaatttgtggcgatgcattttttcaatccagtccatcgaatgaaattaattgagattatacgcggaattgatacgtcagatgcaacggtagaagtgatcaaatcagtcgctgaaaaaatgggaaaagaaacggttgaagtgaatgagtttcctggatttgtgacgagtcgtatgaattgcataatcggaaatgaagcgatgaatatgctaatggaaggcgtggcatcggcggaagatatcgataaagcaataaaactcggcttgaatcacccgatgggtccgctcgaaatggctgatctcgttggattagatagccgtctccgaaatatggagtacctttattacagtctaggagagaaatatcgcccctcccctttacttgtgaaatatgtaaagtcaggacgtttaggccgaaaatccggccagggattttttaaatataattga

SEQ ID NO: 293 - DNA, 1158 bp, Peribacillus Aracenensis
  source 1..1158: mol_type = genomic DNA
gtgtatattatgaattttgaactatcagatgagattaagtctctaaaacaaggaattcgagaatttattgataacgaagtagatccgcatgccttgttaatagaagaaagcaatgaaattccagcgagtattatggaaaaatcgaaaaaaatgggattatttgctcttagcgttccggaagcatatggcgggttagggcttagcatggttgggaaatgtgccgttcttgaagagttgggaaggacgcataatggttatacaacagtcattggcggacatacgggaatcggtggcgttggaattgttgagatgggtaatgaagcgcaaaaacgcaaatatttaccggacatggcatcaggcgaaaggatcggcgcatttgctttaacggaaccgagtgcgggttcccatgcgaccaatctcaaaacgacggcggttcgaaaaggagacaagtatattttaaacggatctaagcattatattacaaatgctccgatcgctgatatctttacggtcatggctgtcacagatcctactaaaggagcaaaaggaatcacttcttttattgttgaaaaagacttcccagggtttcaaataggaaaaattgaaaagaagatgggtcttcatggatctcattcatcagaagttttctttgaagattgtgaagttccagttgagaacgtattgggtgaagagggacaaggttatgtcaatgcgctgaaaatcttggcgaatggacgcgcaggaatggcagcacgaaaccttggatcttgcgataaattgcttgagatgtcgctagattttgcccatatgagaattcaattcgggaaacccattttcgagcaacaaattatccaacattatttggctgaaatggcattggatacggaagcccttcgtgcgatgacctatcgtgtcgcgtggatggtcgatcaacaaatgaacgtcataaaagaagcggcaatggtcaaattgctaggttcagaaacgtataatcgtgttgcagataaagctgtccaaattcatggggggattggttacatatccgaatatccaatcgaacgtttttatcgtgatgcgcgaatcacgagaatttacgaaggaacatcggaaattcagaagaatattatcgctgcccagatgcatcgaaactataaataa

SEQ ID NO: 294 - DNA, 780 bp, Peribacillus Aracenensis
  source 1..780: mol_type = genomic DNA
atgatatatcaaaatatattgcttgaaagagaagaccggatgggcatcattaagctaaatcgacctgaagtaagaaatgcgttaaataatcaaacagtgaatgagatcctgtcggctttagaagatttagagaatgataaggaaataggtgttattgtttttacaggtgtaggggagaagtcctttgcagctggagctgatattaaccaagttatgaccagaaaatccatagacgcactcacagcaggtggtatgtctgaagtgtatcgtcgaatcgaaaatagtaaaaaagcaaccattgctgcaatcaatgggtttgcactcggtggagggtgtgaactagcgatgtcgtgtgatattcggatagcatcagaaaatgcaaaaatcggactgccggaattaaacttatctgtcattcctgcggctggtgggacacagagattagctagaatcataggtaagggcagggccatgaatatgattttaacaggagaatttatagttgctaatgaggccaaagaaattggattagtttcggatgtcgttcctttggtgaatttgtgggctgctgtacgagaaaaggctgaacgaattgtagcaaagggaccgcttgcggtacaaatggcgaagctcgttgtgaatcggggatttgatgtcgatatggatacggcattgctgttagaaagcttagcacaagccgttttatatggaacggatgataagaaagagggaacacaagcatttcttgaaaaaaggcaagcttcttttacaggaagttaa

SEQ ID NO: 295 - DNA, 756 bp, Peribacillus Aracenensis
  source 1..756: mol_type = genomic DNA
atggatctcggtttgaaagggaaaaatgttttgattacgggtgcggcaaaaggaattggccgaagaattgcattggcggctgccagtgaaggggcgaatattgcgttgcactatcgcgagtctgaagaggcagctgaggaaacagctaaggaaatcagcgagtatggtgtgaaagtgagcctggttaaaggggatattgctagattggaagatgtcaggcggatgaaggaaacgcttgatcaggaactcgagagcgtcgttgattttattgtaaacaatgccggctggacgcagatgaaatcgttctttaaatatgaaccggaagaatggaagagggaagtggatgtttgtttttacggggtattgaatttggcacacacatttatgcccgaaatgattcgtaagaaccaagggaagtttatcaatatcataggtgattcagcgaggacgggtgatcgaaatttaattgtttcagccgctgctaggagtggaacgattagttttctaaagtcattggcacaggatgttggtagaaataatgtgcaatgtaacacggtatcacttggactgattgaccaaggtgcatttggctttaatgaagcaacattggataagcttattaagcaatatcctttgaggagacttggaaaagtggatgatgtgacggggatgattttatttctattatctgaatccgcggattggattaccgggcaagtggtgtcggtgaatggcggacatagtatgttggggtag

SEQ ID NO: 296 - DNA, 771 bp, Peribacillus Aracenensis
  source 1..771: mol_type = genomic DNA
atgaacatttttgtcattatgaagcgcacgtttgataccgaggaaagggttgcgataagcaatgggcgaattgatgagggtggagctgaattcatcatcaacccttatgatgaatatgccattgaggaggccattgtacttcgcgaccaacatggcggtgaagtaacggtggtaaccgttggggaagaagaagcggaaaaagagcttcgtaccgctcttgcgatgggggctgatcaagcggtattgattaatagtgaagatatagaagagattgatcaatttacaacagcctctcttcttgccttgtatttaaaaaagcaggaatatgacatcattcttggaggaaacgtcgcggtggacggcggatccggccaaattgggcctcgtctttcagaatcacttgggatcccacaagtgacaacgattaccaatctgggagttgctaatgggaaagcgaccattgtccgcgatgtagagggagacgaagaaactgtcgaagtgtcattacctgttctcgttacggcgcagcaagggttgaatgagccgcgttatccatcgttaccggggattatgaaggcgaaaaaaaagccacttgaagtggtcgatttagatgaccttgacgtggatgaggacattgtggaagcaaagacaaccactgttcaagtgttccttccgccagccaaacaagctggaaaagtgctggatggagacgctactgaacaagtcaaagagttagtatcacttttaatgtctgaagcaaaagttatttaa

SEQ ID NO: 297 - DNA, 987 bp, Peribacillus Aracenensis
  source 1..987: mol_type = genomic DNA
atgacaaaaaaagtattggtagttggcgaagttcgtgacgggcaattacgtaatgtatcatttcaagcaatcgcagtagggaaagaagcagcagggggaggagaagtggtaggtgtcctcctcggcgataatattgaccatttagcaaacagtttactgcaatatggtgcggaccgtgtcgtggtcgtgaatcatggggaccttaagagttacacaacggatgcttatcaacaagcgcttcttcaagtgatcgacgcagaaaagccggaaggcctgattctcggtcataccgcaataggaaaagacttatcaccgcgtatcgcgatgaagttaaacgcgggattaatttcagatgtcattgccgttgaaaaagatggagatgaagtagtgtttacacgaccgatttactcgggtaaggcatttgagaaaaagaaagtcaaggaagggttgatctttgcgacgattcgtcccaacaatattgcaccacttgagaaggatgaaacaagaacaggagagatcacgagtattactgtagacattaaagatcttcgtacggtgattaaggatgttgttcgaaaagcatctggaggtgttgatttatctgaggctaaagttattgtctcaggtggtcgtggagtaaagaacaaagaaggatttaaaccattacaagagcttgcagacgtattaggtggcgcagtaggtgcttcacgtggagcgtgtgacgcagattattgtgactactccttgcaaattggccaaacagggaaagtcgttactcctgatttatactttgcggttgggatttcaggcgctattcagcatttagcagggatgtcaaattcaaaagttattgttgcgataaataaagatccagaagcacctatattcgaagtagcggattacgggattgtcggtgatttattcgaaatcgtccccattttaacagaagaactaaaaaatgttctgaatgtaaaagaaacagtctga

SEQ ID NO: 298 - DNA, 2109 bp, Peribacillus Aracenensis
  source 1..2109: mol_type = genomic DNA
atggtcatccacttaatggcttttcttctcatcatggcttatgcattctatttgtttgcttccctcgtgaagactcgttatgagtatattaaacttggtaagaaagccgagttcaatcattcgatgaaagaacgatggactgctgtattggttaatgtgtttggacagaaaaagttgatgaaggataagaaaagcggaacaattcatgtgatgtttttttacggatttttgcttgtccagtttggagccattgatttaatttggaaagggttagcaccgggagcacatttaccgctcggtgcggtgtacccatactttgcattgttcgaagaaatggttgtatttatgatcgtcatcgcagtcgtttgggcgttccaccgccgctatattgagaagcttgttcgcttgaaacgaggctggaagtcagggcttgttcttgtttttatcgggggattaatggtctcaaagatgttcgcaaaagggatggagataatttggcttggaaaaccactgaccggatttgagcccattgcatcaggaatcgctgctgcgacaagctggctcggtccaattgccgctggcgtgttgttctttgttttctggtggcttcatttactattcttattatcctttttagtctatgtcccacaatccaagcacgcccatttgcttgctggacctgtcaatgtttttctagggcgtacacataaggttggtcagttatcgtctattaatttcgaagacgaaacgcaagaagtttatggtgccaacaaaattgaagattttaaccagaagcagcttcttgatttatattcttgtgtggagtgcggccgatgtacgaatatgtgcccagcaacaggaacagggaagatgttgtcacccatggatctcattgtgaaaatgcgtgatcacttaacggaaaaagggacagctatcacctcaaaatcagcatggctcccagagtttgtctttagcaatgcgaaggcacacaggcctacattacagggagcagcagaagtagctgcagggtatgatgtcagcttgatcggcgatgtcatcacggtagaggaaatttgggcctgtacaacatgccgtaactgtgaagatcaatgtccggtaatgaacgaacacgtagacaaaatcattgatttacgccgttacctcgtgttaacggaaggtaagatggatgcagatgcccaacgtgctataacaaacatagaacgccaaggaaacccgtggggaatcaaccgcaaagagcgtgaaaactggcgtgaaggacgggatgatattgaggtgccgaccgtcaaagagctggagaaaaatggggaagaatttgaatacttattctttgtcggttcgatggggtcttacgataatcgaagccaaaaaattgcgcagtcattcgcaaaagtgttaaacaaagcaggagttaaattcgcgattcttggaaataaagaaaagaattcgggtgatacacctcgtcgcattgggaatgaatttttatttcaggatctggcgaatgcaaacatcgaaacgttccaaaaacataatgtcaaaaaaattgttaccatggacccgcatgcctacaacacgttcaaaaatgagtatcctgagttcggattagaaggcgtagaagtctaccatcatacagaactgttgtttgaactgatacaagaaggaaggattacgccaaagtatgaagtgaatgaaacggttgtataccatgactcctgttatttagggcgctataacaacgtttatgatccgcctagggaaatattaaaagctattccgggtgtggaagtgatagaaatggaacgcaaccgtgaaacagggatgtgctgcggagcaggaggcggtatgatgtggatggaagaagacaccggtcaacgcatcaatgtggcacgtactgagcaggcattggccgtcagcccaagcgtgattggcagcggatgtccgtattgcttaaccatgttaagcgatggaacaaaagcagttgaaatggaagagaatatccaaactctagatattgtggaaatattggaaaaatcaatttttgtgcaaatatcatgtgatagcaatctggaacttacaggatttttaaaatga

SEQ ID NO: 299 - DNA, 513 bp, Peribacillus Aracenensis
  source 1..513: mol_type = genomic DNA
atggaagcaaaatattgtaaggaatcacgagtggtacgaacaagtcgtgtattcccaaatgatgtaaatagtcataatacgttatttggcggtcggttaatgagtgatttggatcaagtagcctccatttccgtattacgacattgccgaagagattgtgtaacggcttcaactgattcagttgactttttacatgcgatccgaccatcagatgcggtctgctttgaatcgtatgtaacatgggcgggtaaatcatccatggaagtgtttgtgaaaattattgccgaagatctaaaaagcggcgagcgtaaaatggcagcgactgccctcttaacatttgtcgcgcttgatcaacacaaacgtccaatacctgttccaccagtcattccggaatcagaagaagagagaaaattacatgaaaccgcaccagagcgagcaagaattcgtaaaaaaagaagacaaaaaagtaaagagttggcggtgtatttaacaacgaatcatccctgggattga

SEQ ID NO: 300 - DNA, 165 bp, Peribacillus Aracenensis
  source 1..165: mol_type = genomic DNA
atgcgtagggctcatcaatataggcctgagtggagtattttgcttcaaaatatactcgataaagataaagaaaagtttaccatcgttcttgttttccacgacgatactaaatcatatgagttaaaaaataatcaatggattgttgatgaagaaaaatggtcataa

SEQ ID NO: 301 - DNA, 759 bp, Peribacillus Aracenensis
  source 1..759: mol_type = genomic DNA
gtgacatacgacctcgagcacattgttaattttggaaaatgggataccaagaatttcagatggaatacttcctcctttaaactttccaatcttaaaggtagaatgactggtggtgtcgcattgacaggaaactacgagaatacaaaatacaataagttagatcataaatactctggtgttgaactaaaaagtggcacattcaagtattcctggaatcgtacgatgcctttaggtccaaaaaacaagaacgctcactatgatgtaacaacaaaatctggctgggcaacgccatcaatcaattgtaataacgaagcaaacgttgttttagacgttggcggcagcgcatcatctcttgcttatttggatgaggcagcaagttttgaaacttattctgacgaagatatcccgactgaatttacagaaaaggcagagagcttatctgaggctataggagacgattttgacggacaagttgaaccattaggcaaggatgtcgttgtcagtcacttcgatagtgcaaagaaagatactatcattctaacccaacaaaatgataatcctatcagtgttaatgatgtagatgacgaggacttttctaaagttgtggtagatgatgttgcatacgaaataggccattttaaaaatgctgcagatgaaaaaatgaatgttgtaaagtttgaaaaggacggaatttacatggcgttagttacaaatcaaacgaatgaagaagctcttaaacttgcagaagaattgaagtga

SEQ ID NO: 302 - DNA, 291 bp, Peribacillus Aracenensis
  source 1..291: mol_type = genomic DNA
gtgcaaggtgttgatgaggacggggtatcttccgagtcaacttcaaaggtcattacagacattaatgaaatacaagcttttgtagaaaaattgaacaaattggaagttgtgcaacttcctaataaggagttattggagaagagtaaagaattaaataaaaaagggaattacttttttataggctgttttcgcataatttgttgctatttaccaagtaaagcggtgtggttgatttcccctccagatgctgctcccgcaggagtctcgcacttgcgctccaatcaaccttaa

SEQ ID NO: 303 - DNA, 879 bp, Peribacillus Aracenensis
  source 1..879: mol_type = genomic DNA
atgttgagagataaaactgttgcatttttaggagccggttcgatggcagagtcgatgatttcaggaattgtgcagatggggagcataccagcagagagaatttatgtgacaaatcgccgcaatcaattacgactcaaggaaatgaatcacgtgtatggcgttcaggcggtccatcaggatgcattgccatatgaagaagttgatttctttattttggcaatgaagccccagggagcagcagatgctctcgatgcattgaaagataaaataaaagtggatcaagttgtgatttctgttttagcgggcatttccactgaattcatggaaagtcatctacagcttggacagcaagttgtgcggttgatgccaaatacgtcgagcatgatccgggagtcggcaactgcgttatgtccgggaagacatacagcgatggacaatgtgatagcagtgaaggaactgtttggctgtttgggaaaagtgttcttaattgaagaagagcaaatggatatttttacaggaattgcaggaagcggacctgcttacttctattatttaatggagcatatggaatatgccggcgttaaaaagggcatggatgaagcgatggtccgtgagattgtcgcccaaacgattttaggggcagccaagatgattatggtgaacgacgaggcaccggcaagtctcagagaaaaagtcacttcaccaaatggaacgacagcatccggacttgaggctttacggaaaaataatggcggcagagccatttcacaggcgattcatcatgcagcgaaacgttcgaaagagctgaatgaagagatggcagtagcgtacaggaaatcgactattccccgagagtattgtggcacttcagtaccataa

SEQ ID NO: 304 - DNA, 1059 bp, Peribacillus Aracenensis
  source 1..1059: mol_type = genomic DNA
atgaagagaatccttaagatcgctagtgcttttatcggaattcttatcggagcagggttcgcctcaggacaagaaaccatgttttattttgtaagcttcgggaaattgggcacaattggagctatcatttcagtcgctatttttggataccttggaatgattttgatgaagcttggcagtcgtacacaaacagattcgcatcaggaagcaatttataagatttgtggtcgctttctcggcggtatcattgattatgttctgaacgccatcctaattggtataggaattgtcatgattgcggggtcaggctcgatctttgatcagcaattcggattaccttcctatataggcaccattcttatgactgttcttgttttgataacagttatgctgaaagttgaccgtgtgattaaggtaattgcatccgtcacaccatttctgattcttgtcgtactctttctatttatttatagtatgtttacaatgaattcatcgtttacgtcacttgaaccacatgcaatggaacaaaattcagctgcgggacattggcttatatctgtaataaactatatttcaataaccattgcaatgggggcttccatgacacttgttatgggtggaaatgaacctgatgaaaggatagcatccattggaggacttataggagggcttgctttaggtctacttgttttgattagtcaccttactattttctcacatattcatactgtatcggacttagatatgccaatgctgggaatcgcaaacagtttttcacctctcttaggtattctgtactctctcgttctgttcgctatgattttcaatacggcagtcagcatgttctactcatttggaacacgcttttcaaatccgcagaccacaaaatttaaagtaatcgttatttcatcactgttgataggatttatagcaagcttctttggcttcactaaacttgtttcctctctctatccaatctttggctatatgggaattgttcttattatcgttctcatcattactccattccgaatgagtcgattaacgaaagaaaattaa

SEQ ID NO: 305 - DNA, 150 bp, Peribacillus Aracenensis
  source 1..150: mol_type = genomic DNA
atgatgcatacaagaaaaaggattgcagtaagatgcggggatacttcctctacgatagcttttattaatgtccatataaaactatctccaaaaatgaaaaataaaattacaaataagaaatccaatgtatacattcctttcgaaaaataa

SEQ ID NO: 306 - DNA, 1929 bp, Peribacillus Aracenensis
  source 1..1929: mol_type = genomic DNA
gtgagtagaattttgttagaaaaggtttcaataatcatacctttccaaacagacaatggcccaagagcggaagcatttaaatggattaaacagtattatgaacgtatcatgcccgaagctgaattatgcttgggtataatcgataacgataaaattaataaatccaaggctgtaaacttagcagctaaaaaagcaacaagagaaatttttgtaatagctgatgcggatatcgtttatgaccctaaacttatagttaaagcaatagaggcacttaatgaagcagcatgggtagttccttttactgaaatttatgacattgaaaggtcaggaacagaaagactaattcaaacagaaccaacgtggccttttgatgttaaatctgaagaatgtaccaaagcaaattggatttacacaggatttgcgggaaaacttattgtcatacccaaagtgaactttgaggcagtcggagggtttgatgaacggtttagtggctggggaggcgaagatgatgctttttcactttctgtccagacactttgtggtaaattagcgaatgtttcaggagaaatttaccatgtgtggcatcctgtttcaaactacggaacaaatccaaatggtaaagcgaatctagaacttctcaaccgttataaacgcgcaagtggaaatagaaaggaaatgaccaatcttatttctgaacgaaagaataatatagaaaagatacaaattaataatattgaggttttaaacagcattgcaaatgcacatatgacatcacctaaaagcaaaatttgttttgccatccttgttcatgaaaagagagagttagtcgatcaactaattaaaaatgtccgttctttttgccctaacagtgcaatcgtcttatacaacgggggatctgataggacgctttgtgaaggtctaggtgttcccgtttgcccctccagtcgtaaattaaagtatgggcatactgccatttattttcttgaaacgatggaatggttggaacaattagggactcagtatgaatattttattaatattgactcagatgctttgtttatcaaaaaaggatatgaagaattcattcaaaatgaaatgaaagatacggattacatgggggtggactttagggttccaagtaaagattggtatattggaagggaacttgagaaagacgttaatagatggaagaaattatttaatattaatcctttgtatggagttttcaatgttggacaggtaatttcgaggcctattgttaaagcattacttgaaccagaaaggatgggaaagttaagaaaagctttaatggaaactacttcctgggggatggatgagattatctttgtaaatatggccaaggaacttggattcaggcaaaaaaaatatccaaaccccctggactcagagatgatacgttatcgcccttactttacactggaagaaatgatatactaccatactaaaaatagcggttatctatgtcatcccattattcgagacaaagctgaccctgtcaggaaattaatccaacatattgaaaagggccatgattcagatctatatacaaacaaggaatatccatggcatgaagacaatccaaataattattccatttcgcttccgataaaaggcaaatttggtattttagagcttgtcgttcgctctggttctgctttgacccactattggcaacccccggggggggaatggtataaatctgagatattcgctagaggtgttacgggaattcctatattattcgaaactcattcaggtgtatttgtggtagtatgcaaattaataaatggtgaagtttgcttttggtggagagacagcaataaccagaacagcccttggtatggaccatctgtttttcagcttgggaatgtaaatccgataaaaggaagtgaatttattaaagagtaa

SEQ ID NO: 307 - DNA, 489 bp, Peribacillus Aracenensis
  source 1..489: mol_type = genomic DNA
atgggtttagagtatctgagtgtgggcggggcaatttctgatttggagagatgtaatgtgaaacttggtatcatgtgcggaatcccattaagcggtaaatcaacatatgctaaagttctacagagcgacggatgggtacgtgtatctattgatgacctcaggctttccttacatggtcaaatttataaagcagaggctgaaccacaagtgtggaaaacagctgaacttatggtcaggtcgttgctaaaaagtggtcataaagtaattgtagataccacaaacagaacaagaaagcgtcgtaaacaatggagacgtgtggctaaagaatttgggcttacgttagaaatttaccaagtggatacagattatgaaatatgtaaagcaaggaacaaagatctaatgcgactacctcaagatgtattaaaacaaattcataaagaataccaaaaaccgacatcggatgagggaactattattatggtaaattag

SEQ ID NO: 308 - DNA, 894 bp, Peribacillus Aracenensis
  source 1..894: mol_type = genomic DNA
gtggaaaagtatatttcttttgatgtcggcgggacaaaagtaaaacacgggctcttattagagaacggaaccattctttcacaaggcagttacagtaccccgtgtacaaatctggataaatttataatgaaaatggtagaaacaattaatatgtacttaagaaataatcatgtgttgggtgtagctataagtttaccaggctttattaacccgaatacaggttactcagaacaaggtggtgctgttaccgcgttgattaatcagaatttaaagaatttattagaagcaaaagttcctctacgggttgaaattgaaaatgatggaaactgtgctgctatagcagaaaaaacaagcggtaatgcccaaaattgtaccgattttatatgtgtcacaattggcactggaataggaggggggatttttgttgacggtaaacttttacatggtcatagatttagaggcggtgaatttggttttatgattactcaagcaaatgggaaaaatttcggtgatatatggcactccacaggttcaacttctgccttaattaggagctataaaaaacttaagggaataagtgaatatgaaaatgttaaaggggagaccgttttttcagaggccactaaaagtaaatcggtaaaaaaacttattgacggatgggctagaaatattagttatggaattttcaacctagcagcaactttaaacccacaaaaaattttaattagtggcggagtatcctcccaacaggatttgttatcaactataaataaacaactagacggtctcccttggtggaatgatattaagattcctgttgaactatgtaaacatcgaaatgaagcaggaatgattggggcaatgtatcattttattcaacaacaaagattataa

SEQ ID NO: 309 - DNA, 786 bp, Peribacillus Aracenensis
  source 1..786: mol_type = genomic DNA
atggatattcataaaccatttaacgataaaatgagaaaaaccttagtattgctcaatgatcccctagttaaggattatattccggtgacggattggttcactgaacgaaaggcaaaaaaattgataaaaacctatcccagtctgtttattaaacccaataaaggaagaataggtataggcgttatgcgtttaagaaggataggagactctcagtatgaagttcactatcaagataaggcagaaaaatatgagacaatagctcaaggattagcagctttgaaaaaaaagtttaatccatcaaaaaagtatcttattcaacagggcattgatcttgccaccgttctcgaacgtccgtttgattttcgagttgtcatgcataaattcaatggaaagtgggaaagatcgggctggtgtgcaaaaatttcacctcccaaaatgattgttactaatcatgctaaaggaggtataataatttccgcagaacaagcattagcagctaataaaagtaattttgattataataaggcactaaatgagttaaatgaagtatgtcacaagatatgttcggtatatgattcccacttttctttttgtaaagtgggtctggatatggctattgataagaatggacacatttggtttattgaagcaaatacttcaccagatcaggccatgtttcgtaaattaggagatcaacgaatatataaagagataaaaagtaaagatttacaaatccgtagaataagtaagaaaatattaaaagatttaaatcacaattcagaataa

SEQ ID NO: 310 - DNA, 1179 bp, Peribacillus Aracenensis
  source 1..1179: mol_type = genomic DNA
atggaaaatgtcagagtatacgggagggcaaaacaattgagtactttaaaacggcctattattggtgtcttcattccccatccaatcatcaaagctttaaataaacaaaaagatacattgaaaagctatccacgaattttacaacttgcaaaatcaagtaaaaaagcaggtgtgaccctattttttttctcatttaaaaactttgattttaagcagaagttaatctttggtacatattttgataaagattcgaagaaatggaaacaaacatattaccctttacctgatattctctataatcgcggtgcaggcggaggggcaagtaaatttattgcagaacatatattagatatacttgatgaacatcaggtgataaagcttaattcaaaatcatactttgataaatgggaagtataccaagatctaagtcaaattccagaggttagcaaatatcttccgtattcagtcatgtataaagaggatagtgatttacaaagatttttgaaacagaataatgaagtttatttaaaaggagtgcgaggtgggcgggggaaatggattttccgaatccgcaagcagccaaatgggcacttcgaatatggttaccatggtaataacatggttatcgccgaagaaaaaaaatgggataatttagtccaaaaaattcataagttttatggtaagagagaatttataatccagaaagctattaatctattaacattacaggatagtatagttgatttccgtgccgaattacagagagacggcaaaggagagctaaaaattattggagttgccgcaagaatagggaaatcgaaatcgcccattaccattcattcctcagcatatccgattgagtattttttcaaggaattccttcattattctgaggaaaaggtaaatgaattaatggaaagcattaatgaatttcttattacaatttatcatgctttagaaaaagtgtatgggcaatttggagaaattggtattgattttgggattgatcaaactggagagatatggtttattgaaccaaattccaagtcagccaaagtttcccttatgaaagcctatgataagaagacgtttaaaaaatcgtgcttaaacccactattattttccaaatacctttatgagaaaagaaaagaggaaatgtcagaaaaaatgttaaattaa

SEQ ID NO: 311 - DNA, 1179 bp, Peribacillus Aracenensis
  source 1..1179: mol_type = genomic DNA
atgatggtgaaacctaaatacattacgaatattagtcatattcaacacttgagtgaagaagaaaaaagaatactccaaaccgtttcggagaaatttgttttccgcttaaatgaatactacttaaaccttatagactggtctgatccacaagacccacttcgcaagctggtaattccgtcgtccgaggaattattggaatacggcagatgggacgcatcagatgaggataccaactatgtcgtacaaggttgccagcataaatactctactaccgctttacttttggtttctgaagtctgtggagcctactgtagatattgttttcgcaagcgcttgtttcgttcagatgtaaaagaagcgtcattagatatggcagatggacttgaatatattaaaaaaacaccagagattaataatgttcttcttacaggtggagaccctttgatactaggcactccaaagttacgctggattattgaaaatttacgtaatattgaacatgtacaaattattaggatcggttcaaaaatacctgtatttaatccaatgagaatatatgaagacaaagaactattagatttattacgagagcactcttctgtgcacaaaaagatatatgtaatggctcatattaatcatccccgtgaaattacatccgatgcacttaaagctattgaagccctgcatgaagcaggagtaatcattgtaaatcaaactcctgtactaaagggaataaacgatgatccaactgttctcgctaatctgttagataaactatcttgggcaggagtgaatccttactatttctttgtaaatcgccctgtagccggaaactcttcgtttgttctaccattggaacaggtatatcaaatagtggagaaagcgaaggccaaaacctctggcctcggcaaacgagtcaaattagttatgagtcatacttctggaaaaattgaaattctcgcgattgagaatggaaaggcatatcttaaatatcaccaatcgcgtgatggtgtttatggaaagttgatgattttggactgtccaccaactgcttcctggtttgatgacttaccaaataacgagcaattttgggaaaaaccaactaaaatgacggatagtgttgtctctgtgaaccagctacctcccacccctcagaataaacgtccttctaatgattaa

SEQ ID NO: 312 - DNA, 363 bp, Peribacillus Aracenensis
  source 1..363: mol_type = genomic DNA
atggatgttccagaagaattagacctaatttctgtatttggagctattccaaagaggaaagatgagacagctgctttttattacgacacatcaacatttgttttagaaaatgaaaaagaaaaatatgagattatcctttcccctttttatcacgaatttagtttaagtgttaaggaaatgaaaacaaataaagtattgtcatatattgaattactttctgttaataaaattgagattgtggaagacaaaaaggagcattcaaaaattcgtttgtttcacggcgattcggacagatatgtaaatattatcgaaataactttaaagcctagattccatgtgattttcagagaacaatattgttga

SEQ ID NO: 313 - DNA, 399 bp, Peribacillus Aracenensis
  source 1..399: mol_type = genomic DNA
gtggcatataaaccccactgcatttatgatgcaggccttttaaattattatttgaggcaaaaactaattggtgtgattgtcctagagatggcatttgctgaaggctcagcaaatgattggctacccttagctatggttgatggctttcatgttgaccatgttacgagtacagctatttatggagtattcttaacagcaatgcttatcggaagtgttacagcaggagcatttcttgataaatatggccccgttcctgttcttcgctttgcatctgtattagcagtgataggaatggctcttgttatttttaactcgaatttcacaataggtgtaatgggtgttttcatatggggactaggcgccagatgcgaagttagagttttggggagaaggtactga

SEQ ID NO: 314 - DNA, 2193 bp, Peribacillus Aracenensis
  source 1..2193: mol_type = genomic DNA
ttgaaattgaaaaaagtatcagtaattattgcagtatataatacagaagaatttttagatgagtgtttaaattcagtggtgaatcaaacatatagtaacttggaagttctacttattaatgatggatcattggatcagtctggtgctatcattaatgaatttgctaagagggataaacggattatcagcttccataatgatgagaggaaaggagtgggagcagctcgtaatctgggtttagataatgctacgggtgagttcgtatactttattgatagtgatgattttattgctctcgatacaattggaaggttggttgagaatattgggaaacacgatattctttccggaaagcaaatccggttaattaataaagaggatagtaaaatcgggaatatggttgaagaagaagctgatgatggaatggtaatagacgagattaaagagaaagtgcaaaaaggacgtgtacgtttaagaagagggattcaacaatcgtttcgtggtatgtctatcctgcacactcttatttcgcatgattttataaaagtgaataatttgcggttttcagaagaagtgcattgttattcagatctatccttaatcgttcctatcataagtgaaatgaggaaattcccacttttaacacgttgctattatttcaagcgcaggcgcaatgaccccatctccaatcctgcattaatgcaatcggatcgggaaaaaaaggttttggactttttatcaatctataatcagatgaaagatcaatatagtatggaccaacgagctggttcatatctagactggttatttttaaatatatatcgaaaacagattatcatgctattttccaatcaaggatgtatcgatgaattttttaacaaagtagccgtttctgttgataaaattgatgtatcaaaaaggaaaagtcttaatgttgtagtgaaaagagagctaaagctattacgtaaaaggaaactaggatcttataaaaagctgataggtctccatcattttgcccgtaacatgaagagggcattgaagagcaggcagaaaatgtacatttatttatatcgctctgtgttcatgcgtataccactaaaagaaaaaacaatcgtattcgaaagtttcttagggaaaaactattcagatagtccgaagtacatttatgaatatatgcttgagcataatcccgattttaaatatatatggatttttaataagacaaggaaagagattccaggtaatgcaaaacaagtgaaacggtttagcttagcttactattattatttcgcgacgtctaaattttgggtaagtaattcacgccttccacttaaattaaataagcgtgaagggaatatctatttgcagacttggcatggaacaccgttgaagaagcttgtttttgatatgaatgatatttattcggccaatccgaattataagaagcatttctttaatcaatcaagacgttgggactatcttatttcaccgaatcaatattcttcggatatatttagaagtgcctttaagtttgaaaaggagatgctcgaattcggttatccaagaaatgatatcttatataaaagggataatgaggagtctatccaaaatttaaaagagagtctccaaatacctcttgataaaaaagttatcttatacgccccgacgtggcgggatgatgaattttatgaacctggaaagtataaatttgccattcaaatggatttacataaaatgagagaacaattaggggatgaatatgtcgttttattacgcatgcattactttattgccgatgagatcgacacagatggtttagaaggttttgtatataattattcaaaatacgatgatattgctgaactttacttgatttctgatttattgatcactgattattcttctgtattttttgattatgcaaacttgaaacgtccaatcttgttttttacctatgatcttgagaaatatagagatacattaagaggtttttatatagatattgaaacagaagtgcctggcccactagtgaaaactacggatgaaatcattgatgccgttacgaatattgaacaagttaaagcacaatatcaagagacgtatgatcgcttttacgataaattctgcggttgggataatggcaattcggctgagaacgtcgtgaaaaccgtatttggcttgggtgtaaaatag

SEQ ID NO: 315 - DNA, 1095 bp, Peribacillus Aracenensis
  source 1..1095: mol_type = genomic DNA
atgggggaagggttaaataaaaaaactcgatatttttacgagttgaattttatacgtgctattgcttgtttatgtgttgtgatggttcatgtctcagcaaaaaattatcatttaaatgatcagaacttcaattggctgacactatttttaaatcaagttgcaagatatggtacaccatgctttgcaatcttgagtggttttctgttatacaatcaagcaattaaaaagggatttaattttaaaaagtttgttacatctagatttaccaaaattgttatcccatttcttatatggagttttctttatttacttgttagacaatataagttcccttggtctgagggaggagtcagtataaaagattttttattacttttctcacttggtgatagttattatcatctttattttattgttgtggtgattcaattttatttactattccctattttgcaattggctaaaacgaaaaatagtatgttagctttaacaatcatagctctttttataaattattattttatgcggcaaccatttgatacaggaaatgaaacttttaatctacttatccaggatagatcatcaatatttaagtggattttttattttatcttcggaggacttttagtatacttttgggaacctcttgtaaaatgggttgaaaaaaatgtgaattttagtattttactcggtgttattagtatatgtttcgttacatatgagtacaatacattcggttttttttcatctacgcgcattgctaatttgtttcacatgccattatttctcgttgtactaattggtgtttattatgttatggagcgttggaagaaaataagaaactatataatggaacttggtaatttatcaatgggtatttatttagttcatccaatggtgttatatgtaatacaaaatcacatacctgaactattaactcaaacaagatggattcctttagcttttcttattactgtactttcttcgattcttttagttaaaattattaataaaattccgtttggtcaatttgttgttacagttgcatctccaaaaaaagtaaaatatcaagaggtacaaaggaaagctagttaa

SEQ ID NO: 316 - DNA, 219 bp, Peribacillus Aracenensis
  source 1..219: mol_type = genomic DNA
atgcaaaggatgaatgataaaagcttttttaactttacccaggatcaattcctccaattcggaatttttcactataatatggattttgtgtatcgcattgtatacacgatgctgatgatgattaatgttgggtggtatataacttatgtgaaaacccaaaagtttgataaaataacattattgattgagagctcggaggggtcaggttatgaagaatga

SEQ ID NO: 317 - DNA, 1116 bp, Peribacillus Aracenensis
  source 1..1116: mol_type = genomic DNA
atgataaaaacaaaaaataacacacgcatagtagttggaatgtctggtggagtagattcttctgtttccgcattgcttctgaaagagcagggctatgacgtaatcggaatcttcatgaaaaactgggacgatactgacgaaaacggtgtgtgtacagcaacagaagattataacgatgtaattcgagtttgcaatcaaatcggcattccttactattctgttaactttcaaaagaaatattgggataaaatatttacttattttcttgatgaatataagtctggacgtactccgaatgcggatgtcatgtgtaataaagaaattaaattcaatgcattcttagaacatgctttaagtcttggggcagattatttagcaacgggtcattatgcccgtatagagaaaacgaatgacggagctaagttgcttcgcggtttagataaaaataaagaccagacctactttttgaatcagctttcagatgaacagctacagaaagttatgttccctataggaagcatggataaatcggaagtaagagaaattgcagagagagccaatttagctactgctaccaaaaaagatagtacgggtctttgttatataggagagagaaactttaaagaatttcttagtaattacctgcctgcacagccagggatcatcgaaacaattgaaggggaatctattggtaagcatgatggcctcatgtattatacaatcggccaacgacacggcttagggattggaggggctggtgatccatggtatgtaataggtaaggatttgaagcgtaatatcctatacgcgggacagggtattggaaacgaaaagctttattcgacttcaattgtggctataaatatgagttgggtatgcggtcttcctaagaataaattgttccaatgttcagctaagtttcgttatcgtcagcctgataataatgtaacggttgagcttcttgataacaatgaagcaaaagtaactttccataatccaatccgagcggttacacccggacaagcagttgttttttatgaaggagaagaatgtcttggtggaggaacaatcgatttagtatttaataatggagagcgactaacctatgtcagctga

SEQ ID NO: 318 - DNA, 564 bp, Peribacillus Aracenensis
  source 1..564: mol_type = genomic DNA
atgaatggtagctgtacaattgaaagtgaaagaaggaaatgggtattggattgctatttgaaaaagtacttaagcgagggaagaaaattggcagtaagtaaaacaaacgcaatgagaatactggacactaaccttatagaatatattatcacctcttatggtttagaggatggggaaattgacggtgtttctgttgctcaaaagctaggaagagaagctggcatagtatataaaacgcttgtggtacaaggcagcagtaaagaacattatgtttttttagttccagttgaagctcagctggatttaaagaaagctgctaaaactgttaaagaaaagaaaattgaaatgactgcggtgaaggatattcaaaaattaacaggatatgttcgcgggggatgctcgcctatcggcatgaaaaagctattccctactttcattgataaaagatcaaagtctcttgaaactctcattgtcagcggaggaagtataggaactcagattgaactgcagttagagaatcttgtcaaagtaacaaaagcccattttgcagatttattaagatag

SEQ ID NO: 319 - DNA, 1377 bp, Peribacillus Aracenensis
  source 1..1377: mol_type = genomic DNA
atggtgctattatctaaagatgtaacaacatctattaaagaagtaagtatgcttgtcgccaaagcgaaaaatgctcaagaaattttcgcctcattttcacaagaaaaaattgatgaaattgttaaaaagatatcattatactctagtaaagaggcagaaaaattagcaaaattagcaaatgaagaaacaggatttggtaattggcaagataaagttattaagaataaattcgcgagtgaagtcatttatgaatatataaaagatatcaagactgttggcattttaagcgatgaatcagcaactaaagtgatagaagtcgctgttcctgttggattggtagctggattaatcccatcgactaatccaacttcaaccgttatttacaaggcattaattgctttaaaagccggtaatgctattattttctccccgcatccgatggctttaaaatcaattattgaaacagtcaacattataaccgaggcagctatcgaagctggagcaccagaaggcattatcggatgtataacacttccaactatagagggtacaaatgaactaatgaagcatcgtgacgtctcattaattttagcaacaggtggggaagcgatggtgaaagcagcgtatagttcaggaacgccagccatcggtgtaggccctggtaatgcaccagcgtttatagaacagtcagcagatattaaacaggcagttaaacgtatcatagatagcaaaacatttgataatggtgttatttgtgcttcagaacaatctgttgttgtcgaacaaatatcgaaagaagaagtagttcaagaatttataaatcaaggagcatattttttaagtaataaagaatcagaagagttgtctcattttatactaagagataacggaacaatgaatcccgctatcgttggaaaatcgcctcaagcgattgctgatttgattggattaactatacctgaagggattcgcgtattaatttcagagcaaacgacagtaggcaaatggaatccgtattcaagagaaaaactaacacctattttagcattctacacggaagaaacatgggaaaaagcatttaagagatgtgttgaattactaatgaatgaaggtaaaggacatacatttattcttcattcaaataatgaagaaataattaaagagttttcgttaaaaatacctgtttctagaatgattgtaaatacgcctggttcccttggtggtattggcggttctgcaaatctaataccttcactaacattgggatgcggtgctatcggaggaagtgtgacttcagacaacgtcggtccattaaaccttatcaatactagacgtgtagcatatggagttagagagttagaagacataaaaggataa

SEQ ID NO: 320 - DNA, 1212 bp, Peribacillus Aracenensis
  source 1..1212: mol_type = genomic DNA
atggatgtgttacaaaatattaagtttcatgatattatcgatatagagacccttgaaaaggaattaattagactatcccattgggtaaatacgccaattagagtagtggatattaatggattttctgtacgtaatgaaagtaatttaatctcttattctgctttaatttacaaatctaataaaggaaataaacaatgcctgcttgatgattctcaagcagcttttcttgccatgcaacaaaataaagccatgacctatacgaataagagcgggttatcaaatggtgttgcagcaataagtgtaggcggtatatatattggttccgttatagtggggcaggtacttattcgaggtaaacaaactcatcaatcaattgatatagaattactttccgaagaatatggtattccacttaatcaacttcaaaaaactttagaaacgattcctattattgaaagtgaagagtttatcaatgacctatatttcgcttcacatatggctgaatatatcggaaaaattggtgagattaacataaccaataaaaaagtgtcagacgaataccaaaaacgcgtttttcttgaacagcaactaaaaaacataacttcaaataacaatcaatcacaaataaattctcacttcatactcacaacactgaatacaattgcaagaatggctctaattgaaaatgcatccgaaacagaagaattagtatttaatttatcagactggcttaggtataatctaaacagcaaagaggatttgcgtaaaataaaggacgaaattgaaaacaataaacggtaccttgatatcctatcgttacggtatagtgatcgaatttcctacaaaataaacatagatgacgaaatattagactataaaataccaactggtattctcctacctattattgaaaattgttttgtccatggacttaaagataagcaatctggaggagaaattattttatcaggcagaatggtaaataacggaaacatcctgattagggtttctgacaatggaaaagggatagagccttacatgaaaaatttattaaactcgatgaatgaaaacgttcaatcgtatgaagggtttagtttgcataatacacacagtcgtcttagaaactactttggacccgattacggcttaactatcgaaagcgaccttgtttacagaacgattgttattatctctattccttgtatcaactaa

SEQ ID NO: 321 - DNA, 768 bp, Peribacillus Aracenensis
  source 1..768: mol_type = genomic DNA
atgtgtaagctaatgattgtagatgacgagcctctagaaagacaagcattaagaatcattttaaagaggcgtttcttaaatttatgcattttagaagatgcaaaaaatggtgtggaagcaattcgacttgctacccgatttaaacctgatatcattctaatggatatccaactacctgggaaaaatggaatgtccgttcaaaaaaagattatacaattcttaccgaatgtaaagacaattattattaccgctctcgaagatttcaactgtgcacaaacagcattaaaatatggtgtattggactatcttttaaaacctgctcgtacgtcagatattgaaatcgccgtcgataaggccattaaatcaatcaaccaggtttctttattggatagtatttcatctaaacctgctacttcttccaaaaaagcaataaattcaattttaaattatatccatgcaaactataaccagccgttaacgttaaatgaaattgctacttatactcacttaaatcctcaatatttaagtaggtattttaaagaaacagttggtatgacattcacaatgtatttaacaaatttacgaatagaaactgcgaagaaattacttattaactctgataagtccattacgcaaattgctttggaagttgggtattcagacccttcatacttcagtaaagtgtttgataaacacgtgaaatcttctccttataaattcaaaatgagacattataacagggatgatataatgtctggaaagaagtga

SEQ ID NO: 322 - DNA, 2313 bp, Peribacillus Aracenensis
  source 1..2313: mol_type = genomic DNA
atgatggaagaaaaaggctgtgattttatgccaaagcataaaaaaaaacttctagaatttaatgcagaattatcgcaacaatggcacccggataaaaacggttcccttaccccaagtgacgttactcctggctctggtaaaaaagtatggtgggtttgtgagaaggcgcatgagtgggaggcatacatttatcatcgctccaacggtaagggctgcccatattgtagtggaaataaagttgatttaactaaaagtttagcagtgaaatttccaaacttaaaaaatgagtggcatccattgaaaaataaagtatcggcatttgaaattggacccggatcaggtaaaaaagcctggtggaagtgtcaaaatggacatgaatgggaagcggttatatcaagtcgtacaagaactggagctaataattgcccttactgctctggaaaaaaagcaagctctaaatataaccttgcaaaaaaacatcctactcttgcaagtgaatggcacccagagaaaaatggaattttaacaccatatgacgtaactccaggatcaggtaaaaaagtatggtggttatgtgaagaaggacatgaatgggaagtaacagttcatcaccgagctaaaggtaggggttgcccgtattgtagtagaagaatggttacaacagaaacttccttagctaatgataaccccactcttgcaagtgaatggcattcagagaaaaacggtacaattacaccacacgatgtaacaagtggctctggaaaaaaagcgtggtggttatgtgagaaagggcatgagtgggaggctgtaatttcaagtcgtaataatggcagaggctgccctaaatgctcaagcgctacctcttttccagaacaagcgattttttattacctatcaaatgcttatcagcaagtaacaaatcgaaccctcattgatgggatggaagtagatatatttattgaagatgaaaatattgccgtagaatatgatggagcgtattatcatgaaaaaaggtataaagaagataaaagaaaaactcgtgagcttctaaaaagaaagataaaactaattcgtcttcgtgaagagcctttaaaactattaaatatcaaaggactaatagaaatttcgacaaatcatcaggatttagaaagtgcattcacaaagctgatcgacattataaaggatattaccggaaaaacgatatcaactgaatttaaccttgatgaagacagagttgatattgttgaaaaataccgttttaaaataagagaatccagtattggaaaccatcctgaattaatgaaacaatggcatccagaaaaaaacgggaatttggacccatttaccttctcattaggctctggcgaaaaagtttggtggatatgtaaaaatggacatgaatataaaacgtttatcactcacagaacaaggggacatggttgcccttattgtaccggaagaaaagtcgatgaaagtaattgtctagcaaatgtaaatcctaaactagcaagtgaatggcatcctgataagaatggcgagttgactccatatgatgtaaccattagtgcaggacataatatttggtggaaatgtgaaaaagggcatgagtggagaacaaggattgttaaaagaagcaatagaggagataattgcccgtattgtagtggtcggcaagtaaatacagaaaattgtctagctaccctgaatccagtacttgcgagtgagtggcaccaagaaaaaaacgatgacttaacgccatttgatgttacgctcttttcaaataaaaaggtatggtggaagtgtcagaaaggtcatgagtgggaagcagtagtttcaagccgagcagccaatagaggttgtgcctattgttctggaaaaaaagcaagtgatgaatacaacttagctgtaataaaccctgaaatagcagcacaatggcacccgaggaaaaacggtgatttaacgccttatcatgttacacctaattccggtaaaaaggtttggtggttatgtgagagtgggcacgaatgggaaacaagcataacaaaacggaatggaagacagtatggctgcccatattgcagtggaagatatgctacaaaggaaaattgcctagcaaatgataacccatcgctctctaatgagtggcacccggtgaaaaatggtgatataaccccgtttgatgtcactccgaaatcgggaaaaacagcgtggtggaaatgtgaaaacggacatgagtggcaagaccaaatttatcaacgatcgctaggtaaagaatgtcctcaatgtaaaaagacgttttcaactagagtttaa

SEQ ID NO: 323 - DNA, 456 bp, Peribacillus Aracenensis
  source 1..456: mol_type = genomic DNA
atggaatattcatttgttattattttgatcttgttggggaaaatatctacagccaaaacccaagaaggtaggtcccatatgaagaagtttttactaatttttttcagtgtattttttattttaacaataccaatacaagcaaattcacaaaaggaaaataaaattgattacgaaaaaacaaaatatgctcttatagcaagccttagccctgccattaatgaagccgttgctaaaatctataaagatattcccggtggtgatcgtcaatgggcagggtgggaaactgaaattttatctattaaacaattatatggaattggtggggcatataggataacagtaaaaatacatacatatgttggtgcacataatccacctaatggaatagacacaatcactatagaagtaggtggaggggaacaaaaaattataaaatatgaacataaagaggattga

SEQ ID NO: 324 - DNA, 705 bp, Peribacillus Aracenensis
  source 1..705: mol_type = genomic DNA
atgcctattattaaagatattcagttatacgttccgaagaataagaatctgaactggtcgttcttccatgagactagatgtattacttttttctatagtcgtcttctgccgaaactacaagcaaaagatgataagggagtacagatctattgtataaaggagatagaacagagagagcaaattgacacattcgccctcatcttcaactacttccctgtatacgtggaagcagatgctgagggtattttatctttgacctccggtagagaaaagaaggagaagactcttgaaatcgtgcacgaaggtatgaaacgtgctgcagatgaattaaactgggataaggcaatacttgatgacatttataaaagtattaaacaatcaggttatgagaatatttatccactattgaaaaagaacagtcccaataggaagtacgtatgtagcatcatctgtcatcatgagataaataccattgatgtatacatggaaattaaaaagagaaacggtgatatcgtcaataaagaactgctattctctgttgaaaatacggacgaacagcatttatttagtgattatggtaacttaaaatggagacttaaccacaaggtagagttttccgataaggactataaacaagtctatcgtttaacgttccttgaaaaggacaatcctgaaaatttagtgtggaagattgaaaagaactaa